European Patent Application EP 4 428 232 A1, published September 11, 2024. Title: 分离的Cas13蛋白及其应用. Applicant: 广州瑞风生物科技有限公司. The sequence listing filed with the application follows.

SEQUENCE LISTING (105 sequences)

SEQ ID NO: 1 - protein, 1025 aa, synthetic construct
MNPQARTRKPETPLKPVGNEHFAVFINIARHNAFIAITELSKIYGMTPPNEDELATSRFIAAFDSTTIDVRKLKQRLKRLSSLMPFLKSLQDKTDAEIIGILKDLLSLVNQFRNYYSHYNTSDFLTINSNEFITSDKVSILENIFEKAVLSLTNSEKAYDRFEIISLLKSEKRADKPYFYEFIENNKISEKAIAFFFCLFLDKPNAMKFLKRLKGFKGADTKQFRATLEAYTTYCIQLPEPKFLSDRPNLAIILDGIEHLKRCPIEVHKTLSFRDKQKFERKVMREDLNGDLQEENIELLRYDDRFAEFAMRYLDDFDILSDAKKQNTYRFEIQLGKKVVESKKLAEETTEAQDKIPVRFKPVKAFGKLADIPRKKDEAVIDWQQDLEELYAYEPHYKIENHSIGIKKIATEDTFRLNNPEELPDAYLSEYQLRNIIFLSLESSNKEEFFMACQIRIGKIKSLYKALSAPTHYKESIKQKYNELINNNLLPKPLVKYLTHSLDELPTYKSKAIKKLKFWQDETENLLAEVKRHNEKSEKARKENKFFKSFLKSGQIATWLIKDIQHFLPLQGKLSVLKYNALQAKLAIYNSEELKEMLTDFQVYDTPKGTDRNMPEKGGGHQFIKTVFDKNPQKLPPHWLHFYNDYLNAKKQWIEDKIKFLTAMPDTEAEIMKQQPLFYFLDLGSNYEEGEKIVYFRENSPAYIAKYCEELLKKPVDLPIALSYDLVANMRTGLEKAKSVTDFIDDKYQSEPPYYHLPRQYDLFKAFGDKPSEKLFATDKKPLHEVYGEYKAKKTDPRTIKKIKGFLDQEQRIRYLKVCDKLLVKILEKYLAKETELKNVQLTDAQGKLILDKVLETEFEMPPYGFKVRLKDYGRYRRFVKDRRLVSMQDYLNQSVFTPDTLITELNLYEKQRSEFLKIVLEFEKRLLSASDTLNINLADQQTTLGEDKIRDYITHNYLLEVALRNNFISENEARAMLWFRNGALHNQLPDLQKLVGLIDTEEQKTQRYFLKGMEMYKKGIEKIS

SEQ ID NO: 2 - protein, 1192 aa, synthetic construct
MTILEKYMPLNEMGKIKSLVDELKGIPGAMNATLRQEIFQNIKKTKLQVKFLEEYPETLFTDSGNLIPIIGNNDNSSSGTPSKQEVSDIDANQASRINYLPHETMGEIKSVYGTYIEMAFHNFYLTMHHIYAVVFGEDIMEEAKKEFDKNNTNSTKYFTFDFANERTIWKPMFDRAERAKPEQKEHFEKLVVKHFPFLKAIDALEDRKRKTKIQALCVFSLVLRELRNVYSHYLFYPFKNQVDKYKENIPFVLDMMEILYTGAQREVKGRFGFDDKKMQCAKKYERNKDHSQRDHQGKIIKAVPKKNFRYNLYKKEDSEAIITPFGLVFLTSLFLEKKYAKILSDKTHCIKYTDQEVLCEIISVYRIRLHIQKLSVTKDTDALALDIINELQRCPKRLFEMLSPDDQQKFRIKPTDSQYADDVLMIRHQDRFAHLLLKYIDDAHLFNCIRFQVSLGRYFFRFYDKSCIDSTGDKRVRSISKNVNGFGRITDIEDYRKEVYGDMIREYEDVHANTSMEKPYITDHHAKYLISNNRIGLYIRKEEDTQCLLPELTPDGARNFAPTCWLSIYELPALAFLLHLYNGDGSRVEEIIQTKVANYQRLFADVRDGKVCPVKDEAELTTILQTYGNIEPSQLPRKLLDYLLKKEICAQDLFNTWAQSKIQRMIAQTDSLLQHLEKDLQAVSDLKQNKFGKKAFVAIKPGHIADFLAHDMMFFQPSMKDCNNKLTGLNFRILQSSMAVYDGNFDELSRIMRSAHIIGNANDACCNPIVMAVCRKHKGFSNIIRFYQAYLKERKAYLQQCANERHYDSLSFLHASQNKWRERTQAYYRSLAAKYLAENYDGVDTTKSIELPRGLFETYIRQELSEIGSTKSMAGDATKNTSYLIYGYFRQVMSDDAQTFYDTRRCYQLFDVLYRKSPRDNHSYYSTAQIREMLMRSHSKSIRKDIDNYISQTTAAERTKEKERCDALLRKIKDTETELKVYKIQDILLFLIAKRLLLDRKVENDSAVQMNAINQIRLRNIADGNTLSQKIPISISIKSRKGDPKIIQQDDLKLKNYSQFYSIISDRRLPSLLDLINSRVIKRTDIEDELSNYDKSHPHVLKSVFEFEKHYFDTHPIPSDTAYMALPDTGEMLKESNLTAEKQKEVRKIRNSFAHLSYPSRNITGAASTELPKKAEIISKNLIEHLSNAEIK

SEQ ID NO: 3 - protein, 1272 aa, synthetic construct
MYHLSDANHGKHIAGTYYEMAMGNFIHTLSHMLVRAGIKVNKLEDNYSIEREIMNLTAPGAYDAQRAALSRLLYRHFPFFGPIMADHTDHILSSKRKKVQSASDDGNLDLGQELKDEVAGASACQMIRYLATIAGALVYYRNMYSHKNHYDNAQDIAAQQEREQKLALWLDVVFRGARDILLTRKSHPQPDTDFLTQNGTINYYIEKNGKSAYNPNFYFKPGLKTDNGWVMTDFGKFFFCSLFLRRADAERFAAETDLYVGSPFKITAQERARLQEAENKRAADEQARASSAGFPHIVNPRTIGPSESPQNNIIREMLNMHRARIPRERRIDADMSEGILAMDIMNELRRCPLSLYNTLSPEAKASFEKTGVTPEGGIVSNLLVRHSDRYPELALRAIDQMELLPTIRFHVRLGSLRFRFYEKKLIDGSHTLRTVQKAVNGFGRWQEVEPRRVEKYTAIQARCQNDKGIDQFLPDSPTTTPYITDWRTTYNIHANRIGLAWNLPQMSDGIYLPNLDTDKGDNLHRKALIDMPAPMCYLSIFDLPALLFYCHIYTHYHGTKYHLPSAESIIQAKYDALHKFFSFAAAQNHSAEQLREKQLELNLADNEIPDKLRCMMQTKPFFKNGRQQLSPLGYPIMKNWIGVAEQRKHAAQVLRDVANEAADRLASFEKKHQRVVVGGRDNRYGRRGHADIRHGSLARYLATSMVRWQPALDQPGGDKLTSANHRALAGFLSEYGLHGSNINKLRNVLKEAGLIEGSHPHPFLAHVLESAPANIEALYVAYLKHEQSHATALKNKFTDRNGIVQPSEVPAFVRFNSSRWRNDSATTARRYLQTPPAPGSSDSAEHNAPIMLPDGLFTTHIMTLLNKVLGQNDRVPEEDYLRHDLPRIASIINPNGKTYGAAYIIRAWFDQVENQDVQPFYDLPRFYREISLLAPRRKPNQELIRDYFSEEQIAQKIQTVPKKQRSEKVGHTIDTEKDIRRYRLQDITLYLTLLDMLTLMLSRNEAERTDRQMKSSTAERVSNMRLVDFDHSFDFDLLGSTSGEAAYSYLHQRSGITISMPALSLRSYGSIFRVLADSRFETLMDALNRQGVTHVNFGDITSELALYDTLRSHFLLQAHNVEQDAFSAKRGVLENHTSPFFYRSGNLQLDDQGNITNPSTDAIRNHYGELIKILDRYSLKIDKKTKDGKSQDILLRDLMAELRNAAAHNRYPKADFFFRQFDHFLNTCKPTDSNLTAPNYIRTVLEFLKSIVDNNFTPLLHEESPENESKSE

SEQ ID NO: 4 - protein, 1183 aa, synthetic construct
MPMSTIIDKYMPLNDWNRIESLIGELRAISGAMNCAVRRAVFENIKKAKLQIKFNDQYPESIFTDKNGSIPIVGTTEANNPENGGNNECEQSNNYLSIDYLPRVTQEDKKSVYGTYFEMAFHNFFITLHHIYSLIFGEDIMEVAKSEYSQTQTDSFQDDFANKYTVWNPLFTRLRRAKAEQKERFEELAIKHFPFLKALDALKGENRVSKVDALERFSVVVRELRNIYLHYCIIPSDKQKKEYSDNISFIFDLMDLLFTGAKREVKTRFALSDDQMSCADKYEPNSDRSLRDIHGKTLRIVPKKNFRYHLYKVGDDAKIISPFGLVFLASLFLEKKYAKILSDKAHVVRLNDKGVICEMISVYRIRLHINRLSISKSTDTLALDIINELQRCPKKVFELLPPVAQQRFRVKPESSHAPEVLMVRHNDRFVHLLLKYIDDAKLFEHIRFQVSLGRYFFRFYDKICIDTSSEKRVRSICKDVHGFGRISEIEELRREKWKDILREYDEVHANTADEKPYITDHRANYLIGNNKVGIYLLKEGDEQCIMPELLPNGARNHAPTCWLSTYELPALAFLLHLYNADGARVEEIIEKQVAGYRRLFADVRDGSVAPVASVEELDELLKGYGDMQACNLPRKMLDYLLMKDVNAHDLFRKWAEAELQQMIEQTDRLSQRIDDDIKAAANMRQNKFGKKSFVAVKPGKIADFLAHDMMLFQPCTEDNSNKLTGLNFRILQSVMAVYNGDFDELSRVLRNAHIIGNATDEMCNPIVMAVCHKSMEFGNIVDFYKAYLRERRIYLERCLRHGDFESLGFLHASQIRWQERSKEYYRALAARYLVDEYGGTESAKAIELPRGLFEPYIRKELSEMNAMKSLACNSDYNVSYLIYGYFKRVMSDDAQPFYDEKKCYRLFNVLYRKSPHDSPVYRNTAEIRDMLMQNSPNSIRKDIESYLSNTIIADRAKEKERCTALLREMKKCETELKRYKIQDMLLFLIAKRILSDLPAAHDSAVQMQAISRIHLKDITDGNTLSEKISLSVKVVSKNGYIKKLTQHNLKLKNYSQFYAILSDRRLPSLLDLVRSNYINRNDIEAELDNYDKVHPEVMKAIIGLEKKHFEKHGFDDSGIVPDLSSILAETTMPADKQYEVRKIRNSFAHSHYPGYHVANAGITELPKKAETIFNTLKSSLSDE

SEQ ID NO: 5 - protein, 1190 aa, synthetic construct
METTINNRIGKGEYYTEESKEFLAAYFNQAIHNVFIVLNHIAKRFGMDELSSDEELKNWLIGRQREKKRNAIDRQRFLELIDRHFPFLRIANADKKDAKRENDLEDNLALLITLLNDLTERRNKYSHAITHASIESNDRELVWRLYSIYDANINLVKRDYFESNVHTEINEDPYEKQVEHLRRFCMNNDRTKVDEKGKKKPAMPNPRFRTPFLNAETNQLSIYGLVFFVSLFLEKKYAIQMQKNVYGLKDARDTKFKMTNEVFCRSRIIMPRVRLHSDKSTDALVLDMLNELAKAPEVLFDQLTDPFKEKFYIESIDSLEESDIITPVRAIRKQNRFMYFALRYLDESNAFSKLRFQIDLGNYHYHLYESKINDQTESRHLTRKLFGFGKLIAFEQEFAPEEWKMKSKDLDYYEGATQPFIAKTYPHYHLEENKIGILFNGQAEVQWPHLDVEEHESFPKYKRRANEKADAFLSGNELLAAAFCHHLYASIGKPNTVEKIIRDKYHALRQLFSDLKSGNLQNLLGDNTSNEAISQLLFEKYRLTLSEVPVRLHAFLSGQEQADTKAIARGKLELMAQQNKKRIERFDAMKKAVVKVGKAQYRTLRSGDIGDWLVRDFMRFQPIGYKRNQAGKQEPDLKSKANPKKYQLIQKSLALYEQEKNNLLGLFKSCNLLSSENEHPFLNEVVQSMPATWQDFYERYLHARSRFLEKCIEKGIKKNSYQACYSFLKIKPQLKDKEKLYQGWDAQMNLPTNMFIDAIHDWFRQTHHESLRTWFTQQEKPHQLIGLIRKYIELAHTDQIQGFYDMFPLRYDFYKKEFPNGLVLHERINKQKQIWEAQLIQTKKRLEDAASKLKKVKQQVESLPDQELRFRNETEAMVYFTKLFDSSIVKNAILKLQRDQKALRVNTIGEKIIKIYTAKYDAIHQEVRDFKSMLTTEKMIRRVKAEDCVTLFMLTDLMNQSQITIGQEQRTIKLSDIQPMGETQIQGILDAVQVLEQKLDFFSSDEQGKISQVKLGEWTIFSTDTKVKKQGNFKQLLKDRRLNNLAHYILPDIAGGAIRVRRNLLEMELDQYDRNRIPIIKLMYELEYAIYKVDPFSVELKYKKFSQCLREYAQKAVLNVEQVEHLNVLIAIRNAIMHNQYPNRDHLKAIVPFTVSEYAPVQEGLTIARQLLACAQVSVNIILSTISKFE

SEQ ID NO: 6 - protein, 1158 aa, synthetic construct
MKEKIKNKSSIIRIIMSNYDDKGLKEFKVLYNKQGGVDTFTCKTDIVDGTIIFLEIEKHLRDFGDDFSWDISSDGKSVEITKLINGKETRKYKVSIKNSSTKDKKNLVELEVEDLKESAIDRRRTKSSTKRVLLSKDVMERYAEIAFSKKERWEEIDSQKIYKVKRFLDYRSNMLIYFQFINDFLTKGIPDELDKNGEIKQLELWKLIDDDETISDKNLNQVSKNLYTYISQEIKDSQTRAENNREKNKEKEHFKEFYAFNDISEESIREDVKKFIYLYANLRHNLMHYNYSFFENLFEGKDLVIEKTKSLLSSTLDLNIFKELSNIVELREENKTNYLDDETTIRVLGKEKKAKTLHKIYSILCSRKNGFNKFINSFFSTDGIEEEFLKSEIKKDFLERLNWVEKSLIEKINNPPSDTKLKYKNDKTIENMTKEKEEKLELISLLNPQVSDYKTENFTPYYWDIHQSPSYKKLYNDRKVLVSELSKLIAIGINSDTKKRITDLNAELLKIKIKMEKITKLNSKIRLQYKLQMAFGFIYANYSKVYKEKRVLNINGFVQNFDPTKLNKEKELESRLIYLKAPYNIFEDNKSLDFNMKIVENIPVSEKSIFRIKPENNLSKFYILSYLLLPVELRGDFLGYVKHHYYGIKNVDFEEIPDIKEDKPNENSDSFFHNLRLFEKNSKKFELIKYRLVEFGNLKDHLPRIYEKFGIKPDVLEYIENSGNKDSKLFDRNILLPIMKYYQHIFKLLNDIEVHALLRFSEKDSISLDESIKECSKGKFLNFGKLLFLSRYGLEAKKDNKFKDIFNRENGLSITKDDAKTERKKYFEIFETRNKIAHLNYKQLFHDLLFDSNININKELEGIIQETKTIGLNAQTLGYNFLNDFYMRKEMFISNQKKSSMTLINNPLSKDKDTKEIGLLKLYGLSKSQPKDLILAKYKELMNLIEKTEDSILKKKDFLPVKEVSITVKKSTPNKKGIMVELPEILQIKDLNEMDLLAYASNIRGKLHKDSSDLFGIYKKLTIKELKKKLINLFIKGEKRYLNLELVNKTGYMAIYESTGLYPKSYEILNHEISFSEISMKNWYEHDFKPIFQIDGSLPNNTDYKNGVFIYTSPYEFRDKELMKKQRTVHKRDIEKTFYNENDMDYTGIYNQKIKALY

SEQ ID NO: 7 - protein, 931 aa, synthetic construct
MMGNKKSVAKANGLKSTFVLGENTAYMTSFGRGNAAQPEKHIRDATVTDIQHTFRAKTDGGRTVHIEGRVGASDVLLPDAANQLHAKDAVEQMYFGKAFSDNIHIQIAYNIMDIKKIFGVYANIIVHTVNNLCCDGDKQDDFLGMFKTQNRYQVAAWAHKIVSLHLVKNELRGGGFFMDQEVWRAHVRTDFKSLNLAVNAFMKKYPQKYPYWSVKIVSDFIVQEMGIKNKVILEKAAESYAEFETVAKRLEKSAYYFSDIFAGKDGKFDEQKAFDLLRVLGMMRQEAFHEKNSSASWLYNLDAEADEDIKAALRTVVDTKVNGINTNFAKQNKVNLLVLQEIYPQKSKADLVREYYDFSVRKAFKNLGFSVKTLRETMCAFDAASVITDKQYDTVRGKLYSLFDFVIYNYCLENEAVCNAFVEELRANLDPENKTALYQTLAEKVWAEIGDIVLQRILPQMHAKKIQERSKETDAETVEMQGYVQAPKDLSLFSKAVYCISMFLDGKEINSFLSALINKFENISSLCAVLAYNGLEPEFVAPFTFFADSQAIAEDLRYIKSIARMSKGKKATKDSPVTVKEMQYFDAAAVLGETDTEKVKAAFHLGDKSASTADKAFRNFVVNNVINSNRFVYVVRFINPKNAREIMQNRALIAFVLKDIPQSQLVRYCGTAGIACNADEPNTEAMVNALADMLLQVRFDAFSNVQQKVKADSAEAVQKEKYKAIIGLYLTVLYLLVKTLVKINMNYAIAFGILERDCQIMNQKHGKNPKRDRDAFYMREQQNKQYVYNARAITELFIENGWLNKRVQKSVENNAALYSDEAFYKYRNLVAHLNVISALPKYAKNITKVKSLFDVYHYILFLSLCEDKYSNLPEAVTKSLCKNGKTMLENAREYQTVCKDFLYGLNTPFAYNAARYINLSNREKFLAGFGK

SEQ ID NO: 8 - DNA, 3078 bp, synthetic construct
  source 1..3078: mol_type = other DNA
atgaatccacaagcacgtacacgtaaacctgaaacaccacttaaacccgtaggaaatgaacattttgctgtatttatcaatatcgcacgccacaatgcttttattgctatcactgagctaagtaaaatctacggtatgactcctcccaatgaagatgaattagctacatctcgttttatagccgcctttgactccacaacaattgatgtacgtaagctaaaacagcgattgaaaagactttcaagtttgatgccttttttgaaatctttacaggataaaaccgatgctgaaattatcggaatccttaaagacctcctctctcttgttaatcaatttagaaactactattctcactataatacttccgattttctcacaatcaatagtaacgaatttattacttctgataaagtttcaatcttagaaaatatttttgaaaaggctgtcttatcattaaccaattcagaaaaggcttatgatagatttgaaattatttctttactgaaaagtgaaaaacgagcggataagccttatttctatgaatttatcgaaaacaacaaaatctctgaaaaagctattgctttcttcttctgtttgtttttggataaacccaacgccatgaagttcttaaaaaggctcaaaggatttaaaggggctgatactaagcaatttagagcaactttggaagcctatacgacttactgtattcagttacctgaacctaaatttctatctgaccgaccaaatcttgccataatcttagacggaatcgaacatctaaaaaggtgtccaattgaagttcataaaacccttagtttcagagacaaacaaaaatttgaacgaaaagtaatgagggaagacctcaatggggacttgcaggaggaaaatattgaattactcagatatgatgatagattcgctgagtttgccatgcgttatttggatgattttgatattttgtccgatgccaaaaaacagaacacataccgttttgaaattcaattaggaaagaaggtggtagaatctaaaaaattggcagaagaaactaccgaggcacaggataaaatccctgtcaggttcaagcctgtgaaggcatttggcaaattggcggatattcctcgtaagaaagatgaagccgttattgactggcaacaagatttggaagaactatacgcttacgaacctcattacaagattgaaaatcactctattggtatcaagaaaattgcaaccgaagatacttttcgtttgaacaatcccgaagaattacctgatgcttatctgagtgaatatcagttgcgtaacattatttttctgagtttagaatcaagcaacaaagaagaatttttcatggcttgccaaatacggattggtaaaatcaaaagcctatacaaagctctctcagcacctacacactacaaagaaagcataaagcaaaaatataatgagctgattaacaataatttactacctaagccattggtcaaatacttaacgcatagtttagacgaattgccaacttacaaatcaaaagccatcaaaaaattgaagttttggcaagacgaaacagaaaatttattggcggaagtcaaaagacataatgagaaatcggagaaggctcgaaaggaaaataaattctttaagtccttcttgaaatcagggcaaatagctacttggttgataaaagatattcagcactttttgcctttgcaaggtaaactttctgtgctaaaatataatgcacttcaagctaaattggcgatttacaattcggaagaattgaaagagatgctcactgattttcaagtctatgataccccaaaaggaacggacagaaatatgcctgaaaaaggcggagggcatcaatttatcaagactgtttttgataaaaatccccaaaaattacctcctcattggttgcatttttataatgattacctcaatgctaaaaagcaatggattgaagacaaaatcaagtttctgacagccatgccagacactgaggctgaaattatgaagcaacagccacttttctactttttggatttaggttcaaattatgaagagggtgagaaaatagtctatttccgtgagaactcgcccgcatacatagccaagtattgcgaagagttactcaaaaagcccgttgatttaccgattgccctgagctatgaccttgtggctaatatgcgtacaggcttagaaaaagctaaatctgttaccgattttattgacgataaatatcaatcagaacctccatattatcatctcccaagacaatacgatttattcaaagcatttggcgataaaccttctgaaaaactgtttgctactgacaaaaagcccctgcatgaagtgtatggagagtataaagccaagaaaacagatccaagaacgattaaaaagataaagggatttttagaccaagaacaacgcatccgatacctgaaagtttgtgataaactcttggtgaaaatattagaaaaataccttgccaaagaaacggagcttaaaaacgttcaattgacggacgcacaaggaaaattgattttggataaagtgttagagacagaatttgaaatgcctccctatggtttcaaggtgcgtttgaaggactatggacgttatcgccgttttgtcaaagaccgccgattggtttctatgcaagactatctcaatcaaagtgtctttacgcccgacacgctcattacagaattaaatctttacgaaaaacagcgaagtgagtttttgaaaatagtgcttgaatttgaaaaacgacttttgtctgcctcagacacattgaacattaacttagctgaccaacaaacaacattaggtgaggataaaatacgagactacataacccacaactaccttttggaagtggctttacgaaataattttatctcagaaaatgaagcaagagccatgttgtggtttagaaatggagcattgcataaccaattgcccgacctacaaaaattagtaggtttgattgataccgaagaacaaaaaacacaaagatactttctgaaaggaatggaaatgtataaaaaaggaattgagaaaatatcataa

SEQ ID NO: 9 - DNA, 3579 bp, synthetic construct
  source 1..3579: mol_type = other DNA
atgacaatcctggaaaaatatatgcccttgaatgaaatgggcaaaatcaaatcgttggtcgatgaacttaaaggcatccctggggcaatgaacgccaccctacggcaggaaatctttcagaacatcaaaaaaacaaaactacaggtaaagtttttggaagaatatcctgagacgctttttacggattcgggaaatctcattcctatcattggcaataatgataactcatcctcgggaacgccctcaaaacaagaggtctctgacatagacgccaatcaagcaagccgaataaactatctgccccatgaaacaatgggagagataaaatctgtgtacggcacgtacattgagatggctttccataacttttacctgacaatgcatcatatctatgcggtcgtctttggagaagacatcatggaagaggccaaaaaagaatttgacaagaacaacaccaactctacaaaatacttcaccttcgactttgccaatgaacgaaccatatggaagcctatgttcgatcgagctgaaagagcaaaacctgaacaaaaagaacacttcgagaaattggtcgtcaaacatttcccatttctcaaagcaatagatgcccttgaagacagaaagagaaagacaaaaatacaggcattatgtgtattctcgttagttttgcgggaattgagaaacgtctattcacactatcttttctatccctttaagaatcaagtagacaaatacaaagagaacatcccctttgtacttgatatgatggagattctatataccggtgcccaaagagaagtcaaagggcgctttggttttgatgacaagaagatgcaatgcgccaaaaaatatgaacgcaacaaagatcattcacagcgagaccaccaaggaaaaatcatcaaagctgtaccaaagaaaaactttagatacaatctgtataaaaaggaagatagcgaggcaataataactccctttggcttggtgtttctcaccagccttttcctcgaaaagaaatatgccaagatcctatctgacaagacacattgcataaaatatacggatcaagaggttttatgtgagattatctcagtatatcgcattcgcctgcacattcagaaactcagtgtcacgaaagatacggatgcgttagcccttgatattatcaacgagttgcagcgttgtccgaaaaggcttttcgaaatgctatcaccagatgaccaacagaaatttcggatcaagcctaccgattcgcaatacgctgatgatgttttgatgattcgtcatcaagaccgtttcgcacacctcctgttaaaatatatagacgatgcccacctctttaattgtattcggttccaagtctctttgggccggtatttcttccgtttctatgacaagagttgcattgattccaccggcgacaaacgggtgcgctccattagtaagaatgtaaacggatttggaagaatcactgacatagaagattacaggaaagaagtgtatggagatatgatacgcgaatatgaggatgtccatgcaaacacttctatggaaaagccttatattacagaccaccatgcgaaatatctgattagcaacaacaggattggcctctatatcaggaaagaggaagatacgcaatgccttttgccagagctgacgcctgatggcgcacgtaacttcgcaccgacgtgttggttgagtatttatgaactgcctgcccttgcttttctacttcacctttacaacggagacggatcaagggtagaagaaattattcaaacgaaagttgccaactaccaacgcctgtttgcagatgtccgagacggcaaggtctgtccagtgaaagacgaagcagagttgactacgatactccagacctacggaaatatagaaccatcccagcttcctcgcaaattgcttgattatctattaaagaaagagatatgcgcacaggatttgttcaacacatgggcacaatccaaaatacaacggatgatagcccagaccgacagcctgctgcaacaccttgaaaaagaccttcaagctgtttctgacctcaaacagaataaattcggaaagaaagccttcgttgccatcaagccggggcatatcgcagactttctggcacacgacatgatgttctttcagccctccatgaaggattgcaacaacaaactcacagggctgaactttcgcatcttgcagtcatccatggctgtctacgatgggaatttcgatgaactgtcacgtatcatgcggagtgcacacatcataggcaatgcaaatgatgcgtgttgcaatccaattgtaatggcggtatgccgcaagcataaaggattcagtaatatcatccggttctatcaggcatacctgaaggagcgcaaggcatacctacagcaatgcgccaatgagaggcattacgactccttgagtttcctgcatgcatcacaaaacaaatggagagaaaggacccaggcttactaccggtcattagcagcgaaatacttggcagaaaattatgacggtgtggataccaccaaatccatcgaactgcccagaggtttgtttgaaacatatatccggcaagaactctccgagataggtagcacgaagtccatggccggcgatgccaccaaaaacacatcctacctcatatacggctatttcaggcaagttatgagcgatgacgcccagaccttctatgatacccgcagatgctatcagctgtttgatgtgctttatcgcaaatcaccacgcgacaaccattcctactatagcacggcacaaatccgcgaaatgcttatgcgcagtcactccaaatccattcgcaaggacatagacaactatatatcccaaacaacggcagcagaaagaacaaaagaaaaagaacgctgcgatgccctgcttaggaaaataaaagataccgaaactgaactgaaggtctacaaaattcaggacatattgcttttccttattgccaagcgcttgctgctggacagaaaagtggaaaatgactcggcggtgcagatgaacgcaatcaaccaaattcggttgaggaacatcgcagacggcaatacactctctcagaaaatacctattagcatcagcataaagtcaaggaaaggagatcccaagattattcaacaggatgacctaaaactaaagaattactctcagttctactcgattatcagcgaccgccgtttaccatcgttgcttgatctgattaactctcgagttattaagagaacggacatcgaagacgaattgagcaactacgacaagtcacatccccatgtactgaaatccgtctttgagtttgaaaagcactattttgatactcacccgataccatcagataccgcctacatggcattacctgacacaggcgaaatgctgaaagagagcaacttgactgctgaaaagcagaaagaggttcgcaagatacgtaattcctttgcccacctttcatatccgagcagaaatatcaccggtgcagcatccacagaattgcccaaaaaagcagaaatcatatcaaaaaacctgatcgagcacctaagcaatgcagaaatcaagtaa

SEQ ID NO: 10 - DNA, 3819 bp, synthetic construct
  source 1..3819: mol_type = other DNA
atgtatcatctttcggacgcaaaccacggcaaacacatcgctggcacctattacgaaatggcgatgggaaatttcatacacactctttcacacatgctggttcgtgctggcatcaaagtgaataagctggaagacaactactccatcgagcgcgaaatcatgaatctgaccgcccctggggcgtacgatgcccagcgtgcggctctgtctcgcctcctttaccgccacttccccttcttcggccccataatggccgaccacaccgaccacatactttcctccaagcgcaagaaggtgcaatctgccagtgatgatggcaatctggatttgggccaagagttaaaagatgaagttgcaggagcttcggcctgccaaatgatccgctatcttgccaccatcgctggggcattggtctactatcgcaatatgtactcgcacaagaatcactacgacaacgcgcaggatatcgcagcacaacaagaacgcgaacagaaactggccctatggttggatgtcgtcttccgcggcgcacgcgacattcttctcacacgcaagtctcatccccagcccgacaccgacttcctcacccaaaatggcaccatcaattattacatcgaaaaaaacggcaagtcggcctacaatcccaacttctatttcaaacccggactgaaaaccgacaacggctgggtgatgaccgacttcggcaaatttttcttttgctcgcttttcttgcgcagggccgatgccgaacggttcgccgcagaaaccgacctctatgttggcagcccgttcaagattaccgcacaggaacgtgctcgccttcaggaggccgaaaacaagcgtgccgccgacgagcaggctcgcgcgagcagcgctggatttccccacatcgtcaacccacgcaccatcggcccgagcgagtcgcctcaaaacaatatcattcgcgaaatgctcaatatgcaccgtgctcgcatccctcgcgaacgccgcatcgatgccgacatgtcggaaggtattctggcaatggacattatgaatgagctgcgccggtgcccattgtcgctctacaacacactctcccctgaggccaaagcctccttcgaaaaaacgggcgtcacccccgagggggggattgtgtccaacctactcgtccgccattccgaccggtacccggagctcgcactccgtgccatcgaccaaatggaactcctccctaccatcagatttcatgtccgcctcggctccctccgattccgcttctacgaaaagaaactcatcgacgggtcgcacaccctccgcaccgtccaaaaggcagtcaatggcttcggacgttggcaggaggtggaaccccgacgcgttgaaaaatacaccgccatccaggcccgctgccagaacgacaaaggcatcgaccagttcctcccagacagccccaccaccaccccatacatcaccgactggcgcaccacctacaatatccacgccaaccgcatcggtctggcttggaacctgccgcaaatgtccgatggcatctaccttcccaatcttgataccgacaagggcgacaatctacaccgaaaagcgctaatcgacatgccggctccgatgtgctacctcagcatcttcgacctccctgcactgctcttctactgccatatctacacgcactaccatggcaccaaataccatctgccctccgccgagagcattatacaggccaaatacgacgcactgcataagttcttttccttcgccgcagcgcagaaccactccgccgaacagctgcgggaaaaacaactcgaactcaatctcgccgacaacgaaatcccagacaaactccgatgcatgatgcagacaaagccgttcttcaaaaatggacgacaacagctttctcctttaggctatcccatcatgaaaaattggatcggtgtggccgaacagcgcaaacatgcggcccaggtgctccgcgatgtggcgaacgaggccgctgaccgtcttgctagcttcgaaaaaaaacaccagcgcgttgtcgtaggcggacgcgacaaccgctacggccggcgtggccatgccgacatacgccacggctccctggctcgctacctggcaacaagcatggtccgatggcaacccgccttggaccagcccggcggcgacaaactgacctccgccaaccaccgcgccctggcgggcttcctgtccgaatacggactgcacggctccaacatcaacaaactccgtaatgtgctgaaagaagccggcctcatcgaaggctcccatccacaccccttcctcgctcatgtccttgaatccgcccccgccaacatcgaagcgctctacgtcgcctacctcaaacacgagcagtcccacgccaccgcgctgaaaaataaattcaccgaccgcaacggtattgtgcagccgtccgaggtacccgcattcgtcaggttcaattcctcgcgttggcgcaacgactccgccaccaccgcccgccgctaccttcagactccacccgcacctggcagttccgactctgccgaacacaacgcacccatcatgctccctgacggcctcttcacaacccacatcatgacactcctcaataaagttctgggccaaaacgatagggttcccgaggaagactacctgcgacacgacctcccccgcatcgcctccatcatcaatcccaacggcaaaacctacggcgcagcctacatcatccgcgcatggttcgatcaagtggaaaaccaagacgtccagcctttctacgacctcccgcgcttctaccgcgaaatttctctgctcgcaccgcggcgaaaacccaatcaggaactcattcgcgactacttctccgaagagcagatcgcacagaaaatacaaaccgtccccaaaaaacaacgctccgaaaaagtgggccacaccatcgacacagaaaaggacatacgacgctaccgcctccaagacatcacgctttacctcaccctgctcgacatgcttaccctgatgctttcacgcaacgaggccgaaagaaccgaccgccaaatgaaatcttcaactgcagaacgtgtctccaatatgcgcctcgtcgacttcgaccacagcttcgacttcgacctccttggcagcacctccggcgaggccgcctactcctacctccaccaacgcagtggcatcaccatctccatgcctgccctctccctccgcagctatggctccatcttccgcgtcttggccgacagccgcttcgaaaccctcatggacgctctgaatcgccagggggtgacacacgtcaacttcggcgatatcacctccgaactcgcactctacgacaccctccgctcccacttcctcctccaggcacacaacgtcgaacaggacgcattctccgccaaacgcggcgtcctcgaaaaccacacctcaccattcttctaccgcagcggcaatctgcagctcgacgaccaaggaaacatcaccaacccttcgaccgacgccatccgcaaccactacggcgaactaatcaaaatactggaccgctactccctcaaaatcgacaaaaaaacaaaagatggaaagtcgcaagatatcctgctccgcgacctgatggccgaactgcgcaacgccgccgctcacaaccgataccccaaggccgacttcttcttcaggcagttcgatcacttcctcaacacctgtaaaccgacagactcaaacctcactgcaccaaactacattcggactgtactcgaattcttgaaaagcattgtggacaacaacttcacccccctgctacacgaagaatctccggaaaatgaaagcaaaagtgaataa

SEQ ID NO: 11 - DNA, 3552 bp, synthetic construct
  source 1..3552: mol_type = other DNA
atgcctatgtcgacgattattgacaaatatatgccacttaatgactggaacagaatagagtcattgataggtgagttaagggcaatttccggggcgatgaattgtgcggtgcgcagagctgtttttgagaatatcaagaaagcaaaacttcaaatcaagttcaatgaccaataccctgaatccatttttaccgacaaaaatggatctatacccatagttggcactaccgaagcaaataatccggaaaatggtgggaataacgaatgtgagcaatcaaataattatttgagtatagattatctgccacgagtgacccaggaagataaaaagtcggtctatgggacttattttgaaatggcgtttcacaacttttttatcacattgcaccatatctactccctcattttcggtgaagacattatggaagtggcaaaaagtgaatactcccaaacacaaaccgattcttttcaagatgattttgccaataaatatactgtgtggaatcctctgttcacaagattaaggcgagccaaagctgagcagaaagagcgttttgaagagcttgcaataaagcattttcctttcctaaaagcactcgatgcgctcaaaggtgagaatcgggtttctaaggttgatgcgcttgagcggttttctgtagtcgttcgtgaattgagaaacatttatctgcactactgcatcatcccgagcgacaagcagaagaaggaatacagcgacaatatctctttcatcttcgatttaatggatctactgttcactggcgcaaagagggaggtgaagaccaggtttgctttaagcgacgaccaaatgagctgtgccgacaagtatgagccaaatagcgaccgctccctacgcgacattcacggcaaaacgttaagaatagttcccaagaaaaatttccggtatcatctatataaggttggtgacgacgcgaagataatctcgccatttggccttgtgtttcttgccagtctgtttcttgaaaaaaaatatgccaaaatattgtccgacaaggcacacgtcgttcgccttaatgacaagggtgtgatttgtgagatgatttcggtatatcgcattcgcctgcatatcaatagactaagcatctcaaaaagcacagataccttggcattggacattatcaacgaactgcaacgctgcccgaaaaaggtctttgagctgctgccgccagtcgcacagcagcgattcagggtgaagcctgaatcatcacacgcccccgaagtgctcatggttcgccacaacgaccgttttgttcatcttttgctgaaatatattgatgatgctaagctgtttgagcacattcgatttcaagtatctttaggccgttacttcttccggttctacgacaagatttgcatcgacacctcaagtgaaaagagggtgcgctccatctgcaaagatgtgcacggattcggacgtatttctgagattgaagagcttcgcagggaaaaatggaaagatattctgcgggaatatgatgaggtgcacgccaatactgccgacgagaagccctatatcaccgaccaccgagccaactacttgattggtaacaacaaggtgggaatctatctgctgaaggagggcgacgaacagtgcattatgcctgaactgttgcccaatggtgcccggaatcatgcgccaacttgctggctcagcacctacgagctgccggctcttgctttcttgctgcatctctacaatgcagatggagcaagggttgaggagattattgagaagcaggttgccggctaccgacgtctgtttgccgatgtgcgcgatggcagtgtcgcccctgtggcaagtgtggaggagcttgatgagttgctgaagggctacggtgatatgcaggcgtgcaatctgccgcgtaagatgctcgactatctgcttatgaaagatgtcaatgcacacgatttgttccgcaaatgggccgaagcggaattgcagcagatgattgagcagacagaccggctgtcgcagcgcatcgacgacgacattaaagccgcagccaatatgaggcaaaacaaattcggaaagaagtcttttgtggcagtgaagccgggtaaaatcgccgatttccttgcgcacgacatgatgctgtttcagccttgcaccgaggacaacagcaacaagctgactggccttaatttccgcatcttgcagtcggttatggctgtctacaatggtgacttcgatgaactgtcgagagtgctccgcaatgcccacatcattggcaacgcaaccgatgagatgtgcaatcccattgtaatggctgtatgccacaagagcatggaatttggcaatattgtagatttctacaaggcatatctccgtgagcgacgcatctatcttgagcggtgcttgcggcacggcgattttgagtctcttggatttcttcatgcctctcagatccgatggcaggaaagaagcaaggaatactatcgtgctttggctgcacgatacctcgtagatgaatacggcggaacagagtcggcaaaagccatcgaacttccgcgaggtttgtttgagccatatatccgcaaggaactatcggagatgaatgctatgaaatcattggcatgcaactccgactacaatgtttcatacctaatctatggctatttcaagagagttatgtccgatgatgctcagcctttctacgacgaaaagaaatgctatcgactcttcaatgtgctctatcgcaaatcgcctcacgactcgccggtctatcgcaatacggctgaaatacgcgatatgttgatgcagaatagcccgaactctatccgaaaggatattgaatcgtatctcagcaacaccattatagccgatagagccaaggagaaagagcgttgcacggcattgctcagggaaatgaagaagtgtgaaaccgagctgaaacgctacaagattcaggatatgctgctatttctgattgcaaagcgcattctgtctgacctaccggctgcacatgattcggctgttcaaatgcaggcaataagcaggattcatcttaaggacattaccgacggcaacactttgtcggagaagatttcactgagcgtgaaagtagtatcaaaaaacggatatattaagaagttgacacagcataacttgaaactgaagaactattctcagttttatgccattctcagcgaccgacgactgccgtcgttgctcgacttggttcgctctaattacatcaatcggaacgacatcgaagccgaactcgacaattacgacaaagttcacccggaagtgatgaaggcaattatcgggctcgagaagaaacacttcgaaaagcacggctttgacgattctggcatagttcctgatttaagcagcatccttgccgaaacgacaatgcccgcagacaaacaatatgaagtacgcaagattcgcaacagttttgctcattctcattatcctggttatcatgtcgcaaatgctggcataacagagttgcccaaaaaggctgaaaccatatttaacacattaaaaagtagcttgagcgatgaataa

SEQ ID NO: 12 - DNA, 3573 bp, synthetic construct
  source 1..3573: mol_type = other DNA
atggaaacaacgataaacaacagaatcgggaaaggtgaatactatacagaggaaagcaaggagtttcttgctgcctactttaatcaggccatacacaatgttttcattgtactaaatcatattgcgaaacgctttgggatggatgaattgtcttcggacgaagaactaaaaaactggttaattggacgacaacgtgaaaagaaacgaaatgcgattgatcgtcaacgcttcttagaattgattgatcggcattttccttttttacgcattgctaatgctgacaaaaaagacgcgaaaagagaaaacgatttagaagataatcttgccttactcataacgctattaaatgacttaactgaaagacgcaataagtatagtcatgcaattactcacgcaagcatagaaagtaatgatcgcgaattagtttggcgtttgtacagcatttatgatgccaatatcaacctcgttaaacgagattattttgaatccaatgtgcatacagaaatcaatgaagacccttatgaaaaacaagttgaacacttgcgccgattctgtatgaacaacgacagaaccaaagttgatgaaaaagggaaaaagaaacctgctatgccgaatccaagatttaggacaccctttttaaatgcggaaaccaatcaactgagtatttacggtttggtgttttttgtgtcgctttttttggaaaagaagtatgcaattcagatgcagaaaaatgtatatggtttaaaagatgctcgcgatacaaagtttaaaatgaccaatgaggtattttgcagaagtcggatcatcatgcctcgtgttcgcttgcacagcgataaatcaacggatgctcttgtattggatatgctcaatgaattggccaaagcaccagaggtgctattcgatcaactgacagacccttttaaagagaaattctatatcgagtcgatagatagccttgaagaatcagacattattactcctgtcagagcgattcgcaaacaaaataggtttatgtatttcgcacttcggtatttagatgaaagcaatgccttttctaaactacgcttccaaatagatcttggcaattatcattatcacctttatgaatctaaaataaacgatcaaactgaaagccgacatctaacgcgcaaactatttggttttgggaaactgatagcctttgaacaagaatttgcgcccgaagaatggaaaatgaaaagcaaagatttagattattatgaaggagcaacacagccctttattgcaaaaacgtacccacattatcatctcgaagaaaataaaatcggtattttatttaacggacaagcagaagtacaatggccacacttagatgtggaagaacatgaaagtttcccaaaatacaaacgtcgtgctaacgaaaaagcagatgcgtttctaagtgggaatgaattgttggcagcggcattctgtcatcatttgtatgcctccattggaaagcccaataccgtagaaaaaataatccgcgacaagtatcatgccttgcggcaattattttccgatttaaaatcaggaaacttacaaaacttgttaggcgataatacgagtaatgaagccatttctcaactgctttttgaaaaatataggcttacactatcagaagttcccgttcgactacatgcttttttgagtggacaagaacaagccgatacaaaagcaatagctagagggaaactagaactaatggcccaacaaaacaaaaaaagaattgaacggtttgatgcaatgaagaaagccgttgttaaggtaggcaaggctcaatatcgaacactccgttcaggggatattggggattggcttgtgcgtgattttatgcgttttcaaccaattggctataaacgcaatcaagcaggtaaacaagaaccagacttaaaaagcaaagcaaatcccaagaaatatcagttaatccaaaaaagtttagccctttacgaacaagagaaaaataacctcttgggtttatttaaaagttgcaacttattgtcatcagaaaacgaacatccatttcttaatgaagttgtgcagtcaatgccagcgacatggcaagatttctatgaacgttatctccatgcccgttctcgttttttggaaaaatgtatcgaaaaaggtattaagaaaaattcctaccaagcgtgttactcatttctaaaaataaaaccccaattaaaggataaggaaaaactatatcagggttgggatgctcaaatgaacttaccaacgaatatgtttattgatgccattcacgactggtttcgccaaacacaccatgaatcattacggacatggtttacacaacaagaaaaaccacatcaactcatcggacttattcgcaaatacattgaattagcacacaccgaccagatacaaggcttttatgatatgtttccgttgcgttacgacttttacaaaaaagaatttccaaatgggcttgttcttcacgagcggattaacaagcaaaaacaaatctgggaagctcaactcatacaaaccaaaaaacggttagaagatgcagcaagcaaattaaaaaaagtgaaacagcaagtcgaatcgttgcccgaccaagagcttcgatttcgcaatgaaacagaggcgatggtctattttaccaagttatttgactcaagcattgtcaagaatgcaattctcaaactgcaaagagatcagaaagcacttcgtgtaaatacaattggagaaaaaattatcaagatttatacagcaaaatacgatgccattcatcaagaggtacgagactttaaatccatgctgacaactgaaaaaatgattcgtcgggttaaggcagaggattgtgtaacgctatttatgctgaccgatttgatgaatcaaagtcaaatcacgattggacaagaacagcgaactattaaactcagcgatattcaacctatgggcgaaacgcaaattcaaggcattcttgatgcagttcaggtattggagcaaaaattagattttttttccagtgatgaacaaggaaaaataagtcaggttaagctgggcgaatggacgattttttcaactgatacaaaagtaaagaagcaaggaaattttaaacaattgttaaaagatcgccgcctcaacaacctagcacactatattttgccagatatagcaggaggagcgattcgagtacgacgcaatttgttggagatggagttagatcaatacgaccgtaatcgcattcctattattaaactgatgtatgaactcgaatatgcgatctataaggttgatccattttcagtagaactaaaatataaaaagtttagccaatgcttgcgtgaatatgctcaaaaagcagttttgaatgttgaacaagtggaacatttgaatgtgttgattgccatacgcaatgccattatgcacaaccaatatcccaatcgagaccatttaaaagctatcgtgccatttacggtaagcgaatatgcgccagttcaagaaggattaaccattgcgcggcagcttctagcatgtgcgcaagtgagcgtcaacattattttatccaccatctcaaaatttgaataa

SEQ ID NO: 13 - DNA, 3477 bp, synthetic construct
  source 1..3477: mol_type = other DNA
atgaaagagaaaatcaaaaataaaagttccataatcagaataataatgtcaaactatgatgacaaaggcttgaaagaattcaaagttttatataataagcaaggtggagtagatacttttacttgcaaaactgatattgttgatggaactattatttttttagaaattgaaaaacatttaagagattttggagacgatttttcgtgggatatttcaagtgatggtaaatcagttgagattacaaaacttataaatggaaaagaaacaagaaagtacaaagtaagtattaaaaattcaagtacaaaagataaaaagaatttagttgaattagaggtcgaggacttaaaagaaagtgcaatagatagaaggaggactaaaagtagtacaaaaagagttttgctttctaaagatgtaatggaaagatatgcagaaattgcttttagtaaaaaagaacgttgggaagagatagattctcaaaaaatttataaagtcaaaagatttttagattatcgttctaatatgcttatatattttcagtttattaatgattttttgactaaagggatacctgatgaattagataaaaatggagaaataaaacagttggaactttggaaacttatagatgatgatgaaactatatctgataaaaacttaaatcaagtctccaagaatttatatacttatatttctcaagaaattaaagatagtcaaactagagctgaaaataacagagaaaaaaataaagaaaaagagcattttaaagaattttatgcatttaatgatatttctgaagaaagcataagagaggacgttaaaaaattcatatatttatacgctaatttaagacataatttaatgcattataattactctttttttgaaaatctttttgagggtaaagatcttgttattgaaaaaactaaaagtctgttgagttctactttagatttaaatatttttaaggaactttcaaacatagtagagttgagagaagagaataaaacaaactatcttgatgatgaaacaactataagagttcttggaaaagaaaaaaaagcaaaaactttgcataaaatttatagtattctttgtagtagaaaaaatggttttaacaagtttattaactcatttttttctacagatggtatagaggaagagtttttaaaatcagagataaaaaaagattttttagaaaggttaaattgggttgaaaagtcattaattgaaaaaataaacaatccaccaagtgatacaaagttaaaatataaaaatgacaaaactatagaaaatatgaccaaagaaaaggaggaaaaattagagttaatctctcttttgaatccacaagttagcgattataagaccgagaattttactccatattattgggacatacatcagagcccttcatacaagaaactatataatgatagaaaagttttagtttcggaactttcaaaactaatagccattggtataaatagtgataccaagaaaagaataactgatttaaatgctgaacttttaaagattaagataaaaatggaaaaaattactaagcttaactcaaaaataagacttcaatataagttacaaatggcatttggtttcatttatgccaattattcaaaagtatacaaagaaaaaagagtacttaatataaatggatttgtgcaaaactttgacccgacaaaactaaataaagagaaagaattagaatcaaggttaatttatttaaaagctccttataatatatttgaagacaataagtctttagatttcaatatgaaaattgtagaaaacattccagtttcagaaaaatcaatctttagaataaaaccagagaataatctttccaagttttatattctatcttatttacttctacctgtagaacttaggggagattttttaggatatgttaaacatcattactatgggataaaaaatgtagattttgaagaaatacctgatattaaagaagataagcctaatgaaaattctgatagctttttccataatttgagactttttgaaaaaaatagtaaaaaatttgaattaataaaatatagattagtggaatttggtaatttgaaagaccatcttccaagaatttatgaaaaatttggaatcaaaccagatgttttagaatatatcgaaaattcagggaataaggattccaaactttttgatagaaacatactgttgcctattatgaagtattatcaacatatttttaaacttcttaatgatattgaggttcatgctttgttaagattttcggagaaagattctatatctcttgatgaaagcataaaagaatgtagtaaggggaaattcctaaattttggaaagcttctgtttttatctagatatggattagaagcgaaaaaagataataagtttaaagatatttttaatcgagagaatggattatcaataacaaaagatgatgctaaaactgaaagaaagaaatattttgaaatatttgaaacaagaaacaaaatagctcacttaaactacaaacagcttttccatgacttattatttgatagtaatatcaatataaacaaggaattagaaggaattattcaagaaactaaaactatcgggcttaatgctcaaactttaggttacaacttcttaaatgacttttatatgagaaaagagatgtttataagtaatcagaaaaagtcctcaatgactctaataaataaccctttatctaaagataaagataccaaagaaataggactcttaaaattatatggtttatcaaagtctcaacctaaagatttaattttagctaaatataaagaacttatgaatttaattgaaaaaacagaggattctattcttaagaaaaaagattttttacctgtgaaagaagtttctattacagttaaaaaatccacgccaaataaaaaaggaataatggttgaacttccagaaatacttcaaataaaggatttaaatgaaatggatttacttgcttatgcttcaaatattagaggtaaacttcataaagattcttccgacctttttggaatctataaaaaattaactataaaagagttgaaaaagaaacttataaatctttttataaaaggagaaaaaaggtatctcaacctagaacttgtaaacaagactggttatatggcaatatatgaatctacaggtttatatcctaaatcttatgaaatattaaatcacgaaatctcttttagtgaaattagtatgaaaaattggtatgaacatgattttaaacctatattccaaattgatggaagtctaccaaataatacagattataaaaatggtgtgtttatttacacaagtccctacgaatttagagataaagagcttatgaaaaaacagagaactgtacacaaaagagatatagaaaaaacattttataatgaaaacgatatggattacacaggtatctacaatcaaaaaataaaagctctctattga

SEQ ID NO: 14 - DNA, 2796 bp, synthetic construct
  source 1..2796: mol_type = other DNA
atgatggggaataaaaagtcggttgcaaaagccaacggcttaaaatctactttcgttttgggcgaaaatacggcgtatatgacttcgttcggcaggggaaatgcggcacagccggaaaaacatatccgcgacgctacggtgacggatattcaacatactttccgtgcaaaaaccgacgggggcagaacggtgcatatcgaaggcagagtcggggcgtccgatgtgttgctgccggatgccgctaaccaactgcacgccaaagatgccgttgagcaaatgtatttcggcaaagcgttttcggacaatatccacatccaaatcgcctacaacattatggacattaaaaagattttcggtgtgtatgccaatatcatagtgcataccgtcaacaatctttgctgtgacggagacaagcaggacgatttcctcggtatgtttaaaacgcaaaatcggtatcaagttgcggcgtgggcacataaaattgtttcgttgcatttggtgaaaaacgagttgcgcggcggcggattttttatggaccaagaggtttggcgtgcacatgtcagaacggatttcaagtccttgaatcttgcggtgaatgcttttatgaaaaagtatccccaaaaatatccgtattggagtgtgaaaattgtatctgactttatcgtgcaggaaatgggcataaagaataaagtcattttggaaaaagcggccgagagttatgcggaatttgaaactgtcgccaaacgccttgaaaaatccgcttattatttttcggacatatttgccggcaaagacggtaaatttgatgaacaaaaggcctttgatttattgcgcgttttgggtatgatgcggcaagaagccttccacgaaaaaaacagttctgcttcttggctgtacaatttggacgcggaagccgacgaggacatcaaagccgcgctgagaaccgttgtcgataccaaagtaaacggtatcaatacgaattttgccaaacaaaataaggtaaaccttcttgttttgcaggaaatttacccgcaaaaaagcaaggcggacttggtgcgcgagtattatgacttttcggtgcgcaaggcgtttaaaaatctcggtttttccgtgaaaactttacgcgaaacgatgtgtgcatttgatgcggcttctgtaatcaccgacaagcaatatgacactgtgcgcggaaaactgtatagtttgtttgattttgtgatttacaattattgcttggaaaacgaggcggtttgcaatgcctttgttgaagaattgcgcgccaatttggacccggaaaacaaaacggctttgtaccaaacccttgccgagaaagtttgggcggaaatcggcgacattgtgctgcagcgaattttgccgcagatgcatgcgaaaaaaattcaagagagatccaaagaaaccgatgccgaaacggttgaaatgcaagggtatgtgcaggcgccgaaggacttgtcgctgttttcaaaggcggtgtattgtatttccatgtttttggacggcaaggaaatcaacagttttttaagcgcgttgattaacaagtttgaaaatatttcttccttgtgtgcagtactggcgtataacggattggaaccggaatttgtcgcgccctttacattttttgccgacagtcaagccattgccgaggatttgcggtatatcaaatccattgcccgtatgagcaaaggcaaaaaagcaacgaaagacagccccgttaccgtgaaagaaatgcaatatttcgatgctgccgccgtgttgggcgaaacggacacggaaaaagtgaaagcggcatttcacttgggtgacaagtcggcttccacggcggacaaggcgttccgaaatttcgtggtgaataatgtaatcaattccaaccgttttgtgtatgtggttcgctttattaacccgaaaaatgcacgcgaaattatgcaaaaccgtgcgctgattgcgtttgtgttgaaagatattccgcaaagccagttggtgcgctattgcggtacggcggggattgcctgtaacgcggacgagccgaataccgaagccatggtaaatgcgcttgcagatatgctgttgcaggtgcggtttgatgctttcagtaatgtgcaacaaaaggtcaaggcggattctgcagaggctgtgcaaaaggagaaatacaaagcgattatcgggttgtatttgactgtgctgtatttactggtaaaaacacttgtaaaaatcaatatgaattatgccattgcattcgggattttggagcgtgactgtcaaattatgaaccaaaagcacggcaaaaatccgaaacgcgaccgcgacgcattttatatgcgcgaacagcaaaacaagcagtatgtttataacgcacgcgccattacagaattgtttatagaaaacggatggctgaataagcgcgtgcaaaaaagcgtggaaaataacgccgcactgtattcggacgaagcgttttataaatacagaaatcttgtggcgcatttgaatgtgatttccgcacttccgaaatacgcaaaaaacattaccaaggtgaaatctttgttcgatgtgtatcattacattttgttcttgtcgctttgcgaggataaatacagcaatctgcccgaagcggtgacgaaatccctttgcaaaaacggtaaaacgatgttggaaaacgcgcgggaataccaaacggtttgcaaagattttctgtatgggttgaacacgccgtttgcgtataacgccgcgcggtatatcaacctttccaaccgtgaaaagttcctggcggggtttgggaagtaa

SEQ ID NO: 15 - RNA, 36 nt, synthetic construct
  source 1..36: mol_type = other RNA
gttgttacagcccttagtttgtagggtaatgacaac

SEQ ID NO: 16 - RNA, 36 nt, synthetic construct
  source 1..36: mol_type = other RNA
gttgtagatgacctcgttttggaggggaaacacaac

SEQ ID NO: 17 - RNA, 36 nt, synthetic construct
  source 1..36: mol_type = other RNA
gttgtagaagccgttcattcgggacggtatgacaac

SEQ ID NO: 18 - RNA, 36 nt, synthetic construct
  source 1..36: mol_type = other RNA
gttgtaaatacccacgttttggtgggctaatacaac

SEQ ID NO: 19 - RNA, 36 nt, synthetic construct
  source 1..36: mol_type = other RNA
gttgtgtgtgcctttcaaattgaaggcgttcccaac

SEQ ID NO: 20 - RNA, 31 nt, synthetic construct
  source 1..31: mol_type = other RNA
atgactataccagcaatggctggattaaaac

SEQ ID NO: 21 - RNA, 37 nt, synthetic construct
  source 1..37: mol_type = other RNA
ggttttacacccgtgtaaaactacacagttctaaaac

SEQ ID NO: 22 - protein, 1114 aa, synthetic construct
MGSSHHHHHHSSGLVPRGSHMASMTGGQQMGRGSPAAKKKKLDGSVDMNPQARTRKPETPLKPVGNEHFAVFINIARHNAFIAITELSKIYGMTPPNEDELATSRFIAAFDSTTIDVRKLKQRLKRLSSLMPFLKSLQDKTDAEIIGILKDLLSLVNQFRNYYSHYNTSDFLTINSNEFITSDKVSILENIFEKAVLSLTNSEKAYDRFEIISLLKSEKRADKPYFYEFIENNKISEKAIAFFFCLFLDKPNAMKFLKRLKGFKGADTKQFRATLEAYTTYCIQLPEPKFLSDRPNLAIILDGIEHLKRCPIEVHKTLSFRDKQKFERKVMREDLNGDLQEENIELLRYDDRFAEFAMRYLDDFDILSDAKKQNTYRFEIQLGKKVVESKKLAEETTEAQDKIPVRFKPVKAFGKLADIPRKKDEAVIDWQQDLEELYAYEPHYKIENHSIGIKKIATEDTFRLNNPEELPDAYLSEYQLRNIIFLSLESSNKEEFFMACQIRIGKIKSLYKALSAPTHYKESIKQKYNELINNNLLPKPLVKYLTHSLDELPTYKSKAIKKLKFWQDETENLLAEVKRHNEKSEKARKENKFFKSFLKSGQIATWLIKDIQHFLPLQGKLSVLKYNALQAKLAIYNSEELKEMLTDFQVYDTPKGTDRNMPEKGGGHQFIKTVFDKNPQKLPPHWLHFYNDYLNAKKQWIEDKIKFLTAMPDTEAEIMKQQPLFYFLDLGSNYEEGEKIVYFRENSPAYIAKYCEELLKKPVDLPIALSYDLVANMRTGLEKAKSVTDFIDDKYQSEPPYYHLPRQYDLFKAFGDKPSEKLFATDKKPLHEVYGEYKAKKTDPRTIKKIKGFLDQEQRIRYLKVCDKLLVKILEKYLAKETELKNVQLTDAQGKLILDKVLETEFEMPPYGFKVRLKDYGRYRRFVKDRRLVSMQDYLNQSVFTPDTLITELNLYEKQRSEFLKIVLEFEKRLLSASDTLNINLADQQTTLGEDKIRDYITHNYLLEVALRNNFISENEARAMLWFRNGALHNQLPDLQKLVGLIDTEEQKTQRYFLKGMEMYKKGIEKISTGGGPGGGAAAGSGSPKKKRKVGSGSKRPAATKKAGQAKKKK

SEQ ID NO: 23 - protein, 1281 aa, synthetic construct
MGSSHHHHHHSSGLVPRGSHMASMTGGQQMGRGSPAAKKKKLDGSVDMTILEKYMPLNEMGKIKSLVDELKGIPGAMNATLRQEIFQNIKKTKLQVKFLEEYPETLFTDSGNLIPIIGNNDNSSSGTPSKQEVSDIDANQASRINYLPHETMGEIKSVYGTYIEMAFHNFYLTMHHIYAVVFGEDIMEEAKKEFDKNNTNSTKYFTFDFANERTIWKPMFDRAERAKPEQKEHFEKLVVKHFPFLKAIDALEDRKRKTKIQALCVFSLVLRELRNVYSHYLFYPFKNQVDKYKENIPFVLDMMEILYTGAQREVKGRFGFDDKKMQCAKKYERNKDHSQRDHQGKIIKAVPKKNFRYNLYKKEDSEAIITPFGLVFLTSLFLEKKYAKILSDKTHCIKYTDQEVLCEIISVYRIRLHIQKLSVTKDTDALALDIINELQRCPKRLFEMLSPDDQQKFRIKPTDSQYADDVLMIRHQDRFAHLLLKYIDDAHLFNCIRFQVSLGRYFFRFYDKSCIDSTGDKRVRSISKNVNGFGRITDIEDYRKEVYGDMIREYEDVHANTSMEKPYITDHHAKYLISNNRIGLYIRKEEDTQCLLPELTPDGARNFAPTCWLSIYELPALAFLLHLYNGDGSRVEEIIQTKVANYQRLFADVRDGKVCPVKDEAELTTILQTYGNIEPSQLPRKLLDYLLKKEICAQDLFNTWAQSKIQRMIAQTDSLLQHLEKDLQAVSDLKQNKFGKKAFVAIKPGHIADFLAHDMMFFQPSMKDCNNKLTGLNFRILQSSMAVYDGNFDELSRIMRSAHIIGNANDACCNPIVMAVCRKHKGFSNIIRFYQAYLKERKAYLQQCANERHYDSLSFLHASQNKWRERTQAYYRSLAAKYLAENYDGVDTTKSIELPRGLFETYIRQELSEIGSTKSMAGDATKNTSYLIYGYFRQVMSDDAQTFYDTRRCYQLFDVLYRKSPRDNHSYYSTAQIREMLMRSHSKSIRKDIDNYISQTTAAERTKEKERCDALLRKIKDTETELKVYKIQDILLFLIAKRLLLDRKVENDSAVQMNAINQIRLRNIADGNTLSQKIPISISIKSRKGDPKIIQQDDLKLKNYSQFYSIISDRRLPSLLDLINSRVIKRTDIEDELSNYDKSHPHVLKSVFEFEKHYFDTHPIPSDTAYMALPDTGEMLKESNLTAEKQKEVRKIRNSFAHLSYPSRNITGAASTELPKKAEIISKNLIEHLSNAEIKTGGGPGGGAAAGSGSPKKKRKVGSGSKRPAATKKAGQAKKKK

SEQ ID NO: 24 - protein, 1361 aa, synthetic construct
MGSSHHHHHHSSGLVPRGSHMASMTGGQQMGRGSPAAKKKKLDGSVDMYHLSDANHGKHIAGTYYEMAMGNFIHTLSHMLVRAGIKVNKLEDNYSIEREIMNLTAPGAYDAQRAALSRLLYRHFPFFGPIMADHTDHILSSKRKKVQSASDDGNLDLGQELKDEVAGASACQMIRYLATIAGALVYYRNMYSHKNHYDNAQDIAAQQEREQKLALWLDVVFRGARDILLTRKSHPQPDTDFLTQNGTINYYIEKNGKSAYNPNFYFKPGLKTDNGWVMTDFGKFFFCSLFLRRADAERFAAETDLYVGSPFKITAQERARLQEAENKRAADEQARASSAGFPHIVNPRTIGPSESPQNNIIREMLNMHRARIPRERRIDADMSEGILAMDIMNELRRCPLSLYNTLSPEAKASFEKTGVTPEGGIVSNLLVRHSDRYPELALRAIDQMELLPTIRFHVRLGSLRFRFYEKKLIDGSHTLRTVQKAVNGFGRWQEVEPRRVEKYTAIQARCQNDKGIDQFLPDSPTTTPYITDWRTTYNIHANRIGLAWNLPQMSDGIYLPNLDTDKGDNLHRKALIDMPAPMCYLSIFDLPALLFYCHIYTHYHGTKYHLPSAESIIQAKYDALHKFFSFAAAQNHSAEQLREKQLELNLADNEIPDKLRCMMQTKPFFKNGRQQLSPLGYPIMKNWIGVAEQRKHAAQVLRDVANEAADRLASFEKKHQRVVVGGRDNRYGRRGHADIRHGSLARYLATSMVRWQPALDQPGGDKLTSANHRALAGFLSEYGLHGSNINKLRNVLKEAGLIEGSHPHPFLAHVLESAPANIEALYVAYLKHEQSHATALKNKFTDRNGIVQPSEVPAFVRFNSSRWRNDSATTARRYLQTPPAPGSSDSAEHNAPIMLPDGLFTTHIMTLLNKVLGQNDRVPEEDYLRHDLPRIASIINPNGKTYGAAYIIRAWFDQVENQDVQPFYDLPRFYREISLLAPRRKPNQELIRDYFSEEQIAQKIQTVPKKQRSEKVGHTIDTEKDIRRYRLQDITLYLTLLDMLTLMLSRNEAERTDRQMKSSTAERVSNMRLVDFDHSFDFDLLGSTSGEAAYSYLHQRSGITISMPALSLRSYGSIFRVLADSRFETLMDALNRQGVTHVNFGDITSELALYDTLRSHFLLQAHNVEQDAFSAKRGVLENHTSPFFYRSGNLQLDDQGNITNPSTDAIRNHYGELIKILDRYSLKIDKKTKDGKSQDILLRDLMAELRNAAAHNRYPKADFFFRQFDHFLNTCKPTDSNLTAPNYIRTVLEFLKSIVDNNFTPLLHEESPENESKSETGGGPGGGAAAGSGSPKKKRKVGSGSKRPAATKKAGQAKKKK

SEQ ID NO: 25 - protein, 1272 aa, synthetic construct
MGSSHHHHHHSSGLVPRGSHMASMTGGQQMGRGSPAAKKKKLDGSVDMPMSTIIDKYMPLNDWNRIESLIGELRAISGAMNCAVRRAVFENIKKAKLQIKFNDQYPESIFTDKNGSIPIVGTTEANNPENGGNNECEQSNNYLSIDYLPRVTQEDKKSVYGTYFEMAFHNFFITLHHIYSLIFGEDIMEVAKSEYSQTQTDSFQDDFANKYTVWNPLFTRLRRAKAEQKERFEELAIKHFPFLKALDALKGENRVSKVDALERFSVVVRELRNIYLHYCIIPSDKQKKEYSDNISFIFDLMDLLFTGAKREVKTRFALSDDQMSCADKYEPNSDRSLRDIHGKTLRIVPKKNFRYHLYKVGDDAKIISPFGLVFLASLFLEKKYAKILSDKAHVVRLNDKGVICEMISVYRIRLHINRLSISKSTDTLALDIINELQRCPKKVFELLPPVAQQRFRVKPESSHAPEVLMVRHNDRFVHLLLKYIDDAKLFEHIRFQVSLGRYFFRFYDKICIDTSSEKRVRSICKDVHGFGRISEIEELRREKWKDILREYDEVHANTADEKPYITDHRANYLIGNNKVGIYLLKEGDEQCIMPELLPNGARNHAPTCWLSTYELPALAFLLHLYNADGARVEEIIEKQVAGYRRLFADVRDGSVAPVASVEELDELLKGYGDMQACNLPRKMLDYLLMKDVNAHDLFRKWAEAELQQMIEQTDRLSQRIDDDIKAAANMRQNKFGKKSFVAVKPGKIADFLAHDMMLFQPCTEDNSNKLTGLNFRILQSVMAVYNGDFDELSRVLRNAHIIGNATDEMCNPIVMAVCHKSMEFGNIVDFYKAYLRERRIYLERCLRHGDFESLGFLHASQIRWQERSKEYYRALAARYLVDEYGGTESAKAIELPRGLFEPYIRKELSEMNAMKSLACNSDYNVSYLIYGYFKRVMSDDAQPFYDEKKCYRLFNVLYRKSPHDSPVYRNTAEIRDMLMQNSPNSIRKDIESYLSNTIIADRAKEKERCTALLREMKKCETELKRYKIQDMLLFLIAKRILSDLPAAHDSAVQMQAISRIHLKDITDGNTLSEKISLSVKVVSKNGYIKKLTQHNLKLKNYSQFYAILSDRRLPSLLDLVRSNYINRNDIEAELDNYDKVHPEVMKAIIGLEKKHFEKHGFDDSGIVPDLSSILAETTMPADKQYEVRKIRNSFAHSHYPGYHVANAGITELPKKAETIFNTLKSSLSDETGGGPGGGAAAGSGSPKKKRKVGSGSKRPAATKKAGQAKKKK

SEQ ID NO: 26 - protein, 1279 aa, synthetic construct
MGSSHHHHHHSSGLVPRGSHMASMTGGQQMGRGSPAAKKKKLDGSVDMETTINNRIGKGEYYTEESKEFLAAYFNQAIHNVFIVLNHIAKRFGMDELSSDEELKNWLIGRQREKKRNAIDRQRFLELIDRHFPFLRIANADKKDAKRENDLEDNLALLITLLNDLTERRNKYSHAITHASIESNDRELVWRLYSIYDANINLVKRDYFESNVHTEINEDPYEKQVEHLRRFCMNNDRTKVDEKGKKKPAMPNPRFRTPFLNAETNQLSIYGLVFFVSLFLEKKYAIQMQKNVYGLKDARDTKFKMTNEVFCRSRIIMPRVRLHSDKSTDALVLDMLNELAKAPEVLFDQLTDPFKEKFYIESIDSLEESDIITPVRAIRKQNRFMYFALRYLDESNAFSKLRFQIDLGNYHYHLYESKINDQTESRHLTRKLFGFGKLIAFEQEFAPEEWKMKSKDLDYYEGATQPFIAKTYPHYHLEENKIGILFNGQAEVQWPHLDVEEHESFPKYKRRANEKADAFLSGNELLAAAFCHHLYASIGKPNTVEKIIRDKYHALRQLFSDLKSGNLQNLLGDNTSNEAISQLLFEKYRLTLSEVPVRLHAFLSGQEQADTKAIARGKLELMAQQNKKRIERFDAMKKAVVKVGKAQYRTLRSGDIGDWLVRDFMRFQPIGYKRNQAGKQEPDLKSKANPKKYQLIQKSLALYEQEKNNLLGLFKSCNLLSSENEHPFLNEVVQSMPATWQDFYERYLHARSRFLEKCIEKGIKKNSYQACYSFLKIKPQLKDKEKLYQGWDAQMNLPTNMFIDAIHDWFRQTHHESLRTWFTQQEKPHQLIGLIRKYIELAHTDQIQGFYDMFPLRYDFYKKEFPNGLVLHERINKQKQIWEAQLIQTKKRLEDAASKLKKVKQQVESLPDQELRFRNETEAMVYFTKLFDSSIVKNAILKLQRDQKALRVNTIGEKIIKIYTAKYDAIHQEVRDFKSMLTTEKMIRRVKAEDCVTLFMLTDLMNQSQITIGQEQRTIKLSDIQPMGETQIQGILDAVQVLEQKLDFFSSDEQGKISQVKLGEWTIFSTDTKVKKQGNFKQLLKDRRLNNLAHYILPDIAGGAIRVRRNLLEMELDQYDRNRIPIIKLMYELEYAIYKVDPFSVELKYKKFSQCLREYAQKAVLNVEQVEHLNVLIAIRNAIMHNQYPNRDHLKAIVPFTVSEYAPVQEGLTIARQLLACAQVSVNIILSTISKFETGGGPGGGAAAGSGSPKKKRKVGSGSKRPAATKKAGQAKKKK

SEQ ID NO: 27 - protein, 1247 aa, synthetic construct
MGSSHHHHHHSSGLVPRGSHMASMTGGQQMGRGSPAAKKKKLDGSVDMKEKIKNKSSIIRIIMSNYDDKGLKEFKVLYNKQGGVDTFTCKTDIVDGTIIFLEIEKHLRDFGDDFSWDISSDGKSVEITKLINGKETRKYKVSIKNSSTKDKKNLVELEVEDLKESAIDRRRTKSSTKRVLLSKDVMERYAEIAFSKKERWEEIDSQKIYKVKRFLDYRSNMLIYFQFINDFLTKGIPDELDKNGEIKQLELWKLIDDDETISDKNLNQVSKNLYTYISQEIKDSQTRAENNREKNKEKEHFKEFYAFNDISEESIREDVKKFIYLYANLRHNLMHYNYSFFENLFEGKDLVIEKTKSLLSSTLDLNIFKELSNIVELREENKTNYLDDETTIRVLGKEKKAKTLHKIYSILCSRKNGFNKFINSFFSTDGIEEEFLKSEIKKDFLERLNWVEKSLIEKINNPPSDTKLKYKNDKTIENMTKEKEEKLELISLLNPQVSDYKTENFTPYYWDIHQSPSYKKLYNDRKVLVSELSKLIAIGINSDTKKRITDLNAELLKIKIKMEKITKLNSKIRLQYKLQMAFGFIYANYSKVYKEKRVLNINGFVQNFDPTKLNKEKELESRLIYLKAPYNIFEDNKSLDFNMKIVENIPVSEKSIFRIKPENNLSKFYILSYLLLPVELRGDFLGYVKHHYYGIKNVDFEEIPDIKEDKPNENSDSFFHNLRLFEKNSKKFELIKYRLVEFGNLKDHLPRIYEKFGIKPDVLEYIENSGNKDSKLFDRNILLPIMKYYQHIFKLLNDIEVHALLRFSEKDSISLDESIKECSKGKFLNFGKLLFLSRYGLEAKKDNKFKDIFNRENGLSITKDDAKTERKKYFEIFETRNKIAHLNYKQLFHDLLFDSNININKELEGIIQETKTIGLNAQTLGYNFLNDFYMRKEMFISNQKKSSMTLINNPLSKDKDTKEIGLLKLYGLSKSQPKDLILAKYKELMNLIEKTEDSILKKKDFLPVKEVSITVKKSTPNKKGIMVELPEILQIKDLNEMDLLAYASNIRGKLHKDSSDLFGIYKKLTIKELKKKLINLFIKGEKRYLNLELVNKTGYMAIYESTGLYPKSYEILNHEISFSEISMKNWYEHDFKPIFQIDGSLPNNTDYKNGVFIYTSPYEFRDKELMKKQRTVHKRDIEKTFYNENDMDYTGIYNQKIKALYTGGGPGGGAAAGSGSPKKKRKVGSGSKRPAATKKAGQAKKKK

SEQ ID NO: 28 - protein, 1020 aa, synthetic construct
MGSSHHHHHHSSGLVPRGSHMASMTGGQQMGRGSPAAKKKKLDGSVDMMGNKKSVAKANGLKSTFVLGENTAYMTSFGRGNAAQPEKHIRDATVTDIQHTFRAKTDGGRTVHIEGRVGASDVLLPDAANQLHAKDAVEQMYFGKAFSDNIHIQIAYNIMDIKKIFGVYANIIVHTVNNLCCDGDKQDDFLGMFKTQNRYQVAAWAHKIVSLHLVKNELRGGGFFMDQEVWRAHVRTDFKSLNLAVNAFMKKYPQKYPYWSVKIVSDFIVQEMGIKNKVILEKAAESYAEFETVAKRLEKSAYYFSDIFAGKDGKFDEQKAFDLLRVLGMMRQEAFHEKNSSASWLYNLDAEADEDIKAALRTVVDTKVNGINTNFAKQNKVNLLVLQEIYPQKSKADLVREYYDFSVRKAFKNLGFSVKTLRETMCAFDAASVITDKQYDTVRGKLYSLFDFVIYNYCLENEAVCNAFVEELRANLDPENKTALYQTLAEKVWAEIGDIVLQRILPQMHAKKIQERSKETDAETVEMQGYVQAPKDLSLFSKAVYCISMFLDGKEINSFLSALINKFENISSLCAVLAYNGLEPEFVAPFTFFADSQAIAEDLRYIKSIARMSKGKKATKDSPVTVKEMQYFDAAAVLGETDTEKVKAAFHLGDKSASTADKAFRNFVVNNVINSNRFVYVVRFINPKNAREIMQNRALIAFVLKDIPQSQLVRYCGTAGIACNADEPNTEAMVNALADMLLQVRFDAFSNVQQKVKADSAEAVQKEKYKAIIGLYLTVLYLLVKTLVKINMNYAIAFGILERDCQIMNQKHGKNPKRDRDAFYMREQQNKQYVYNARAITELFIENGWLNKRVQKSVENNAALYSDEAFYKYRNLVAHLNVISALPKYAKNITKVKSLFDVYHYILFLSLCEDKYSNLPEAVTKSLCKNGKTMLENAREYQTVCKDFLYGLNTPFAYNAARYINLSNREKFLAGFGKTGGGPGGGAAAGSGSPKKKRKVGSGSKRPAATKKAGQAKKKK

SEQ ID NO: 29 - DNA, 720 bp, synthetic construct
  source 1..720: mol_type = other DNA
atggtgagcaagggcgaggagctgttcaccggggtggtgcccatcctggtcgagctggacggcgacgtaaacggccacaagttcagcgtgtccggcgagggcgagggcgatgccacctacggcaagctgaccctgaagttcatctgcaccaccggcaagctgcccgtgccctggcccaccctcgtgaccaccctgacctacggcgtgcagtgcttcagccgctaccccgaccacatgaagcagcacgacttcttcaagtccgccatgcccgaaggctacgtccaggagcgcaccatcttcttcaaggacgacggcaactacaagacccgcgccgaggtgaagttcgagggcgacaccctggtgaaccgcatcgagctgaagggcatcgacttcaaggaggacggcaacatcctggggcacaagctggagtacaactacaacagccacaacgtctatatcatggccgacaagcagaagaacggcatcaaggtgaacttcaagatccgccacaacatcgaggacggcagcgtgcagctcgccgaccactaccagcagaacacccccatcggcgacggccccgtgctgctgcccgacaaccactacctgagcacccagtccgccctgagcaaagaccccaacgagaagcgcgatcacatggtcctgctggagttcgtgaccgccgccgggatcactctcggcatggacgagctgtacaagtaa

SEQ ID NO: 30 - DNA, 30 bp, synthetic construct
  source 1..30: mol_type = other DNA
tgccgttcttctgcttgtcggccatgatat

SEQ ID NO: 31 - DNA, 4828 bp, synthetic construct
  source 1..4828: mol_type = other DNA
cctgcaggcagctgcgcgctcgctcgctcactgaggccgcccgggcgtcgggcgacctttggtcgcccggcctcagtgagcgagcgagcgcgcagagagggagtggccaactccatcactaggggttcctgcggcctctagactcgaggcgttgacattgattattgactagttattaatagtaatcaattacggggtcattagttcatagcccatatatggagttccgcgttacataacttacggtaaatggcccgcctggctgaccgcccaacgacccccgcccattgacgtcaataatgacgtatgttcccatagtaacgccaatagggactttccattgacgtcaatgggtggagtatttacggtaaactgcccacttggcagtacatcaagtgtatcatatgccaagtacgccccctattgacgtcaatgacggtaaatggcccgcctggcattatgcccagtacatgaccttatgggactttcctacttggcagtacatctacgtattagtcatcgctattaccatggtgatgcggttttggcagtacatcaatgggcgtggatagcggtttgactcacggggatttccaagtctccaccccattgacgtcaatgggagtttgttttggcaccaaaatcaacgggactttccaaaatgtcgtaacaactccgccccattgacgcaaatgggcggtaggcgtgtacggtgggaggtctatataagcagagctctctggctaactaccggtgccaccatggtgagcaagggcgaggagctgttcaccggggtggtgcccatcctggtcgagctggacggcgacgtaaacggccacaagttcagcgtgtccggcgagggcgagggcgatgccacctacggcaagctgaccctgaagttcatctgcaccaccggcaagctgcccgtgccctggcccaccctcgtgaccaccctgacctacggcgtgcagtgcttcagccgctaccccgaccacatgaagcagcacgacttcttcaagtccgccatgcccgaaggctacgtccaggagcgcaccatcttcttcaaggacgacggcaactacaagacccgcgccgaggtgaagttcgagggcgacaccctggtgaaccgcatcgagctgaagggcatcgacttcaaggaggacggcaacatcctggggcacaagctggagtacaactacaacagccacaacgtctatatcatggccgacaagcagaagaacggcatcaaggtgaacttcaagatccgccacaacatcgaggacggcagcgtgcagctcgccgaccactaccagcagaacacccccatcggcgacggccccgtgctgctgcccgacaaccactacctgagcacccagtccgccctgagcaaagaccccaacgagaagcgcgatcacatggtcctgctggagttcgtgaccgccgccgggatcactctcggcatggacgagctgtacaagtaaagcggccgaattcctagagctcgctgatcagcctcgactgtgccttctagttgccagccatctgttgtttgcccctcccccgtgccttccttgaccctggaaggtgccactcccactgtcctttcctaataaaatgaggaaattgcatcgcattgtctgagtaggtgtcattctattctggggggtggggtggggcaggacagcaagggggaggattgggaagagaatagcaggcatgctggggaggtaccgagggcctatttcccatgattccttcatatttgcatatacgatacaaggctgttagagagataattggaattaatttgactgtaaacacaaagatattagtacaaaatacgtgacgtagaaagtaataatttcttgggtagtttgcagttttaaaattatgttttaaaatggactatcatatgcttaccgtaacttgaaagtatttcgatttcttggctttatatatcttgtggaaaggacgaaacaccggagaccacggcaggtctcagttttagtactctggaaacagaatctactaaaacaaggcaaaatgccgtgtttatctcgtcaacttgttggcgagatttttgcggccgcaggaacccctagtgatggagttggccactccctctctgcgcgctcgctcgctcactgaggccgggcgaccaaaggtcgcccgacgcccgggctttgcccgggcggcctcagtgagcgagcgagcgcgcagctgcctgcaggggcgcctgatgcggtattttctccttacgcatctgtgcggtatttcacaccgcatacgtcaaagcaaccatagtacgcgccctgtagcggcgcattaagcgcggcgggtgtggtggttacgcgcagcgtgaccgctacacttgccagcgccctagcgcccgctcctttcgctttcttcccttcctttctcgccacgttcgccggctttccccgtcaagctctaaatcgggggctccctttagggttccgatttagtgctttacggcacctcgaccccaaaaaacttgatttgggtgatggttcacgtagtgggccatcgccctgatagacggtttttcgccctttgacgttggagtccacgttctttaatagtggactcttgttccaaactggaacaacactcaaccctatctcgggctattcttttgatttataagggattttgccgatttcggcctattggttaaaaaatgagctgatttaacaaaaatttaacgcgaattttaacaaaatattaacgtttacaattttatggtgcactctcagtacaatctgctctgatgccgcatagttaagccagccccgacacccgccaacacccgctgacgcgccctgacgggcttgtctgctcccggcatccgcttacagacaagctgtgaccgtctccgggagctgcatgtgtcagaggttttcaccgtcatcaccgaaacgcgcgagacgaaagggcctcgtgatacgcctatttttataggttaatgtcatgataataatggtttcttagacgtcaggtggcacttttcggggaaatgtgcgcggaacccctatttgtttatttttctaaatacattcaaatatgtatccgctcatgagacaataaccctgataaatgcttcaataatattgaaaaaggaagagtatgagtattcaacatttccgtgtcgcccttattcccttttttgcggcattttgccttcctgtttttgctcacccagaaacgctggtgaaagtaaaagatgctgaagatcagttgggtgcacgagtgggttacatcgaactggatctcaacagcggtaagatccttgagagttttcgccccgaagaacgttttccaatgatgagcacttttaaagttctgctatgtggcgcggtattatcccgtattgacgccgggcaagagcaactcggtcgccgcatacactattctcagaatgacttggttgagtactcaccagtcacagaaaagcatcttacggatggcatgacagtaagagaattatgcagtgctgccataaccatgagtgataacactgcggccaacttacttctgacaacgatcggaggaccgaaggagctaaccgcttttttgcacaacatgggggatcatgtaactcgccttgatcgttgggaaccggagctgaatgaagccataccaaacgacgagcgtgacaccacgatgcctgtagcaatggcaacaacgttgcgcaaactattaactggcgaactacttactctagcttcccggcaacaattaatagactggatggaggcggataaagttgcaggaccacttctgcgctcggcccttccggctggctggtttattgctgataaatctggagccggtgagcgtggaagccgcggtatcattgcagcactggggccagatggtaagccctcccgtatcgtagttatctacacgacggggagtcaggcaactatggatgaacgaaatagacagatcgctgagataggtgcctcactgattaagcattggtaactgtcagaccaagtttactcatatatactttagattgatttaaaacttcatttttaatttaaaaggatctaggtgaagatcctttttgataatctcatgaccaaaatcccttaacgtgagttttcgttccactgagcgtcagaccccgtagaaaagatcaaaggatcttcttgagatcctttttttctgcgcgtaatctgctgcttgcaaacaaaaaaaccaccgctaccagcggtggtttgtttgccggatcaagagctaccaactctttttccgaaggtaactggcttcagcagagcgcagataccaaatactgtccttctagtgtagccgtagttaggccaccacttcaagaactctgtagcaccgcctacatacctcgctctgctaatcctgttaccagtggctgctgccagtggcgataagtcgtgtcttaccgggttggactcaagacgatagttaccggataaggcgcagcggtcgggctgaacggggggttcgtgcacacagcccagcttggagcgaacgacctacaccgaactgagatacctacagcgtgagctatgagaaagcgccacgcttcccgaagggagaaaggcggacaggtatccggtaagcggcagggtcggaacaggagagcgcacgagggagcttccagggggaaacgcctggtatctttatagtcctgtcgggtttcgccacctctgacttgagcgtcgatttttgtgatgctcgtcaggggggcggagcctatggaaaaacgccagcaacgcggcctttttacggttcctggccttttgctggccttttgctcacatgt

SEQ ID NO: 32 - DNA, 7701 bp, synthetic construct
  source 1..7701: mol_type = other DNA
cctgcaggcagctgcgcgctcgctcgctcactgaggccgcccgggcgtcgggcgacctttggtcgcccggcctcagtgagcgagcgagcgcgcagagagggagtggccaactccatcactaggggttcctgcggcctctagactcgaggcgttgacattgattattgactagttattaatagtaatcaattacggggtcattagttcatagcccatatatggagttccgcgttacataacttacggtaaatggcccgcctggctgaccgcccaacgacccccgcccattgacgtcaataatgacgtatgttcccatagtaacgccaatagggactttccattgacgtcaatgggtggagtatttacggtaaactgcccacttggcagtacatcaagtgtatcatatgccaagtacgccccctattgacgtcaatgacggtaaatggcccgcctggcattatgcccagtacatgaccttatgggactttcctacttggcagtacatctacgtattagtcatcgctattaccatggtgatgcggttttggcagtacatcaatgggcgtggatagcggtttgactcacggggatttccaagtctccaccccattgacgtcaatgggagtttgttttggcaccaaaatcaacgggactttccaaaatgtcgtaacaactccgccccattgacgcaaatgggcggtaggcgtgtacggtgggaggtctatataagcagagctctctggctaactaccggtgccaccatgccggcagctaagaaaaagaaactggatggcagcgtcgacatgaccatcctggagaagtacatgcccctgaacgagatgggcaagatcaagagcctggtggacgagctgaagggcatccccggcgccatgaacgccaccctgagacaggagatcttccagaacatcaagaaaaccaagctgcaggtgaagttcctggaggagtaccccgagacactgttcaccgacagcggcaacctgatccccatcatcggcaacaacgacaacagcagcagcggcacccccagcaagcaggaggtgagcgacatcgacgccaaccaggccagcagaatcaactacctgccccacgagacaatgggcgagatcaagagcgtgtacggcacctacatcgagatggccttccacaacttctacctgaccatgcaccacatctacgccgtggtgttcggcgaggacatcatggaggaggccaagaaggagttcgacaagaacaacaccaacagcaccaagtacttcaccttcgacttcgccaacgagagaaccatctggaagcccatgttcgacagagccgagagagccaagcccgagcagaaggagcacttcgagaagctggtggtgaagcacttccccttcctgaaggccatcgacgccctggaggacagaaagagaaagaccaagatccaggccctgtgcgtgttcagcctggtgctgagagagctgagaaacgtgtacagccactacctgttctaccccttcaagaaccaggtggacaagtacaaggagaacatccccttcgtgctggacatgatggagatcctgtacaccggcgcccagagagaggtgaagggcagattcggcttcgacgacaagaagatgcagtgcgccaagaagtacgagagaaacaaggaccacagccagagagatcaccagggcaagatcatcaaggccgtgcccaagaagaacttcagatacaacctgtacaagaaggaggacagcgaggccatcatcacccccttcggcctggtgttcctgaccagcctgttcctggagaagaagtacgccaagatcctgagcgacaagacccactgcatcaagtacaccgaccaggaggtgctgtgcgagatcatcagcgtgtacagaatcagactgcacatccagaagctgagcgtgaccaaggacaccgacgccctggccctggacatcatcaacgagctgcagagatgccccaagagactgttcgagatgctgagccccgacgaccagcagaagttcagaatcaagcccaccgacagccagtacgccgacgacgtgctgatgatcagacaccaggacagattcgcccacctgctgctgaagtacatcgacgacgcccacctgttcaactgcatcagattccaggtgagcctgggcagatacttcttcagattctacgacaagagctgcatcgacagcaccggcgacaagagagtgagaagcatcagcaagaacgtgaacggcttcggcagaatcaccgacatcgaggactacagaaaggaggtgtacggcgacatgatcagagagtacgaggacgtgcacgccaacaccagcatggagaagccctacatcaccgaccaccacgccaagtacctgatcagcaacaacagaatcggcctgtacatcagaaaggaggaggacacccagtgcctgctgcccgagctgacccccgacggcgccagaaacttcgcccccacctgctggctgagcatctacgagctgcccgccctggccttcctgctgcacctgtacaacggcgacggcagcagagtggaggagatcatccagaccaaggtggccaactaccagagactgttcgccgacgtgagagacggcaaggtgtgccccgtgaaggacgaggccgagctgaccaccatcctgcagacctacggcaacatcgagcccagccagctgcccagaaagctgctggactacctgctgaagaaggagatctgcgcccaggacctgttcaacacctgggcccagagcaagatccagagaatgatcgcccagaccgacagcctgctgcagcacctggagaaggacctgcaggccgtgagcgacctgaagcagaacaagttcggcaagaaggccttcgtggccatcaagcccggccacatcgccgacttcctggcccacgacatgatgttcttccagcccagcatgaaggactgcaacaacaagctgaccggcctgaacttcagaatcctgcagagcagcatggccgtgtacgacggcaacttcgacgagctgagcagaatcatgagaagcgcccacatcatcggcaacgccaacgacgcctgctgcaaccccatcgtgatggccgtgtgcagaaagcacaagggcttcagcaacatcatcagattctaccaggcctacctgaaggagagaaaggcctacctgcagcagtgcgccaacgagagacactacgacagcctgagcttcctgcacgccagccagaacaagtggagagagagaacccaggcctactacagaagcctggccgccaagtacctggccgagaactacgacggcgtggacaccaccaagagcatcgagctgcccagaggcctgttcgagacatacatcagacaggagctgagcgagatcggcagcaccaagagcatggccggcgacgccaccaagaacaccagctacctgatctacggctacttcagacaggtgatgagcgacgacgcccagaccttctacgacaccagaagatgctaccagctgttcgacgtgctgtacagaaagagccccagagacaaccacagctactacagcaccgcccagatcagagagatgctgatgagaagccacagcaagagcatcagaaaggacatcgacaactacatcagccagaccaccgccgccgagagaaccaaggagaaggagagatgcgacgccctgctgagaaagatcaaggacaccgagacagagctgaaggtgtacaagatccaggacatcctgctgttcctgatcgccaagagactgctgctggacagaaaggtggagaacgacagcgccgtgcagatgaacgccatcaaccagatcagactgagaaacatcgccgacggcaacaccctgagccagaagatccccatcagcatcagcatcaagagcagaaagggcgaccccaagatcatccagcaggacgacctgaagctgaagaactacagccagttctacagcatcatcagcgacagaagattgcccagcctgctggacctgatcaacagcagagtgatcaagagaaccgacatcgaggacgagctgagcaactacgacaagagccacccccacgtgctgaagagcgtgttcgagttcgagaagcactacttcgacacccaccccatccccagcgacaccgcctacatggccctgcccgacaccggcgagatgctgaaggagagcaacctgaccgccgagaagcagaaggaggtgagaaagatcagaaacagcttcgcccacctgagctaccccagcagaaacatcaccggcgccgccagcaccgagctgcccaagaaggccgagatcatcagcaagaacctgatcgagcacctgagcaacgccgagatcaagacaggcggcggccccggcggcggcgccgccgccggcagcggcagccctaagaaaaaacgaaaagttggcagcggaagcaaaaggccggcggccacgaaaaaggccggccaggcaaaaaagaaaaagctcgagtacccatacgatgttccagattacgcttgagaattccccttgagcatctgacttctggctaataaaggaaatttattttcattgcaatagtgtgttggaattttttgtgtctctcaggtaccgagggcctatttcccatgattccttcatatttgcatatacgatacaaggctgttagagagataattggaattaatttgactgtaaacacaaagatattagtacaaaatacgtgacgtagaaagtaataatttcttgggtagtttgcagttttaaaattatgttttaaaatggactatcatatgcttaccgtaacttgaaagtatttcgatttcttggctttatatatcttgtggaaaggacgaaacaccgtgccgttcttctgcttgtcggccatgatatgttgtagatgacctcgttttggaggggaaacacaacttttttgcggccgcaggaacccctagtgatggagttggccactccctctctgcgcgctcgctcgctcactgaggccgggcgaccaaaggtcgcccgacgcccgggctttgcccgggcggcctcagtgagcgagcgagcgcgcagctgcctgcaggggcgcctgatgcggtattttctccttacgcatctgtgcggtatttcacaccgcatacgtcaaagcaaccatagtacgcgccctgtagcggcgcattaagcgcggcgggtgtggtggttacgcgcagcgtgaccgctacacttgccagcgccttagcgcccgctcctttcgctttcttcccttcctttctcgccacgttcgccggctttccccgtcaagctctaaatcgggggctccctttagggttccgatttagtgctttacggcacctcgaccccaaaaaacttgatttgggtgatggttcacgtagtgggccatcgccctgatagacggtttttcgccctttgacgttggagtccacgttctttaatagtggactcttgttccaaactggaacaacactcaactctatctcgggctattcttttgatttataagggattttgccgatttcggtctattggttaaaaaatgagctgatttaacaaaaatttaacgcgaattttaacaaaatattaacgtttacaattttatggtgcactctcagtacaatctgctctgatgccgcatagttaagccagccccgacacccgccaacacccgctgacgcgccctgacgggcttgtctgctcccggcatccgcttacagacaagctgtgaccgtctccgggagctgcatgtgtcagaggttttcaccgtcatcaccgaaacgcgcgagacgaaagggcctcgtgatacgcctatttttataggttaatgtcatgataataatggtttcttagacgtcaggtggcacttttcggggaaatgtgcgcggaacccctatttgtttatttttctaaatacattcaaatatgtatccgctcatgagacaataaccctgataaatgcttcaataatattgaaaaaggaagagtatgagtattcaacatttccgtgtcgcccttattcccttttttgcggcattttgccttcctgtttttgctcacccagaaacgctggtgaaagtaaaagatgctgaagatcagttgggtgcacgagtgggttacatcgaactggatctcaacagcggtaagatccttgagagttttcgccccgaagaacgttttccaatgatgagcacttttaaagttctgctatgtggcgcggtattatcccgtattgacgccgggcaagagcaactcggtcgccgcatacactattctcagaatgacttggttgagtactcaccagtcacagaaaagcatcttacggatggcatgacagtaagagaattatgcagtgctgccataaccatgagtgataacactgcggccaacttacttctgacaacgatcggaggaccgaaggagctaaccgcttttttgcacaacatgggggatcatgtaactcgccttgatcgttgggaaccggagctgaatgaagccataccaaacgacgagcgtgacaccacgatgcctgtagcaatggcaacaacgttgcgcaaactattaactggcgaactacttactctagcttcccggcaacaattaatagactggatggaggcggataaagttgcaggaccacttctgcgctcggcccttccggctggctggtttattgctgataaatctggagccggtgagcgtggaagccgcggtatcattgcagcactggggccagatggtaagccctcccgtatcgtagttatctacacgacggggagtcaggcaactatggatgaacgaaatagacagatcgctgagataggtgcctcactgattaagcattggtaactgtcagaccaagtttactcatatatactttagattgatttaaaacttcatttttaatttaaaaggatctaggtgaagatcctttttgataatctcatgaccaaaatcccttaacgtgagttttcgttccactgagcgtcagaccccgtagaaaagatcaaaggatcttcttgagatcctttttttctgcgcgtaatctgctgcttgcaaacaaaaaaaccaccgctaccagcggtggtttgtttgccggatcaagagctaccaactctttttccgaaggtaactggcttcagcagagcgcagataccaaatactgttcttctagtgtagccgtagttaggccaccacttcaagaactctgtagcaccgcctacatacctcgctctgctaatcctgttaccagtggctgctgccagtggcgataagtcgtgtcttaccgggttggactcaagacgatagttaccggataaggcgcagcggtcgggctgaacggggggttcgtgcacacagcccagcttggagcgaacgacctacaccgaactgagatacctacagcgtgagctatgagaaagcgccacgcttcccgaagggagaaaggcggacaggtatccggtaagcggcagggtcggaacaggagagcgcacgagggagcttccagggggaaacgcctggtatctttatagtcctgtcgggtttcgccacctctgacttgagcgtcgatttttgtgatgctcgtcaggggggcggagcctatggaaaaacgccagcaacgcggcctttttacggttcctggccttttgctggccttttgctcacatgt

SEQ ID NO: 33 - DNA, 7941 bp, synthetic construct
  source 1..7941: mol_type = other DNA
cctgcaggcagctgcgcgctcgctcgctcactgaggccgcccgggcgtcgggcgacctttggtcgcccggcctcagtgagcgagcgagcgcgcagagagggagtggccaactccatcactaggggttcctgcggcctctagactcgaggcgttgacattgattattgactagttattaatagtaatcaattacggggtcattagttcatagcccatatatggagttccgcgttacataacttacggtaaatggcccgcctggctgaccgcccaacgacccccgcccattgacgtcaataatgacgtatgttcccatagtaacgccaatagggactttccattgacgtcaatgggtggagtatttacggtaaactgcccacttggcagtacatcaagtgtatcatatgccaagtacgccccctattgacgtcaatgacggtaaatggcccgcctggcattatgcccagtacatgaccttatgggactttcctacttggcagtacatctacgtattagtcatcgctattaccatggtgatgcggttttggcagtacatcaatgggcgtggatagcggtttgactcacggggatttccaagtctccaccccattgacgtcaatgggagtttgttttggcaccaaaatcaacgggactttccaaaatgtcgtaacaactccgccccattgacgcaaatgggcggtaggcgtgtacggtgggaggtctatataagcagagctctctggctaactaccggtgccaccatgccggcagctaagaaaaagaaactggatggcagcgtcgacatgtaccacctgagcgacgccaaccacggcaagcacatcgccggcacctactacgagatggccatgggcaacttcatccacaccctgagccacatgctggtgagagccggcatcaaggtgaacaagctggaggacaactacagcatcgagagagagatcatgaacctgaccgcccccggcgcctacgacgcccagagagccgccctgagcagactgctgtacagacacttccccttcttcggccccatcatggccgaccacaccgaccacatcctgagcagcaagagaaagaaggtgcagagcgccagcgacgacggcaacctggacctgggccaggagctgaaggacgaggtggccggcgccagcgcctgccagatgatcagatacctggccaccatcgccggcgccctggtgtactacagaaacatgtacagccacaagaaccactacgacaacgcccaggacatcgccgcccagcaggagagagagcagaagctggccctgtggctggacgtggtgttcagaggcgccagagacatcctgctgaccagaaagagccacccccagcccgacaccgacttcctgacccagaacggcaccatcaactactacatcgagaagaacggcaagagcgcctacaaccccaacttctacttcaagcccggcctgaaaaccgacaacggctgggtgatgaccgacttcggcaagttcttcttctgcagcctgttcctgagaagagccgacgccgagagattcgccgccgagacagacctgtacgtgggcagccccttcaagatcaccgcccaggagagagccagactgcaggaggccgagaacaagagagccgccgacgagcaggccagagccagcagcgccggcttcccccacatcgtgaaccccagaaccatcggccccagcgagagcccccagaacaacatcatcagagagatgctgaacatgcacagagccagaatccccagagagagaagaatcgacgccgacatgagcgagggcatcctggccatggacatcatgaacgagctgagaagatgccccctgagcctgtacaacaccctgagccccgaggccaaggccagcttcgagaaaaccggcgtgacccccgagggcggcatcgtgagcaacctgctggtgagacacagcgacagataccccgagctggccctgagagccatcgaccagatggagctgctgcccaccatcagattccacgtgagactgggcagcctgagattcagattctacgagaagaagctgatcgacggcagccacaccctgagaaccgtgcagaaggccgtgaacggcttcggcagatggcaggaggtggagcccagaagagtggagaagtacaccgccatccaggccagatgccagaacgacaagggcatcgaccagttcctgcccgacagccccaccaccaccccctacatcaccgactggagaaccacctacaacatccacgccaacagaatcggcctggcctggaacctgccccagatgagcgacggcatctacctgcccaacctggacaccgacaagggcgacaacctgcacagaaaggccctgatcgacatgcccgcccccatgtgctacctgagcatcttcgacctgcccgccctgctgttctactgccacatctacacccactaccacggcaccaagtaccacctgcccagcgccgagagcatcatccaggccaagtacgacgccctgcacaagttcttcagcttcgccgccgcccagaaccacagcgccgagcagctgagagagaagcagctggagctgaacctggccgacaacgagatccccgacaagctgagatgcatgatgcagaccaagcccttcttcaagaacggcagacagcagctgagccccctgggctaccccatcatgaagaactggatcggcgtggccgagcagagaaagcacgccgcccaggtgctgagagacgtggccaacgaggccgccgacagactggccagcttcgagaagaagcaccagagagtggtggtgggcggcagagacaacagatacggcagaagaggccacgccgacatcagacacggcagcctggccagatacctggccaccagcatggtgagatggcagcccgccctggaccagcccggcggcgacaagctgaccagcgccaaccacagagccctggccggcttcctgagcgagtacggcctgcacggcagcaacatcaacaagctgagaaacgtgctgaaggaggccggcctgatcgagggcagccacccccaccccttcctggcccacgtgctggagagcgcccccgccaacatcgaggccctgtacgtggcctacctgaagcacgagcagagccacgccaccgccctgaagaacaagttcaccgacagaaacggcatcgtgcagcccagcgaggtgcccgccttcgtgagattcaacagcagcagatggagaaacgacagcgccaccaccgccagaagatacctgcagaccccccccgcccccggcagcagcgacagcgccgagcacaacgcccccatcatgctgcccgacggcctgttcaccacccacatcatgaccctgctgaacaaggtgctgggccagaacgacagagtgcccgaggaggactacctgagacacgacctgcccagaatcgccagcatcatcaaccccaacggcaagacctacggcgccgcctacatcatcagagcctggttcgaccaggtggagaaccaggacgtgcagcccttctacgacctgcccagattctacagagagatcagcctgctggcccccagaagaaagcccaaccaggagctgatcagagactacttcagcgaggagcagatcgcccagaagatccagaccgtgcccaagaagcagagaagcgagaaggtgggccacaccatcgacaccgagaaggacatcagaagatacagactgcaggacatcaccctgtacctgaccctgctggacatgctgaccctgatgctgagcagaaacgaggccgagagaaccgacagacagatgaagagcagcaccgccgagagagtgagcaacatgagactggtggacttcgaccacagcttcgacttcgacctgctgggcagcaccagcggcgaggccgcctacagctacctgcaccagagaagcggcatcaccatcagcatgcccgccctgagcctgagaagctacggcagcatcttcagagtgctggccgacagcagattcgagacactgatggacgccctgaacagacagggcgtgacccacgtgaacttcggcgacatcaccagcgagctggccctgtacgacaccctgagaagccacttcctgctgcaggcccacaacgtggagcaggacgccttcagcgccaagagaggcgtgctggagaaccacaccagccccttcttctacagaagcggcaacctgcagctggacgaccagggcaacatcaccaaccccagcaccgacgccatcagaaaccactacggcgagctgatcaagatcctggacagatacagcctgaagatcgacaagaaaaccaaggacggcaagagccaggacatcctgctgagagacttgatggccgagctgagaaacgccgccgcccacaacagataccccaaggccgacttcttcttcagacagttcgaccacttcctgaacacctgcaagcccaccgacagcaacctgaccgcccccaactacatcagaaccgtgctggagttcctgaagagcatcgtggacaacaacttcacccccctgctgcacgaggagagccccgagaacgagagcaagagcgagacaggcggcggccccggcggcggcgccgccgccggcagcggcagccctaagaaaaaacgaaaagttggcagcggaagcaaaaggccggcggccacgaaaaaggccggccaggcaaaaaagaaaaagctcgagtacccatacgatgttccagattacgcttgagaattccccttgagcatctgacttctggctaataaaggaaatttattttcattgcaatagtgtgttggaattttttgtgtctctcaggtaccgagggcctatttcccatgattccttcatatttgcatatacgatacaaggctgttagagagataattggaattaatttgactgtaaacacaaagatattagtacaaaatacgtgacgtagaaagtaataatttcttgggtagtttgcagttttaaaattatgttttaaaatggactatcatatgcttaccgtaacttgaaagtatttcgatttcttggctttatatatcttgtggaaaggacgaaacaccgtgccgttcttctgcttgtcggccatgatatgttgtagaagccgttcattcgggacggtatgacaacttttttgcggccgcaggaacccctagtgatggagttggccactccctctctgcgcgctcgctcgctcactgaggccgggcgaccaaaggtcgcccgacgcccgggctttgcccgggcggcctcagtgagcgagcgagcgcgcagctgcctgcaggggcgcctgatgcggtattttctccttacgcatctgtgcggtatttcacaccgcatacgtcaaagcaaccatagtacgcgccctgtagcggcgcattaagcgcggcgggtgtggtggttacgcgcagcgtgaccgctacacttgccagcgccttagcgcccgctcctttcgctttcttcccttcctttctcgccacgttcgccggctttccccgtcaagctctaaatcgggggctccctttagggttccgatttagtgctttacggcacctcgaccccaaaaaacttgatttgggtgatggttcacgtagtgggccatcgccctgatagacggtttttcgccctttgacgttggagtccacgttctttaatagtggactcttgttccaaactggaacaacactcaactctatctcgggctattcttttgatttataagggattttgccgatttcggtctattggttaaaaaatgagctgatttaacaaaaatttaacgcgaattttaacaaaatattaacgtttacaattttatggtgcactctcagtacaatctgctctgatgccgcatagttaagccagccccgacacccgccaacacccgctgacgcgccctgacgggcttgtctgctcccggcatccgcttacagacaagctgtgaccgtctccgggagctgcatgtgtcagaggttttcaccgtcatcaccgaaacgcgcgagacgaaagggcctcgtgatacgcctatttttataggttaatgtcatgataataatggtttcttagacgtcaggtggcacttttcggggaaatgtgcgcggaacccctatttgtttatttttctaaatacattcaaatatgtatccgctcatgagacaataaccctgataaatgcttcaataatattgaaaaaggaagagtatgagtattcaacatttccgtgtcgcccttattcccttttttgcggcattttgccttcctgtttttgctcacccagaaacgctggtgaaagtaaaagatgctgaagatcagttgggtgcacgagtgggttacatcgaactggatctcaacagcggtaagatccttgagagttttcgccccgaagaacgttttccaatgatgagcacttttaaagttctgctatgtggcgcggtattatcccgtattgacgccgggcaagagcaactcggtcgccgcatacactattctcagaatgacttggttgagtactcaccagtcacagaaaagcatcttacggatggcatgacagtaagagaattatgcagtgctgccataaccatgagtgataacactgcggccaacttacttctgacaacgatcggaggaccgaaggagctaaccgcttttttgcacaacatgggggatcatgtaactcgccttgatcgttgggaaccggagctgaatgaagccataccaaacgacgagcgtgacaccacgatgcctgtagcaatggcaacaacgttgcgcaaactattaactggcgaactacttactctagcttcccggcaacaattaatagactggatggaggcggataaagttgcaggaccacttctgcgctcggcccttccggctggctggtttattgctgataaatctggagccggtgagcgtggaagccgcggtatcattgcagcactggggccagatggtaagccctcccgtatcgtagttatctacacgacggggagtcaggcaactatggatgaacgaaatagacagatcgctgagataggtgcctcactgattaagcattggtaactgtcagaccaagtttactcatatatactttagattgatttaaaacttcatttttaatttaaaaggatctaggtgaagatcctttttgataatctcatgaccaaaatcccttaacgtgagttttcgttccactgagcgtcagaccccgtagaaaagatcaaaggatcttcttgagatcctttttttctgcgcgtaatctgctgcttgcaaacaaaaaaaccaccgctaccagcggtggtttgtttgccggatcaagagctaccaactctttttccgaaggtaactggcttcagcagagcgcagataccaaatactgttcttctagtgtagccgtagttaggccaccacttcaagaactctgtagcaccgcctacatacctcgctctgctaatcctgttaccagtggctgctgccagtggcgataagtcgtgtcttaccgggttggactcaagacgatagttaccggataaggcgcagcggtcgggctgaacggggggttcgtgcacacagcccagcttggagcgaacgacctacaccgaactgagatacctacagcgtgagctatgagaaagcgccacgcttcccgaagggagaaaggcggacaggtatccggtaagcggcagggtcggaacaggagagcgcacgagggagcttccagggggaaacgcctggtatctttatagtcctgtcgggtttcgccacctctgacttgagcgtcgatttttgtgatgctcgtcaggggggcggagcctatggaaaaacgccagcaacgcggcctttttacggttcctggccttttgctggccttttgctcacatgt

SEQ ID NO: 34 - DNA, 7695 bp, synthetic construct
  source 1..7695: mol_type = other DNA
cctgcaggcagctgcgcgctcgctcgctcactgaggccgcccgggcgtcgggcgacctttggtcgcccggcctcagtgagcgagcgagcgcgcagagagggagtggccaactccatcactaggggttcctgcggcctctagactcgaggcgttgacattgattattgactagttattaatagtaatcaattacggggtcattagttcatagcccatatatggagttccgcgttacataacttacggtaaatggcccgcctggctgaccgcccaacgacccccgcccattgacgtcaataatgacgtatgttcccatagtaacgccaatagggactttccattgacgtcaatgggtggagtatttacggtaaactgcccacttggcagtacatcaagtgtatcatatgccaagtacgccccctattgacgtcaatgacggtaaatggcccgcctggcattatgcccagtacatgaccttatgggactttcctacttggcagtacatctacgtattagtcatcgctattaccatggtgatgcggttttggcagtacatcaatgggcgtggatagcggtttgactcacggggatttccaagtctccaccccattgacgtcaatgggagtttgttttggcaccaaaatcaacgggactttccaaaatgtcgtaacaactccgccccattgacgcaaatgggcggtaggcgtgtacggtgggaggtctatataagcagagctctctggctaactaccggtgccaccatgccggcagctaagaaaaagaaactggatggcagcgtcgacatggagaccaccatcaacaacagaatcggcaagggcgagtactacaccgaggagagcaaggagttcctggccgcctacttcaaccaggccatccacaacgtgttcatcgtgctgaaccacatcgccaagagattcggcatggacgagctgagcagcgacgaggagctgaagaactggctgatcggcagacagagagagaagaagagaaacgccatcgacagacagagattcctggagctgatcgacagacacttccccttcctgagaatcgccaacgccgacaagaaggacgccaagagagagaacgacctggaggacaacctggccctgctgatcaccctgctgaacgacctgaccgagagaagaaacaagtacagccacgccatcacccacgccagcatcgagagcaacgacagagagctggtgtggagactgtacagcatctacgacgccaacatcaacctggtgaagagagactacttcgagagcaacgtgcacaccgagatcaacgaggacccctacgagaagcaggtggagcacctgagaagattctgcatgaacaacgacagaaccaaggtggacgagaagggcaagaagaagcccgccatgcccaaccccagattcagaacccccttcctgaacgccgagacaaaccagctgagcatctacggcctggtgttcttcgtgagcctgttcctggagaagaagtacgccatccagatgcagaagaacgtgtacggcctgaaggacgccagagacaccaagttcaagatgaccaacgaggtgttctgcagaagcagaatcatcatgcccagagtgagactgcacagcgacaagagcaccgacgccctggtgctggacatgctgaacgagctggccaaggcccccgaggtgctgttcgaccagctgaccgaccccttcaaggagaagttctacatcgagagcatcgacagcctggaggagagcgacatcatcacccccgtgagagccatcagaaagcagaacagattcatgtacttcgccctgagatacctggacgagagcaacgccttcagcaagctgagattccagatcgacctgggcaactaccactaccacctgtacgagagcaagatcaacgaccagaccgagagcagacacctgaccagaaagctgttcggcttcggcaagctgatcgccttcgagcaggagttcgcccccgaggagtggaagatgaagagcaaggacctggactactacgagggcgccacccagcccttcatcgccaagacctacccccactaccacctggaggagaacaagatcggcatcctgttcaacggccaggccgaggtgcagtggccccacctggacgtggaggagcacgagagcttccccaagtacaagagaagagccaacgagaaggccgacgccttcctgagcggcaacgagctgctggccgccgccttctgccaccacctgtacgccagcatcggcaagcccaacaccgtggagaagatcatcagagacaagtaccacgccctgagacagctgttcagcgacctgaagagcggcaacctgcagaacctgctgggcgacaacaccagcaacgaggccatcagccagctgctgttcgagaagtacagactgaccctgagcgaggtgcccgtgagactgcacgccttcctgagcggccaggagcaggccgacaccaaggccatcgccagaggcaagctggagctgatggcccagcagaacaagaagagaatcgagagattcgacgccatgaagaaggccgtggtgaaggtgggcaaggcccagtacagaaccctgagaagcggcgacatcggcgactggctggtgagagacttcatgagattccagcccatcggctacaagagaaaccaggccggcaagcaggagcccgacctgaagagcaaggccaaccccaagaagtaccagctgatccagaagagcctggccctgtacgagcaggagaagaacaacctgctgggcctgttcaagagctgcaacctgctgagcagcgagaacgagcaccccttcctgaacgaggtggtgcagagcatgcccgccacctggcaggacttctacgagagatacctgcacgccagaagcagattcctggagaagtgcatcgagaagggcatcaagaagaacagctaccaggcctgctacagcttcctgaagatcaagccccagctgaaggacaaggagaagctgtaccagggctgggacgcccagatgaacctgcccaccaacatgttcatcgacgccatccacgactggttcagacagacccaccacgagagcctgagaacctggttcacccagcaggagaagccccaccagctgatcggcctgatcagaaagtacatcgagctggcccacaccgaccagatccagggcttctacgacatgttccccctgagatacgacttctacaagaaggagttccccaacggcctggtgctgcacgagagaatcaacaagcagaagcagatctgggaggcccagctgatccagaccaagaagagactggaggacgccgccagcaagctgaagaaggtgaagcagcaggtggagagcctgcccgaccaggagctgagattcagaaacgagacagaggccatggtgtacttcaccaagctgttcgacagcagcatcgtgaagaacgccatcctgaagctgcagagagatcagaaggccctgagagtgaacaccatcggcgagaagatcatcaagatctacaccgccaagtacgacgccatccaccaggaggtgagagacttcaagagcatgctgaccaccgagaagatgatcagaagagtgaaggccgaggactgcgtgaccctgttcatgctgaccgacctgatgaaccagagccagatcaccatcggccaggagcagagaaccatcaagctgagcgacatccagcccatgggcgagacacagatccagggcatcctggacgccgtgcaggtgctggagcagaagctggacttcttcagcagcgacgagcagggcaagatcagccaggtgaagctgggcgagtggaccatcttcagcaccgacaccaaggtgaagaagcagggcaacttcaagcagctgctgaaggacagaagattgaacaacctggcccactacatcctgcccgacatcgccggcggcgccatcagagtgagaagaaacctgctggagatggagctggaccagtacgacagaaacagaatccccatcatcaagctgatgtacgagctggagtacgccatctacaaggtggaccccttcagcgtggagctgaagtacaagaagttcagccagtgcctgagagagtacgcccagaaggccgtgctgaacgtggagcaggtggagcacctgaacgtgctgatcgccatcagaaacgccatcatgcacaaccagtaccccaacagagatcacctgaaggccatcgtgcccttcaccgtgagcgagtacgcccccgtgcaggagggcctgaccatcgccagacagctgctggcctgcgcccaggtgagcgtgaacatcatcctgagcaccatcagcaagttcgagacaggcggcggccccggcggcggcgccgccgccggcagcggcagccctaagaaaaaacgaaaagttggcagcggaagcaaaaggccggcggccacgaaaaaggccggccaggcaaaaaagaaaaagctcgagtacccatacgatgttccagattacgcttgagaattccccttgagcatctgacttctggctaataaaggaaatttattttcattgcaatagtgtgttggaattttttgtgtctctcaggtaccgagggcctatttcccatgattccttcatatttgcatatacgatacaaggctgttagagagataattggaattaatttgactgtaaacacaaagatattagtacaaaatacgtgacgtagaaagtaataatttcttgggtagtttgcagttttaaaattatgttttaaaatggactatcatatgcttaccgtaacttgaaagtatttcgatttcttggctttatatatcttgtggaaaggacgaaacaccgtgccgttcttctgcttgtcggccatgatatgttgtgtgtgcctttcaaattgaaggcgttcccaacttttttgcggccgcaggaacccctagtgatggagttggccactccctctctgcgcgctcgctcgctcactgaggccgggcgaccaaaggtcgcccgacgcccgggctttgcccgggcggcctcagtgagcgagcgagcgcgcagctgcctgcaggggcgcctgatgcggtattttctccttacgcatctgtgcggtatttcacaccgcatacgtcaaagcaaccatagtacgcgccctgtagcggcgcattaagcgcggcgggtgtggtggttacgcgcagcgtgaccgctacacttgccagcgccttagcgcccgctcctttcgctttcttcccttcctttctcgccacgttcgccggctttccccgtcaagctctaaatcgggggctccctttagggttccgatttagtgctttacggcacctcgaccccaaaaaacttgatttgggtgatggttcacgtagtgggccatcgccctgatagacggtttttcgccctttgacgttggagtccacgttctttaatagtggactcttgttccaaactggaacaacactcaactctatctcgggctattcttttgatttataagggattttgccgatttcggtctattggttaaaaaatgagctgatttaacaaaaatttaacgcgaattttaacaaaatattaacgtttacaattttatggtgcactctcagtacaatctgctctgatgccgcatagttaagccagccccgacacccgccaacacccgctgacgcgccctgacgggcttgtctgctcccggcatccgcttacagacaagctgtgaccgtctccgggagctgcatgtgtcagaggttttcaccgtcatcaccgaaacgcgcgagacgaaagggcctcgtgatacgcctatttttataggttaatgtcatgataataatggtttcttagacgtcaggtggcacttttcggggaaatgtgcgcggaacccctatttgtttatttttctaaatacattcaaatatgtatccgctcatgagacaataaccctgataaatgcttcaataatattgaaaaaggaagagtatgagtattcaacatttccgtgtcgcccttattcccttttttgcggcattttgccttcctgtttttgctcacccagaaacgctggtgaaagtaaaagatgctgaagatcagttgggtgcacgagtgggttacatcgaactggatctcaacagcggtaagatccttgagagttttcgccccgaagaacgttttccaatgatgagcacttttaaagttctgctatgtggcgcggtattatcccgtattgacgccgggcaagagcaactcggtcgccgcatacactattctcagaatgacttggttgagtactcaccagtcacagaaaagcatcttacggatggcatgacagtaagagaattatgcagtgctgccataaccatgagtgataacactgcggccaacttacttctgacaacgatcggaggaccgaaggagctaaccgcttttttgcacaacatgggggatcatgtaactcgccttgatcgttgggaaccggagctgaatgaagccataccaaacgacgagcgtgacaccacgatgcctgtagcaatggcaacaacgttgcgcaaactattaactggcgaactacttactctagcttcccggcaacaattaatagactggatggaggcggataaagttgcaggaccacttctgcgctcggcccttccggctggctggtttattgctgataaatctggagccggtgagcgtggaagccgcggtatcattgcagcactggggccagatggtaagccctcccgtatcgtagttatctacacgacggggagtcaggcaactatggatgaacgaaatagacagatcgctgagataggtgcctcactgattaagcattggtaactgtcagaccaagtttactcatatatactttagattgatttaaaacttcatttttaatttaaaaggatctaggtgaagatcctttttgataatctcatgaccaaaatcccttaacgtgagttttcgttccactgagcgtcagaccccgtagaaaagatcaaaggatcttcttgagatcctttttttctgcgcgtaatctgctgcttgcaaacaaaaaaaccaccgctaccagcggtggtttgtttgccggatcaagagctaccaactctttttccgaaggtaactggcttcagcagagcgcagataccaaatactgttcttctagtgtagccgtagttaggccaccacttcaagaactctgtagcaccgcctacatacctcgctctgctaatcctgttaccagtggctgctgccagtggcgataagtcgtgtcttaccgggttggactcaagacgatagttaccggataaggcgcagcggtcgggctgaacggggggttcgtgcacacagcccagcttggagcgaacgacctacaccgaactgagatacctacagcgtgagctatgagaaagcgccacgcttcccgaagggagaaaggcggacaggtatccggtaagcggcagggtcggaacaggagagcgcacgagggagcttccagggggaaacgcctggtatctttatagtcctgtcgggtttcgccacctctgacttgagcgtcgatttttgtgatgctcgtcaggggggcggagcctatggaaaaacgccagcaacgcggcctttttacggttcctggccttttgctggccttttgctcacatgt

SEQ ID NO: 35 - DNA, 6919 bp, synthetic construct
  source 1..6919: mol_type = other DNA
cctgcaggcagctgcgcgctcgctcgctcactgaggccgcccgggcgtcgggcgacctttggtcgcccggcctcagtgagcgagcgagcgcgcagagagggagtggccaactccatcactaggggttcctgcggcctctagactcgaggcgttgacattgattattgactagttattaatagtaatcaattacggggtcattagttcatagcccatatatggagttccgcgttacataacttacggtaaatggcccgcctggctgaccgcccaacgacccccgcccattgacgtcaataatgacgtatgttcccatagtaacgccaatagggactttccattgacgtcaatgggtggagtatttacggtaaactgcccacttggcagtacatcaagtgtatcatatgccaagtacgccccctattgacgtcaatgacggtaaatggcccgcctggcattatgcccagtacatgaccttatgggactttcctacttggcagtacatctacgtattagtcatcgctattaccatggtgatgcggttttggcagtacatcaatgggcgtggatagcggtttgactcacggggatttccaagtctccaccccattgacgtcaatgggagtttgttttggcaccaaaatcaacgggactttccaaaatgtcgtaacaactccgccccattgacgcaaatgggcggtaggcgtgtacggtgggaggtctatataagcagagctctctggctaactaccggtgccaccatgccggcagctaagaaaaagaaactggatggcagcgtcgacatgatgggcaacaagaagagcgtggccaaggccaacggcctgaagagcaccttcgtgctgggcgagaacaccgcctacatgaccagcttcggcagaggcaacgccgcccagcccgagaagcacatcagagacgccaccgtgaccgacatccagcacaccttcagagccaagaccgacggcggcagaaccgtgcacatcgagggcagagtgggcgccagcgacgtgctgctgcccgacgccgccaaccagctgcacgccaaggacgccgtggagcagatgtacttcggcaaggccttcagcgacaacatccacatccagatcgcctacaacatcatggacatcaagaagatcttcggcgtgtacgccaacatcatcgtgcacaccgtgaacaacctgtgctgcgacggcgacaagcaggacgacttcctgggcatgttcaagacccagaacagataccaggtggccgcctgggcccacaagatcgtgagcctgcacctggtgaagaacgagctgagaggcggcggcttcttcatggaccaggaggtgtggagagcccacgtgagaaccgacttcaagagcctgaacctggccgtgaacgccttcatgaagaagtacccccagaagtacccctactggagcgtgaagatcgtgagcgacttcatcgtgcaggagatgggcatcaagaacaaggtgatcctggagaaggccgccgagagctacgccgagttcgagacagtggccaagagactggagaagagcgcctactacttcagcgacatcttcgccggcaaggacggcaagttcgacgagcagaaggccttcgacctgctgagagtgctgggcatgatgagacaggaggccttccacgagaagaacagcagcgccagctggctgtacaacctggacgccgaggccgacgaggacatcaaggccgccctgagaaccgtggtggacaccaaggtgaacggcatcaacaccaacttcgccaagcagaacaaggtgaacctgctggtgctgcaggagatctacccccagaagagcaaggccgacctggtgagagagtactacgacttcagcgtgagaaaggccttcaagaacctgggcttcagcgtgaaaaccctgagagagacaatgtgcgccttcgacgccgccagcgtgatcaccgacaagcagtacgacaccgtgagaggcaagctgtacagcctgttcgacttcgtgatctacaactactgcctggagaacgaggccgtgtgcaacgccttcgtggaggagctgagagccaacctggaccccgagaacaagaccgccctgtaccagaccctggccgagaaggtgtgggccgagatcggcgacatcgtgctgcagagaatcctgccccagatgcacgccaagaagatccaggagagaagcaaggagacagacgccgagacagtggagatgcagggctacgtgcaggcccccaaggacctgagcctgttcagcaaggccgtgtactgcatcagcatgttcctggacggcaaggagatcaacagcttcctgagcgccctgatcaacaagttcgagaacatcagcagcctgtgcgccgtgctggcctacaacggcctggagcccgagttcgtggcccccttcaccttcttcgccgacagccaggccatcgccgaggacctgagatacatcaagagcatcgccagaatgagcaagggcaagaaggccaccaaggacagccccgtgaccgtgaaggagatgcagtacttcgacgccgccgccgtgctgggcgagacagacaccgagaaggtgaaggccgccttccacctgggcgacaagagcgccagcaccgccgacaaggccttcagaaacttcgtggtgaacaacgtgatcaacagcaacagattcgtgtacgtggtgagattcatcaaccccaagaacgccagagagatcatgcagaacagagccctgatcgccttcgtgctgaaggacatcccccagagccagctggtgagatactgcggcaccgccggcatcgcctgcaacgccgacgagcccaacaccgaggccatggtgaacgccctggccgacatgctgctgcaggtgagattcgacgccttcagcaacgtgcagcagaaggtgaaggccgacagcgccgaggccgtgcagaaggagaagtacaaggccatcatcggcctgtacctgaccgtgctgtacctgctggtgaaaaccctggtgaagatcaacatgaactacgccatcgccttcggcatcctggagagagactgccagatcatgaaccagaagcacggcaagaaccccaagagagacagagacgccttctacatgagagagcagcagaacaagcagtacgtgtacaacgccagagccatcaccgagctgttcatcgagaacggctggctgaacaagagagtgcagaagagcgtggagaacaacgccgccctgtacagcgacgaggccttctacaagtacagaaacctggtggcccacctgaacgtgatcagcgccctgcccaagtacgccaagaacatcaccaaggtgaagagcctgttcgacgtgtaccactacatcctgttcctgagcctgtgcgaggacaagtacagcaacctgcccgaggccgtgaccaagagcctgtgcaagaacggcaagaccatgctggagaacgccagagagtaccagaccgtgtgcaaggacttcctgtacggcctgaacacccccttcgcctacaacgccgccagatacatcaacctgagcaacagagagaagttcctggccggcttcggcaagacaggcggcggccccggcggcggcgccgccgccggcagcggcagccctaagaaaaaacgaaaagttggcagcggaagcaaaaggccggcggccacgaaaaaggccggccaggcaaaaaagaaaaagctcgagtacccatacgatgttccagattacgcttgagaattccccttgagcatctgacttctggctaataaaggaaatttattttcattgcaatagtgtgttggaattttttgtgtctctcaggtaccgagggcctatttcccatgattccttcatatttgcatatacgatacaaggctgttagagagataattggaattaatttgactgtaaacacaaagatattagtacaaaatacgtgacgtagaaagtaataatttcttgggtagtttgcagttttaaaattatgttttaaaatggactatcatatgcttaccgtaacttgaaagtatttcgatttcttggctttatatatcttgtggaaaggacgaaacaccgggttttacacccgtgtaaaactacacagttctaaaactgccgttcttctgcttgtcggccatgatatttttttgcggccgcaggaacccctagtgatggagttggccactccctctctgcgcgctcgctcgctcactgaggccgggcgaccaaaggtcgcccgacgcccgggctttgcccgggcggcctcagtgagcgagcgagcgcgcagctgcctgcaggggcgcctgatgcggtattttctccttacgcatctgtgcggtatttcacaccgcatacgtcaaagcaaccatagtacgcgccctgtagcggcgcattaagcgcggcgggtgtggtggttacgcgcagcgtgaccgctacacttgccagcgccttagcgcccgctcctttcgctttcttcccttcctttctcgccacgttcgccggctttccccgtcaagctctaaatcgggggctccctttagggttccgatttagtgctttacggcacctcgaccccaaaaaacttgatttgggtgatggttcacgtagtgggccatcgccctgatagacggtttttcgccctttgacgttggagtccacgttctttaatagtggactcttgttccaaactggaacaacactcaactctatctcgggctattcttttgatttataagggattttgccgatttcggtctattggttaaaaaatgagctgatttaacaaaaatttaacgcgaattttaacaaaatattaacgtttacaattttatggtgcactctcagtacaatctgctctgatgccgcatagttaagccagccccgacacccgccaacacccgctgacgcgccctgacgggcttgtctgctcccggcatccgcttacagacaagctgtgaccgtctccgggagctgcatgtgtcagaggttttcaccgtcatcaccgaaacgcgcgagacgaaagggcctcgtgatacgcctatttttataggttaatgtcatgataataatggtttcttagacgtcaggtggcacttttcggggaaatgtgcgcggaacccctatttgtttatttttctaaatacattcaaatatgtatccgctcatgagacaataaccctgataaatgcttcaataatattgaaaaaggaagagtatgagtattcaacatttccgtgtcgcccttattcccttttttgcggcattttgccttcctgtttttgctcacccagaaacgctggtgaaagtaaaagatgctgaagatcagttgggtgcacgagtgggttacatcgaactggatctcaacagcggtaagatccttgagagttttcgccccgaagaacgttttccaatgatgagcacttttaaagttctgctatgtggcgcggtattatcccgtattgacgccgggcaagagcaactcggtcgccgcatacactattctcagaatgacttggttgagtactcaccagtcacagaaaagcatcttacggatggcatgacagtaagagaattatgcagtgctgccataaccatgagtgataacactgcggccaacttacttctgacaacgatcggaggaccgaaggagctaaccgcttttttgcacaacatgggggatcatgtaactcgccttgatcgttgggaaccggagctgaatgaagccataccaaacgacgagcgtgacaccacgatgcctgtagcaatggcaacaacgttgcgcaaactattaactggcgaactacttactctagcttcccggcaacaattaatagactggatggaggcggataaagttgcaggaccacttctgcgctcggcccttccggctggctggtttattgctgataaatctggagccggtgagcgtggaagccgcggtatcattgcagcactggggccagatggtaagccctcccgtatcgtagttatctacacgacggggagtcaggcaactatggatgaacgaaatagacagatcgctgagataggtgcctcactgattaagcattggtaactgtcagaccaagtttactcatatatactttagattgatttaaaacttcatttttaatttaaaaggatctaggtgaagatcctttttgataatctcatgaccaaaatcccttaacgtgagttttcgttccactgagcgtcagaccccgtagaaaagatcaaaggatcttcttgagatcctttttttctgcgcgtaatctgctgcttgcaaacaaaaaaaccaccgctaccagcggtggtttgtttgccggatcaagagctaccaactctttttccgaaggtaactggcttcagcagagcgcagataccaaatactgttcttctagtgtagccgtagttaggccaccacttcaagaactctgtagcaccgcctacatacctcgctctgctaatcctgttaccagtggctgctgccagtggcgataagtcgtgtcttaccgggttggactcaagacgatagttaccggataaggcgcagcggtcgggctgaacggggggttcgtgcacacagcccagcttggagcgaacgacctacaccgaactgagatacctacagcgtgagctatgagaaagcgccacgcttcccgaagggagaaaggcggacaggtatccggtaagcggcagggtcggaacaggagagcgcacgagggagcttccagggggaaacgcctggtatctttatagtcctgtcgggtttcgccacctctgacttgagcgtcgatttttgtgatgctcgtcaggggggcggagcctatggaaaaacgccagcaacgcggcctttttacggttcctggccttttgctggccttttgctcacatgt

SEQ ID NO: 36 - DNA, 7690 bp, synthetic construct
  source 1..7690: mol_type = other DNA
cctgcaggcagctgcgcgctcgctcgctcactgaggccgcccgggcgtcgggcgacctttggtcgcccggcctcagtgagcgagcgagcgcgcagagagggagtggccaactccatcactaggggttcctgcggcctctagactcgaggcgttgacattgattattgactagttattaatagtaatcaattacggggtcattagttcatagcccatatatggagttccgcgttacataacttacggtaaatggcccgcctggctgaccgcccaacgacccccgcccattgacgtcaataatgacgtatgttcccatagtaacgccaatagggactttccattgacgtcaatgggtggagtatttacggtaaactgcccacttggcagtacatcaagtgtatcatatgccaagtacgccccctattgacgtcaatgacggtaaatggcccgcctggcattatgcccagtacatgaccttatgggactttcctacttggcagtacatctacgtattagtcatcgctattaccatggtgatgcggttttggcagtacatcaatgggcgtggatagcggtttgactcacggggatttccaagtctccaccccattgacgtcaatgggagtttgttttggcaccaaaatcaacgggactttccaaaatgtcgtaacaactccgccccattgacgcaaatgggcggtaggcgtgtacggtgggaggtctatataagcagagctctctggctaactaccggtgccaccatgccggcagctaagaaaaagaaactggatggcagcgtcgacatgaccatcctggagaagtacatgcccctgaacgagatgggcaagatcaagagcctggtggacgagctgaagggcatccccggcgccatgaacgccaccctgagacaggagatcttccagaacatcaagaaaaccaagctgcaggtgaagttcctggaggagtaccccgagacactgttcaccgacagcggcaacctgatccccatcatcggcaacaacgacaacagcagcagcggcacccccagcaagcaggaggtgagcgacatcgacgccaaccaggccagcagaatcaactacctgccccacgagacaatgggcgagatcaagagcgtgtacggcacctacatcgagatggccttccacaacttctacctgaccatgcaccacatctacgccgtggtgttcggcgaggacatcatggaggaggccaagaaggagttcgacaagaacaacaccaacagcaccaagtacttcaccttcgacttcgccaacgagagaaccatctggaagcccatgttcgacagagccgagagagccaagcccgagcagaaggagcacttcgagaagctggtggtgaagcacttccccttcctgaaggccatcgacgccctggaggacagaaagagaaagaccaagatccaggccctgtgcgtgttcagcctggtgctgagagagctgagaaacgtgtacagccactacctgttctaccccttcaagaaccaggtggacaagtacaaggagaacatccccttcgtgctggacatgatggagatcctgtacaccggcgcccagagagaggtgaagggcagattcggcttcgacgacaagaagatgcagtgcgccaagaagtacgagagaaacaaggaccacagccagagagatcaccagggcaagatcatcaaggccgtgcccaagaagaacttcagatacaacctgtacaagaaggaggacagcgaggccatcatcacccccttcggcctggtgttcctgaccagcctgttcctggagaagaagtacgccaagatcctgagcgacaagacccactgcatcaagtacaccgaccaggaggtgctgtgcgagatcatcagcgtgtacagaatcagactgcacatccagaagctgagcgtgaccaaggacaccgacgccctggccctggacatcatcaacgagctgcagagatgccccaagagactgttcgagatgctgagccccgacgaccagcagaagttcagaatcaagcccaccgacagccagtacgccgacgacgtgctgatgatcagacaccaggacagattcgcccacctgctgctgaagtacatcgacgacgcccacctgttcaactgcatcagattccaggtgagcctgggcagatacttcttcagattctacgacaagagctgcatcgacagcaccggcgacaagagagtgagaagcatcagcaagaacgtgaacggcttcggcagaatcaccgacatcgaggactacagaaaggaggtgtacggcgacatgatcagagagtacgaggacgtgcacgccaacaccagcatggagaagccctacatcaccgaccaccacgccaagtacctgatcagcaacaacagaatcggcctgtacatcagaaaggaggaggacacccagtgcctgctgcccgagctgacccccgacggcgccagaaacttcgcccccacctgctggctgagcatctacgagctgcccgccctggccttcctgctgcacctgtacaacggcgacggcagcagagtggaggagatcatccagaccaaggtggccaactaccagagactgttcgccgacgtgagagacggcaaggtgtgccccgtgaaggacgaggccgagctgaccaccatcctgcagacctacggcaacatcgagcccagccagctgcccagaaagctgctggactacctgctgaagaaggagatctgcgcccaggacctgttcaacacctgggcccagagcaagatccagagaatgatcgcccagaccgacagcctgctgcagcacctggagaaggacctgcaggccgtgagcgacctgaagcagaacaagttcggcaagaaggccttcgtggccatcaagcccggccacatcgccgacttcctggcccacgacatgatgttcttccagcccagcatgaaggactgcaacaacaagctgaccggcctgaacttcagaatcctgcagagcagcatggccgtgtacgacggcaacttcgacgagctgagcagaatcatgagaagcgcccacatcatcggcaacgccaacgacgcctgctgcaaccccatcgtgatggccgtgtgcagaaagcacaagggcttcagcaacatcatcagattctaccaggcctacctgaaggagagaaaggcctacctgcagcagtgcgccaacgagagacactacgacagcctgagcttcctgcacgccagccagaacaagtggagagagagaacccaggcctactacagaagcctggccgccaagtacctggccgagaactacgacggcgtggacaccaccaagagcatcgagctgcccagaggcctgttcgagacatacatcagacaggagctgagcgagatcggcagcaccaagagcatggccggcgacgccaccaagaacaccagctacctgatctacggctacttcagacaggtgatgagcgacgacgcccagaccttctacgacaccagaagatgctaccagctgttcgacgtgctgtacagaaagagccccagagacaaccacagctactacagcaccgcccagatcagagagatgctgatgagaagccacagcaagagcatcagaaaggacatcgacaactacatcagccagaccaccgccgccgagagaaccaaggagaaggagagatgcgacgccctgctgagaaagatcaaggacaccgagacagagctgaaggtgtacaagatccaggacatcctgctgttcctgatcgccaagagactgctgctggacagaaaggtggagaacgacagcgccgtgcagatgaacgccatcaaccagatcagactgagaaacatcgccgacggcaacaccctgagccagaagatccccatcagcatcagcatcaagagcagaaagggcgaccccaagatcatccagcaggacgacctgaagctgaagaactacagccagttctacagcatcatcagcgacagaagattgcccagcctgctggacctgatcaacagcagagtgatcaagagaaccgacatcgaggacgagctgagcaactacgacaagagccacccccacgtgctgaagagcgtgttcgagttcgagaagcactacttcgacacccaccccatccccagcgacaccgcctacatggccctgcccgacaccggcgagatgctgaaggagagcaacctgaccgccgagaagcagaaggaggtgagaaagatcagaaacagcttcgcccacctgagctaccccagcagaaacatcaccggcgccgccagcaccgagctgcccaagaaggccgagatcatcagcaagaacctgatcgagcacctgagcaacgccgagatcaagacaggcggcggccccggcggcggcgccgccgccggcagcggcagccctaagaaaaaacgaaaagttggcagcggaagcaaaaggccggcggccacgaaaaaggccggccaggcaaaaaagaaaaagctcgagtacccatacgatgttccagattacgcttgagaattccccttgagcatctgacttctggctaataaaggaaatttattttcattgcaatagtgtgttggaattttttgtgtctctcaggtaccgagggcctatttcccatgattccttcatatttgcatatacgatacaaggctgttagagagataattggaattaatttgactgtaaacacaaagatattagtacaaaatacgtgacgtagaaagtaataatttcttgggtagtttgcagttttaaaattatgttttaaaatggactatcatatgcttaccgtaacttgaaagtatttcgatttcttggctttatatatcttgtggaaaggacgaaacaccggagaccacggcaggtctcagttgtagatgacctcgttttggaggggaaacacaacttttttgcggccgcaggaacccctagtgatggagttggccactccctctctgcgcgctcgctcgctcactgaggccgggcgaccaaaggtcgcccgacgcccgggctttgcccgggcggcctcagtgagcgagcgagcgcgcagctgcctgcaggggcgcctgatgcggtattttctccttacgcatctgtgcggtatttcacaccgcatacgtcaaagcaaccatagtacgcgccctgtagcggcgcattaagcgcggcgggtgtggtggttacgcgcagcgtgaccgctacacttgccagcgccttagcgcccgctcctttcgctttcttcccttcctttctcgccacgttcgccggctttccccgtcaagctctaaatcgggggctccctttagggttccgatttagtgctttacggcacctcgaccccaaaaaacttgatttgggtgatggttcacgtagtgggccatcgccctgatagacggtttttcgccctttgacgttggagtccacgttctttaatagtggactcttgttccaaactggaacaacactcaactctatctcgggctattcttttgatttataagggattttgccgatttcggtctattggttaaaaaatgagctgatttaacaaaaatttaacgcgaattttaacaaaatattaacgtttacaattttatggtgcactctcagtacaatctgctctgatgccgcatagttaagccagccccgacacccgccaacacccgctgacgcgccctgacgggcttgtctgctcccggcatccgcttacagacaagctgtgaccgtctccgggagctgcatgtgtcagaggttttcaccgtcatcaccgaaacgcgcgagacgaaagggcctcgtgatacgcctatttttataggttaatgtcatgataataatggtttcttagacgtcaggtggcacttttcggggaaatgtgcgcggaacccctatttgtttatttttctaaatacattcaaatatgtatccgctcatgagacaataaccctgataaatgcttcaataatattgaaaaaggaagagtatgagtattcaacatttccgtgtcgcccttattcccttttttgcggcattttgccttcctgtttttgctcacccagaaacgctggtgaaagtaaaagatgctgaagatcagttgggtgcacgagtgggttacatcgaactggatctcaacagcggtaagatccttgagagttttcgccccgaagaacgttttccaatgatgagcacttttaaagttctgctatgtggcgcggtattatcccgtattgacgccgggcaagagcaactcggtcgccgcatacactattctcagaatgacttggttgagtactcaccagtcacagaaaagcatcttacggatggcatgacagtaagagaattatgcagtgctgccataaccatgagtgataacactgcggccaacttacttctgacaacgatcggaggaccgaaggagctaaccgcttttttgcacaacatgggggatcatgtaactcgccttgatcgttgggaaccggagctgaatgaagccataccaaacgacgagcgtgacaccacgatgcctgtagcaatggcaacaacgttgcgcaaactattaactggcgaactacttactctagcttcccggcaacaattaatagactggatggaggcggataaagttgcaggaccacttctgcgctcggcccttccggctggctggtttattgctgataaatctggagccggtgagcgtggaagccgcggtatcattgcagcactggggccagatggtaagccctcccgtatcgtagttatctacacgacggggagtcaggcaactatggatgaacgaaatagacagatcgctgagataggtgcctcactgattaagcattggtaactgtcagaccaagtttactcatatatactttagattgatttaaaacttcatttttaatttaaaaggatctaggtgaagatcctttttgataatctcatgaccaaaatcccttaacgtgagttttcgttccactgagcgtcagaccccgtagaaaagatcaaaggatcttcttgagatcctttttttctgcgcgtaatctgctgcttgcaaacaaaaaaaccaccgctaccagcggtggtttgtttgccggatcaagagctaccaactctttttccgaaggtaactggcttcagcagagcgcagataccaaatactgttcttctagtgtagccgtagttaggccaccacttcaagaactctgtagcaccgcctacatacctcgctctgctaatcctgttaccagtggctgctgccagtggcgataagtcgtgtcttaccgggttggactcaagacgatagttaccggataaggcgcagcggtcgggctgaacggggggttcgtgcacacagcccagcttggagcgaacgacctacaccgaactgagatacctacagcgtgagctatgagaaagcgccacgcttcccgaagggagaaaggcggacaggtatccggtaagcggcagggtcggaacaggagagcgcacgagggagcttccagggggaaacgcctggtatctttatagtcctgtcgggtttcgccacctctgacttgagcgtcgatttttgtgatgctcgtcaggggggcggagcctatggaaaaacgccagcaacgcggcctttttacggttcctggccttttgctggccttttgctcacatgt

SEQ ID NO: 37 - DNA, 7930 bp, synthetic construct
  source 1..7930: mol_type = other DNA
cctgcaggcagctgcgcgctcgctcgctcactgaggccgcccgggcgtcgggcgacctttggtcgcccggcctcagtgagcgagcgagcgcgcagagagggagtggccaactccatcactaggggttcctgcggcctctagactcgaggcgttgacattgattattgactagttattaatagtaatcaattacggggtcattagttcatagcccatatatggagttccgcgttacataacttacggtaaatggcccgcctggctgaccgcccaacgacccccgcccattgacgtcaataatgacgtatgttcccatagtaacgccaatagggactttccattgacgtcaatgggtggagtatttacggtaaactgcccacttggcagtacatcaagtgtatcatatgccaagtacgccccctattgacgtcaatgacggtaaatggcccgcctggcattatgcccagtacatgaccttatgggactttcctacttggcagtacatctacgtattagtcatcgctattaccatggtgatgcggttttggcagtacatcaatgggcgtggatagcggtttgactcacggggatttccaagtctccaccccattgacgtcaatgggagtttgttttggcaccaaaatcaacgggactttccaaaatgtcgtaacaactccgccccattgacgcaaatgggcggtaggcgtgtacggtgggaggtctatataagcagagctctctggctaactaccggtgccaccatgccggcagctaagaaaaagaaactggatggcagcgtcgacatgtaccacctgagcgacgccaaccacggcaagcacatcgccggcacctactacgagatggccatgggcaacttcatccacaccctgagccacatgctggtgagagccggcatcaaggtgaacaagctggaggacaactacagcatcgagagagagatcatgaacctgaccgcccccggcgcctacgacgcccagagagccgccctgagcagactgctgtacagacacttccccttcttcggccccatcatggccgaccacaccgaccacatcctgagcagcaagagaaagaaggtgcagagcgccagcgacgacggcaacctggacctgggccaggagctgaaggacgaggtggccggcgccagcgcctgccagatgatcagatacctggccaccatcgccggcgccctggtgtactacagaaacatgtacagccacaagaaccactacgacaacgcccaggacatcgccgcccagcaggagagagagcagaagctggccctgtggctggacgtggtgttcagaggcgccagagacatcctgctgaccagaaagagccacccccagcccgacaccgacttcctgacccagaacggcaccatcaactactacatcgagaagaacggcaagagcgcctacaaccccaacttctacttcaagcccggcctgaaaaccgacaacggctgggtgatgaccgacttcggcaagttcttcttctgcagcctgttcctgagaagagccgacgccgagagattcgccgccgagacagacctgtacgtgggcagccccttcaagatcaccgcccaggagagagccagactgcaggaggccgagaacaagagagccgccgacgagcaggccagagccagcagcgccggcttcccccacatcgtgaaccccagaaccatcggccccagcgagagcccccagaacaacatcatcagagagatgctgaacatgcacagagccagaatccccagagagagaagaatcgacgccgacatgagcgagggcatcctggccatggacatcatgaacgagctgagaagatgccccctgagcctgtacaacaccctgagccccgaggccaaggccagcttcgagaaaaccggcgtgacccccgagggcggcatcgtgagcaacctgctggtgagacacagcgacagataccccgagctggccctgagagccatcgaccagatggagctgctgcccaccatcagattccacgtgagactgggcagcctgagattcagattctacgagaagaagctgatcgacggcagccacaccctgagaaccgtgcagaaggccgtgaacggcttcggcagatggcaggaggtggagcccagaagagtggagaagtacaccgccatccaggccagatgccagaacgacaagggcatcgaccagttcctgcccgacagccccaccaccaccccctacatcaccgactggagaaccacctacaacatccacgccaacagaatcggcctggcctggaacctgccccagatgagcgacggcatctacctgcccaacctggacaccgacaagggcgacaacctgcacagaaaggccctgatcgacatgcccgcccccatgtgctacctgagcatcttcgacctgcccgccctgctgttctactgccacatctacacccactaccacggcaccaagtaccacctgcccagcgccgagagcatcatccaggccaagtacgacgccctgcacaagttcttcagcttcgccgccgcccagaaccacagcgccgagcagctgagagagaagcagctggagctgaacctggccgacaacgagatccccgacaagctgagatgcatgatgcagaccaagcccttcttcaagaacggcagacagcagctgagccccctgggctaccccatcatgaagaactggatcggcgtggccgagcagagaaagcacgccgcccaggtgctgagagacgtggccaacgaggccgccgacagactggccagcttcgagaagaagcaccagagagtggtggtgggcggcagagacaacagatacggcagaagaggccacgccgacatcagacacggcagcctggccagatacctggccaccagcatggtgagatggcagcccgccctggaccagcccggcggcgacaagctgaccagcgccaaccacagagccctggccggcttcctgagcgagtacggcctgcacggcagcaacatcaacaagctgagaaacgtgctgaaggaggccggcctgatcgagggcagccacccccaccccttcctggcccacgtgctggagagcgcccccgccaacatcgaggccctgtacgtggcctacctgaagcacgagcagagccacgccaccgccctgaagaacaagttcaccgacagaaacggcatcgtgcagcccagcgaggtgcccgccttcgtgagattcaacagcagcagatggagaaacgacagcgccaccaccgccagaagatacctgcagaccccccccgcccccggcagcagcgacagcgccgagcacaacgcccccatcatgctgcccgacggcctgttcaccacccacatcatgaccctgctgaacaaggtgctgggccagaacgacagagtgcccgaggaggactacctgagacacgacctgcccagaatcgccagcatcatcaaccccaacggcaagacctacggcgccgcctacatcatcagagcctggttcgaccaggtggagaaccaggacgtgcagcccttctacgacctgcccagattctacagagagatcagcctgctggcccccagaagaaagcccaaccaggagctgatcagagactacttcagcgaggagcagatcgcccagaagatccagaccgtgcccaagaagcagagaagcgagaaggtgggccacaccatcgacaccgagaaggacatcagaagatacagactgcaggacatcaccctgtacctgaccctgctggacatgctgaccctgatgctgagcagaaacgaggccgagagaaccgacagacagatgaagagcagcaccgccgagagagtgagcaacatgagactggtggacttcgaccacagcttcgacttcgacctgctgggcagcaccagcggcgaggccgcctacagctacctgcaccagagaagcggcatcaccatcagcatgcccgccctgagcctgagaagctacggcagcatcttcagagtgctggccgacagcagattcgagacactgatggacgccctgaacagacagggcgtgacccacgtgaacttcggcgacatcaccagcgagctggccctgtacgacaccctgagaagccacttcctgctgcaggcccacaacgtggagcaggacgccttcagcgccaagagaggcgtgctggagaaccacaccagccccttcttctacagaagcggcaacctgcagctggacgaccagggcaacatcaccaaccccagcaccgacgccatcagaaaccactacggcgagctgatcaagatcctggacagatacagcctgaagatcgacaagaaaaccaaggacggcaagagccaggacatcctgctgagagacttgatggccgagctgagaaacgccgccgcccacaacagataccccaaggccgacttcttcttcagacagttcgaccacttcctgaacacctgcaagcccaccgacagcaacctgaccgcccccaactacatcagaaccgtgctggagttcctgaagagcatcgtggacaacaacttcacccccctgctgcacgaggagagccccgagaacgagagcaagagcgagacaggcggcggccccggcggcggcgccgccgccggcagcggcagccctaagaaaaaacgaaaagttggcagcggaagcaaaaggccggcggccacgaaaaaggccggccaggcaaaaaagaaaaagctcgagtacccatacgatgttccagattacgcttgagaattccccttgagcatctgacttctggctaataaaggaaatttattttcattgcaatagtgtgttggaattttttgtgtctctcaggtaccgagggcctatttcccatgattccttcatatttgcatatacgatacaaggctgttagagagataattggaattaatttgactgtaaacacaaagatattagtacaaaatacgtgacgtagaaagtaataatttcttgggtagtttgcagttttaaaattatgttttaaaatggactatcatatgcttaccgtaacttgaaagtatttcgatttcttggctttatatatcttgtggaaaggacgaaacaccggagaccacggcaggtctcagttgtagaagccgttcattcgggacggtatgacaacttttttgcggccgcaggaacccctagtgatggagttggccactccctctctgcgcgctcgctcgctcactgaggccgggcgaccaaaggtcgcccgacgcccgggctttgcccgggcggcctcagtgagcgagcgagcgcgcagctgcctgcaggggcgcctgatgcggtattttctccttacgcatctgtgcggtatttcacaccgcatacgtcaaagcaaccatagtacgcgccctgtagcggcgcattaagcgcggcgggtgtggtggttacgcgcagcgtgaccgctacacttgccagcgccttagcgcccgctcctttcgctttcttcccttcctttctcgccacgttcgccggctttccccgtcaagctctaaatcgggggctccctttagggttccgatttagtgctttacggcacctcgaccccaaaaaacttgatttgggtgatggttcacgtagtgggccatcgccctgatagacggtttttcgccctttgacgttggagtccacgttctttaatagtggactcttgttccaaactggaacaacactcaactctatctcgggctattcttttgatttataagggattttgccgatttcggtctattggttaaaaaatgagctgatttaacaaaaatttaacgcgaattttaacaaaatattaacgtttacaattttatggtgcactctcagtacaatctgctctgatgccgcatagttaagccagccccgacacccgccaacacccgctgacgcgccctgacgggcttgtctgctcccggcatccgcttacagacaagctgtgaccgtctccgggagctgcatgtgtcagaggttttcaccgtcatcaccgaaacgcgcgagacgaaagggcctcgtgatacgcctatttttataggttaatgtcatgataataatggtttcttagacgtcaggtggcacttttcggggaaatgtgcgcggaacccctatttgtttatttttctaaatacattcaaatatgtatccgctcatgagacaataaccctgataaatgcttcaataatattgaaaaaggaagagtatgagtattcaacatttccgtgtcgcccttattcccttttttgcggcattttgccttcctgtttttgctcacccagaaacgctggtgaaagtaaaagatgctgaagatcagttgggtgcacgagtgggttacatcgaactggatctcaacagcggtaagatccttgagagttttcgccccgaagaacgttttccaatgatgagcacttttaaagttctgctatgtggcgcggtattatcccgtattgacgccgggcaagagcaactcggtcgccgcatacactattctcagaatgacttggttgagtactcaccagtcacagaaaagcatcttacggatggcatgacagtaagagaattatgcagtgctgccataaccatgagtgataacactgcggccaacttacttctgacaacgatcggaggaccgaaggagctaaccgcttttttgcacaacatgggggatcatgtaactcgccttgatcgttgggaaccggagctgaatgaagccataccaaacgacgagcgtgacaccacgatgcctgtagcaatggcaacaacgttgcgcaaactattaactggcgaactacttactctagcttcccggcaacaattaatagactggatggaggcggataaagttgcaggaccacttctgcgctcggcccttccggctggctggtttattgctgataaatctggagccggtgagcgtggaagccgcggtatcattgcagcactggggccagatggtaagccctcccgtatcgtagttatctacacgacggggagtcaggcaactatggatgaacgaaatagacagatcgctgagataggtgcctcactgattaagcattggtaactgtcagaccaagtttactcatatatactttagattgatttaaaacttcatttttaatttaaaaggatctaggtgaagatcctttttgataatctcatgaccaaaatcccttaacgtgagttttcgttccactgagcgtcagaccccgtagaaaagatcaaaggatcttcttgagatcctttttttctgcgcgtaatctgctgcttgcaaacaaaaaaaccaccgctaccagcggtggtttgtttgccggatcaagagctaccaactctttttccgaaggtaactggcttcagcagagcgcagataccaaatactgttcttctagtgtagccgtagttaggccaccacttcaagaactctgtagcaccgcctacatacctcgctctgctaatcctgttaccagtggctgctgccagtggcgataagtcgtgtcttaccgggttggactcaagacgatagttaccggataaggcgcagcggtcgggctgaacggggggttcgtgcacacagcccagcttggagcgaacgacctacaccgaactgagatacctacagcgtgagctatgagaaagcgccacgcttcccgaagggagaaaggcggacaggtatccggtaagcggcagggtcggaacaggagagcgcacgagggagcttccagggggaaacgcctggtatctttatagtcctgtcgggtttcgccacctctgacttgagcgtcgatttttgtgatgctcgtcaggggggcggagcctatggaaaaacgccagcaacgcggcctttttacggttcctggccttttgctggccttttgctcacatgt

SEQ ID NO: 38 - DNA, 7684 bp, synthetic construct
  source 1..7684: mol_type = other DNA
cctgcaggcagctgcgcgctcgctcgctcactgaggccgcccgggcgtcgggcgacctttggtcgcccggcctcagtgagcgagcgagcgcgcagagagggagtggccaactccatcactaggggttcctgcggcctctagactcgaggcgttgacattgattattgactagttattaatagtaatcaattacggggtcattagttcatagcccatatatggagttccgcgttacataacttacggtaaatggcccgcctggctgaccgcccaacgacccccgcccattgacgtcaataatgacgtatgttcccatagtaacgccaatagggactttccattgacgtcaatgggtggagtatttacggtaaactgcccacttggcagtacatcaagtgtatcatatgccaagtacgccccctattgacgtcaatgacggtaaatggcccgcctggcattatgcccagtacatgaccttatgggactttcctacttggcagtacatctacgtattagtcatcgctattaccatggtgatgcggttttggcagtacatcaatgggcgtggatagcggtttgactcacggggatttccaagtctccaccccattgacgtcaatgggagtttgttttggcaccaaaatcaacgggactttccaaaatgtcgtaacaactccgccccattgacgcaaatgggcggtaggcgtgtacggtgggaggtctatataagcagagctctctggctaactaccggtgccaccatgccggcagctaagaaaaagaaactggatggcagcgtcgacatggagaccaccatcaacaacagaatcggcaagggcgagtactacaccgaggagagcaaggagttcctggccgcctacttcaaccaggccatccacaacgtgttcatcgtgctgaaccacatcgccaagagattcggcatggacgagctgagcagcgacgaggagctgaagaactggctgatcggcagacagagagagaagaagagaaacgccatcgacagacagagattcctggagctgatcgacagacacttccccttcctgagaatcgccaacgccgacaagaaggacgccaagagagagaacgacctggaggacaacctggccctgctgatcaccctgctgaacgacctgaccgagagaagaaacaagtacagccacgccatcacccacgccagcatcgagagcaacgacagagagctggtgtggagactgtacagcatctacgacgccaacatcaacctggtgaagagagactacttcgagagcaacgtgcacaccgagatcaacgaggacccctacgagaagcaggtggagcacctgagaagattctgcatgaacaacgacagaaccaaggtggacgagaagggcaagaagaagcccgccatgcccaaccccagattcagaacccccttcctgaacgccgagacaaaccagctgagcatctacggcctggtgttcttcgtgagcctgttcctggagaagaagtacgccatccagatgcagaagaacgtgtacggcctgaaggacgccagagacaccaagttcaagatgaccaacgaggtgttctgcagaagcagaatcatcatgcccagagtgagactgcacagcgacaagagcaccgacgccctggtgctggacatgctgaacgagctggccaaggcccccgaggtgctgttcgaccagctgaccgaccccttcaaggagaagttctacatcgagagcatcgacagcctggaggagagcgacatcatcacccccgtgagagccatcagaaagcagaacagattcatgtacttcgccctgagatacctggacgagagcaacgccttcagcaagctgagattccagatcgacctgggcaactaccactaccacctgtacgagagcaagatcaacgaccagaccgagagcagacacctgaccagaaagctgttcggcttcggcaagctgatcgccttcgagcaggagttcgcccccgaggagtggaagatgaagagcaaggacctggactactacgagggcgccacccagcccttcatcgccaagacctacccccactaccacctggaggagaacaagatcggcatcctgttcaacggccaggccgaggtgcagtggccccacctggacgtggaggagcacgagagcttccccaagtacaagagaagagccaacgagaaggccgacgccttcctgagcggcaacgagctgctggccgccgccttctgccaccacctgtacgccagcatcggcaagcccaacaccgtggagaagatcatcagagacaagtaccacgccctgagacagctgttcagcgacctgaagagcggcaacctgcagaacctgctgggcgacaacaccagcaacgaggccatcagccagctgctgttcgagaagtacagactgaccctgagcgaggtgcccgtgagactgcacgccttcctgagcggccaggagcaggccgacaccaaggccatcgccagaggcaagctggagctgatggcccagcagaacaagaagagaatcgagagattcgacgccatgaagaaggccgtggtgaaggtgggcaaggcccagtacagaaccctgagaagcggcgacatcggcgactggctggtgagagacttcatgagattccagcccatcggctacaagagaaaccaggccggcaagcaggagcccgacctgaagagcaaggccaaccccaagaagtaccagctgatccagaagagcctggccctgtacgagcaggagaagaacaacctgctgggcctgttcaagagctgcaacctgctgagcagcgagaacgagcaccccttcctgaacgaggtggtgcagagcatgcccgccacctggcaggacttctacgagagatacctgcacgccagaagcagattcctggagaagtgcatcgagaagggcatcaagaagaacagctaccaggcctgctacagcttcctgaagatcaagccccagctgaaggacaaggagaagctgtaccagggctgggacgcccagatgaacctgcccaccaacatgttcatcgacgccatccacgactggttcagacagacccaccacgagagcctgagaacctggttcacccagcaggagaagccccaccagctgatcggcctgatcagaaagtacatcgagctggcccacaccgaccagatccagggcttctacgacatgttccccctgagatacgacttctacaagaaggagttccccaacggcctggtgctgcacgagagaatcaacaagcagaagcagatctgggaggcccagctgatccagaccaagaagagactggaggacgccgccagcaagctgaagaaggtgaagcagcaggtggagagcctgcccgaccaggagctgagattcagaaacgagacagaggccatggtgtacttcaccaagctgttcgacagcagcatcgtgaagaacgccatcctgaagctgcagagagatcagaaggccctgagagtgaacaccatcggcgagaagatcatcaagatctacaccgccaagtacgacgccatccaccaggaggtgagagacttcaagagcatgctgaccaccgagaagatgatcagaagagtgaaggccgaggactgcgtgaccctgttcatgctgaccgacctgatgaaccagagccagatcaccatcggccaggagcagagaaccatcaagctgagcgacatccagcccatgggcgagacacagatccagggcatcctggacgccgtgcaggtgctggagcagaagctggacttcttcagcagcgacgagcagggcaagatcagccaggtgaagctgggcgagtggaccatcttcagcaccgacaccaaggtgaagaagcagggcaacttcaagcagctgctgaaggacagaagattgaacaacctggcccactacatcctgcccgacatcgccggcggcgccatcagagtgagaagaaacctgctggagatggagctggaccagtacgacagaaacagaatccccatcatcaagctgatgtacgagctggagtacgccatctacaaggtggaccccttcagcgtggagctgaagtacaagaagttcagccagtgcctgagagagtacgcccagaaggccgtgctgaacgtggagcaggtggagcacctgaacgtgctgatcgccatcagaaacgccatcatgcacaaccagtaccccaacagagatcacctgaaggccatcgtgcccttcaccgtgagcgagtacgcccccgtgcaggagggcctgaccatcgccagacagctgctggcctgcgcccaggtgagcgtgaacatcatcctgagcaccatcagcaagttcgagacaggcggcggccccggcggcggcgccgccgccggcagcggcagccctaagaaaaaacgaaaagttggcagcggaagcaaaaggccggcggccacgaaaaaggccggccaggcaaaaaagaaaaagctcgagtacccatacgatgttccagattacgcttgagaattccccttgagcatctgacttctggctaataaaggaaatttattttcattgcaatagtgtgttggaattttttgtgtctctcaggtaccgagggcctatttcccatgattccttcatatttgcatatacgatacaaggctgttagagagataattggaattaatttgactgtaaacacaaagatattagtacaaaatacgtgacgtagaaagtaataatttcttgggtagtttgcagttttaaaattatgttttaaaatggactatcatatgcttaccgtaacttgaaagtatttcgatttcttggctttatatatcttgtggaaaggacgaaacaccggagaccacggcaggtctcagttgtgtgtgcctttcaaattgaaggcgttcccaacttttttgcggccgcaggaacccctagtgatggagttggccactccctctctgcgcgctcgctcgctcactgaggccgggcgaccaaaggtcgcccgacgcccgggctttgcccgggcggcctcagtgagcgagcgagcgcgcagctgcctgcaggggcgcctgatgcggtattttctccttacgcatctgtgcggtatttcacaccgcatacgtcaaagcaaccatagtacgcgccctgtagcggcgcattaagcgcggcgggtgtggtggttacgcgcagcgtgaccgctacacttgccagcgccttagcgcccgctcctttcgctttcttcccttcctttctcgccacgttcgccggctttccccgtcaagctctaaatcgggggctccctttagggttccgatttagtgctttacggcacctcgaccccaaaaaacttgatttgggtgatggttcacgtagtgggccatcgccctgatagacggtttttcgccctttgacgttggagtccacgttctttaatagtggactcttgttccaaactggaacaacactcaactctatctcgggctattcttttgatttataagggattttgccgatttcggtctattggttaaaaaatgagctgatttaacaaaaatttaacgcgaattttaacaaaatattaacgtttacaattttatggtgcactctcagtacaatctgctctgatgccgcatagttaagccagccccgacacccgccaacacccgctgacgcgccctgacgggcttgtctgctcccggcatccgcttacagacaagctgtgaccgtctccgggagctgcatgtgtcagaggttttcaccgtcatcaccgaaacgcgcgagacgaaagggcctcgtgatacgcctatttttataggttaatgtcatgataataatggtttcttagacgtcaggtggcacttttcggggaaatgtgcgcggaacccctatttgtttatttttctaaatacattcaaatatgtatccgctcatgagacaataaccctgataaatgcttcaataatattgaaaaaggaagagtatgagtattcaacatttccgtgtcgcccttattcccttttttgcggcattttgccttcctgtttttgctcacccagaaacgctggtgaaagtaaaagatgctgaagatcagttgggtgcacgagtgggttacatcgaactggatctcaacagcggtaagatccttgagagttttcgccccgaagaacgttttccaatgatgagcacttttaaagttctgctatgtggcgcggtattatcccgtattgacgccgggcaagagcaactcggtcgccgcatacactattctcagaatgacttggttgagtactcaccagtcacagaaaagcatcttacggatggcatgacagtaagagaattatgcagtgctgccataaccatgagtgataacactgcggccaacttacttctgacaacgatcggaggaccgaaggagctaaccgcttttttgcacaacatgggggatcatgtaactcgccttgatcgttgggaaccggagctgaatgaagccataccaaacgacgagcgtgacaccacgatgcctgtagcaatggcaacaacgttgcgcaaactattaactggcgaactacttactctagcttcccggcaacaattaatagactggatggaggcggataaagttgcaggaccacttctgcgctcggcccttccggctggctggtttattgctgataaatctggagccggtgagcgtggaagccgcggtatcattgcagcactggggccagatggtaagccctcccgtatcgtagttatctacacgacggggagtcaggcaactatggatgaacgaaatagacagatcgctgagataggtgcctcactgattaagcattggtaactgtcagaccaagtttactcatatatactttagattgatttaaaacttcatttttaatttaaaaggatctaggtgaagatcctttttgataatctcatgaccaaaatcccttaacgtgagttttcgttccactgagcgtcagaccccgtagaaaagatcaaaggatcttcttgagatcctttttttctgcgcgtaatctgctgcttgcaaacaaaaaaaccaccgctaccagcggtggtttgtttgccggatcaagagctaccaactctttttccgaaggtaactggcttcagcagagcgcagataccaaatactgttcttctagtgtagccgtagttaggccaccacttcaagaactctgtagcaccgcctacatacctcgctctgctaatcctgttaccagtggctgctgccagtggcgataagtcgtgtcttaccgggttggactcaagacgatagttaccggataaggcgcagcggtcgggctgaacggggggttcgtgcacacagcccagcttggagcgaacgacctacaccgaactgagatacctacagcgtgagctatgagaaagcgccacgcttcccgaagggagaaaggcggacaggtatccggtaagcggcagggtcggaacaggagagcgcacgagggagcttccagggggaaacgcctggtatctttatagtcctgtcgggtttcgccacctctgacttgagcgtcgatttttgtgatgctcgtcaggggggcggagcctatggaaaaacgccagcaacgcggcctttttacggttcctggccttttgctggccttttgctcacatgt

SEQ ID NO: 39 - DNA, 6909 bp, synthetic construct
  source 1..6909: mol_type = other DNA
cctgcaggcagctgcgcgctcgctcgctcactgaggccgcccgggcgtcgggcgacctttggtcgcccggcctcagtgagcgagcgagcgcgcagagagggagtggccaactccatcactaggggttcctgcggcctctagactcgaggcgttgacattgattattgactagttattaatagtaatcaattacggggtcattagttcatagcccatatatggagttccgcgttacataacttacggtaaatggcccgcctggctgaccgcccaacgacccccgcccattgacgtcaataatgacgtatgttcccatagtaacgccaatagggactttccattgacgtcaatgggtggagtatttacggtaaactgcccacttggcagtacatcaagtgtatcatatgccaagtacgccccctattgacgtcaatgacggtaaatggcccgcctggcattatgcccagtacatgaccttatgggactttcctacttggcagtacatctacgtattagtcatcgctattaccatggtgatgcggttttggcagtacatcaatgggcgtggatagcggtttgactcacggggatttccaagtctccaccccattgacgtcaatgggagtttgttttggcaccaaaatcaacgggactttccaaaatgtcgtaacaactccgccccattgacgcaaatgggcggtaggcgtgtacggtgggaggtctatataagcagagctctctggctaactaccggtgccaccatgccggcagctaagaaaaagaaactggatggcagcgtcgacatgatgggcaacaagaagagcgtggccaaggccaacggcctgaagagcaccttcgtgctgggcgagaacaccgcctacatgaccagcttcggcagaggcaacgccgcccagcccgagaagcacatcagagacgccaccgtgaccgacatccagcacaccttcagagccaagaccgacggcggcagaaccgtgcacatcgagggcagagtgggcgccagcgacgtgctgctgcccgacgccgccaaccagctgcacgccaaggacgccgtggagcagatgtacttcggcaaggccttcagcgacaacatccacatccagatcgcctacaacatcatggacatcaagaagatcttcggcgtgtacgccaacatcatcgtgcacaccgtgaacaacctgtgctgcgacggcgacaagcaggacgacttcctgggcatgttcaagacccagaacagataccaggtggccgcctgggcccacaagatcgtgagcctgcacctggtgaagaacgagctgagaggcggcggcttcttcatggaccaggaggtgtggagagcccacgtgagaaccgacttcaagagcctgaacctggccgtgaacgccttcatgaagaagtacccccagaagtacccctactggagcgtgaagatcgtgagcgacttcatcgtgcaggagatgggcatcaagaacaaggtgatcctggagaaggccgccgagagctacgccgagttcgagacagtggccaagagactggagaagagcgcctactacttcagcgacatcttcgccggcaaggacggcaagttcgacgagcagaaggccttcgacctgctgagagtgctgggcatgatgagacaggaggccttccacgagaagaacagcagcgccagctggctgtacaacctggacgccgaggccgacgaggacatcaaggccgccctgagaaccgtggtggacaccaaggtgaacggcatcaacaccaacttcgccaagcagaacaaggtgaacctgctggtgctgcaggagatctacccccagaagagcaaggccgacctggtgagagagtactacgacttcagcgtgagaaaggccttcaagaacctgggcttcagcgtgaaaaccctgagagagacaatgtgcgccttcgacgccgccagcgtgatcaccgacaagcagtacgacaccgtgagaggcaagctgtacagcctgttcgacttcgtgatctacaactactgcctggagaacgaggccgtgtgcaacgccttcgtggaggagctgagagccaacctggaccccgagaacaagaccgccctgtaccagaccctggccgagaaggtgtgggccgagatcggcgacatcgtgctgcagagaatcctgccccagatgcacgccaagaagatccaggagagaagcaaggagacagacgccgagacagtggagatgcagggctacgtgcaggcccccaaggacctgagcctgttcagcaaggccgtgtactgcatcagcatgttcctggacggcaaggagatcaacagcttcctgagcgccctgatcaacaagttcgagaacatcagcagcctgtgcgccgtgctggcctacaacggcctggagcccgagttcgtggcccccttcaccttcttcgccgacagccaggccatcgccgaggacctgagatacatcaagagcatcgccagaatgagcaagggcaagaaggccaccaaggacagccccgtgaccgtgaaggagatgcagtacttcgacgccgccgccgtgctgggcgagacagacaccgagaaggtgaaggccgccttccacctgggcgacaagagcgccagcaccgccgacaaggccttcagaaacttcgtggtgaacaacgtgatcaacagcaacagattcgtgtacgtggtgagattcatcaaccccaagaacgccagagagatcatgcagaacagagccctgatcgccttcgtgctgaaggacatcccccagagccagctggtgagatactgcggcaccgccggcatcgcctgcaacgccgacgagcccaacaccgaggccatggtgaacgccctggccgacatgctgctgcaggtgagattcgacgccttcagcaacgtgcagcagaaggtgaaggccgacagcgccgaggccgtgcagaaggagaagtacaaggccatcatcggcctgtacctgaccgtgctgtacctgctggtgaaaaccctggtgaagatcaacatgaactacgccatcgccttcggcatcctggagagagactgccagatcatgaaccagaagcacggcaagaaccccaagagagacagagacgccttctacatgagagagcagcagaacaagcagtacgtgtacaacgccagagccatcaccgagctgttcatcgagaacggctggctgaacaagagagtgcagaagagcgtggagaacaacgccgccctgtacagcgacgaggccttctacaagtacagaaacctggtggcccacctgaacgtgatcagcgccctgcccaagtacgccaagaacatcaccaaggtgaagagcctgttcgacgtgtaccactacatcctgttcctgagcctgtgcgaggacaagtacagcaacctgcccgaggccgtgaccaagagcctgtgcaagaacggcaagaccatgctggagaacgccagagagtaccagaccgtgtgcaaggacttcctgtacggcctgaacacccccttcgcctacaacgccgccagatacatcaacctgagcaacagagagaagttcctggccggcttcggcaagacaggcggcggccccggcggcggcgccgccgccggcagcggcagccctaagaaaaaacgaaaagttggcagcggaagcaaaaggccggcggccacgaaaaaggccggccaggcaaaaaagaaaaagctcgagtacccatacgatgttccagattacgcttgagaattccccttgagcatctgacttctggctaataaaggaaatttattttcattgcaatagtgtgttggaattttttgtgtctctcaggtaccgagggcctatttcccatgattccttcatatttgcatatacgatacaaggctgttagagagataattggaattaatttgactgtaaacacaaagatattagtacaaaatacgtgacgtagaaagtaataatttcttgggtagtttgcagttttaaaattatgttttaaaatggactatcatatgcttaccgtaacttgaaagtatttcgatttcttggctttatatatcttgtggaaaggacgaaacaccgggttttacacccgtgtaaaactacacagttctaaaacggagaccacggcaggtctcattttttgcggccgcaggaacccctagtgatggagttggccactccctctctgcgcgctcgctcgctcactgaggccgggcgaccaaaggtcgcccgacgcccgggctttgcccgggcggcctcagtgagcgagcgagcgcgcagctgcctgcaggggcgcctgatgcggtattttctccttacgcatctgtgcggtatttcacaccgcatacgtcaaagcaaccatagtacgcgccctgtagcggcgcattaagcgcggcgggtgtggtggttacgcgcagcgtgaccgctacacttgccagcgccttagcgcccgctcctttcgctttcttcccttcctttctcgccacgttcgccggctttccccgtcaagctctaaatcgggggctccctttagggttccgatttagtgctttacggcacctcgaccccaaaaaacttgatttgggtgatggttcacgtagtgggccatcgccctgatagacggtttttcgccctttgacgttggagtccacgttctttaatagtggactcttgttccaaactggaacaacactcaactctatctcgggctattcttttgatttataagggattttgccgatttcggtctattggttaaaaaatgagctgatttaacaaaaatttaacgcgaattttaacaaaatattaacgtttacaattttatggtgcactctcagtacaatctgctctgatgccgcatagttaagccagccccgacacccgccaacacccgctgacgcgccctgacgggcttgtctgctcccggcatccgcttacagacaagctgtgaccgtctccgggagctgcatgtgtcagaggttttcaccgtcatcaccgaaacgcgcgagacgaaagggcctcgtgatacgcctatttttataggttaatgtcatgataataatggtttcttagacgtcaggtggcacttttcggggaaatgtgcgcggaacccctatttgtttatttttctaaatacattcaaatatgtatccgctcatgagacaataaccctgataaatgcttcaataatattgaaaaaggaagagtatgagtattcaacatttccgtgtcgcccttattcccttttttgcggcattttgccttcctgtttttgctcacccagaaacgctggtgaaagtaaaagatgctgaagatcagttgggtgcacgagtgggttacatcgaactggatctcaacagcggtaagatccttgagagttttcgccccgaagaacgttttccaatgatgagcacttttaaagttctgctatgtggcgcggtattatcccgtattgacgccgggcaagagcaactcggtcgccgcatacactattctcagaatgacttggttgagtactcaccagtcacagaaaagcatcttacggatggcatgacagtaagagaattatgcagtgctgccataaccatgagtgataacactgcggccaacttacttctgacaacgatcggaggaccgaaggagctaaccgcttttttgcacaacatgggggatcatgtaactcgccttgatcgttgggaaccggagctgaatgaagccataccaaacgacgagcgtgacaccacgatgcctgtagcaatggcaacaacgttgcgcaaactattaactggcgaactacttactctagcttcccggcaacaattaatagactggatggaggcggataaagttgcaggaccacttctgcgctcggcccttccggctggctggtttattgctgataaatctggagccggtgagcgtggaagccgcggtatcattgcagcactggggccagatggtaagccctcccgtatcgtagttatctacacgacggggagtcaggcaactatggatgaacgaaatagacagatcgctgagataggtgcctcactgattaagcattggtaactgtcagaccaagtttactcatatatactttagattgatttaaaacttcatttttaatttaaaaggatctaggtgaagatcctttttgataatctcatgaccaaaatcccttaacgtgagttttcgttccactgagcgtcagaccccgtagaaaagatcaaaggatcttcttgagatcctttttttctgcgcgtaatctgctgcttgcaaacaaaaaaaccaccgctaccagcggtggtttgtttgccggatcaagagctaccaactctttttccgaaggtaactggcttcagcagagcgcagataccaaatactgttcttctagtgtagccgtagttaggccaccacttcaagaactctgtagcaccgcctacatacctcgctctgctaatcctgttaccagtggctgctgccagtggcgataagtcgtgtcttaccgggttggactcaagacgatagttaccggataaggcgcagcggtcgggctgaacggggggttcgtgcacacagcccagcttggagcgaacgacctacaccgaactgagatacctacagcgtgagctatgagaaagcgccacgcttcccgaagggagaaaggcggacaggtatccggtaagcggcagggtcggaacaggagagcgcacgagggagcttccagggggaaacgcctggtatctttatagtcctgtcgggtttcgccacctctgacttgagcgtcgatttttgtgatgctcgtcaggggggcggagcctatggaaaaacgccagcaacgcggcctttttacggttcctggccttttgctggccttttgctcacatgt

SEQ ID NO: 40 - DNA, 7102 bp, synthetic construct
  source 1..7102: mol_type = other DNA
cctgcaggcagctgcgcgctcgctcgctcactgaggccgcccgggcgtcgggcgacctttggtcgcccggcctcagtgagcgagcgagcgcgcagagagggagtggccaactccatcactaggggttcctgcggcctctagactcgaggcgttgacattgattattgactagttattaatagtaatcaattacggggtcattagttcatagcccatatatggagttccgcgttacataacttacggtaaatggcccgcctggctgaccgcccaacgacccccgcccattgacgtcaataatgacgtatgttcccatagtaacgccaatagggactttccattgacgtcaatgggtggagtatttacggtaaactgcccacttggcagtacatcaagtgtatcatatgccaagtacgccccctattgacgtcaatgacggtaaatggcccgcctggcattatgcccagtacatgaccttatgggactttcctacttggcagtacatctacgtattagtcatcgctattaccatggtgatgcggttttggcagtacatcaatgggcgtggatagcggtttgactcacggggatttccaagtctccaccccattgacgtcaatgggagtttgttttggcaccaaaatcaacgggactttccaaaatgtcgtaacaactccgccccattgacgcaaatgggcggtaggcgtgtacggtgggaggtctatataagcagagctctctggctaactaccggtgccaccatgagccccaagaagaagagaaaggtggaggccagcatcgaaaaaaaaaagtccttcgccaagggcatgggcgtgaagtccacactcgtgtccggctccaaagtgtacatgacaaccttcgccgaaggcagcgacgccaggctggaaaagatcgtggagggcgacagcatcaggagcgtgaatgagggcgaggccttcagcgctgaaatggccgataaaaacgccggctataagatcggcaacgccaaattcagccatcctaagggctacgccgtggtggctaacaaccctctgtatacaggacccgtccagcaggatatgctcggcctgaaggaaactctggaaaagaggtacttcggcgagagcgctgatggcaatgacaatatttgtatccaggtgatccataacatcctggacattgaaaaaatcctcgccgaatacattaccaacgccgcctacgccgtcaacaatatctccggcctggataaggacattattggattcggcaagttctccacagtgtatacctacgacgaattcaaagaccccgagcaccatagggccgctttcaacaataacgataagctcatcaacgccatcaaggcccagtatgacgagttcgacaacttcctcgataaccccagactcggctatttcggccaggcctttttcagcaaggagggcagaaattacatcatcaattacggcaacgaatgctatgacattctggccctcctgagcggactgaggcactgggtggtccataacaacgaagaagagtccaggatctccaggacctggctctacaacctcgataagaacctcgacaacgaatacatctccaccctcaactacctctacgacaggatcaccaatgagctgaccaactccttctccaagaactccgccgccaacgtgaactatattgccgaaactctgggaatcaaccctgccgaattcgccgaacaatatttcagattcagcattatgaaagagcagaaaaacctcggattcaatatcaccaagctcagggaagtgatgctggacaggaaggatatgtccgagatcaggaaaaatcataaggtgttcgactccatcaggaccaaggtctacaccatgatggactttgtgatttataggtattacatcgaagaggatgccaaggtggctgccgccaataagtccctccccgataatgagaagtccctgagcgagaaggatatctttgtgattaacctgaggggctccttcaacgacgaccagaaggatgccctctactacgatgaagctaatagaatttggagaaagctcgaaaatatcatgcacaacatcaaggaatttaggggaaacaagacaagagagtataagaagaaggacgcccctagactgcccagaatcctgcccgctggccgtgatgtttccgccttcagcaaactcatgtatgccctgaccatgttcctggatggcaaggagatcaacgacctcctgaccaccctgattaataaattcgataacatccagagcttcctgaaggtgatgcctctcatcggagtcaacgctaagttcgtggaggaatacgcctttttcaaagactccgccaagatcgccgatgagctgaggctgatcaagtccttcgctagaatgggagaacctattgccgatgccaggagggccatgtatatcgacgccatccgtattttaggaaccaacctgtcctatgatgagctcaaggccctcgccgacaccttttccctggacgagaacggaaacaagctcaagaaaggcaagcacggcatgagaaatttcattattaataacgtgatcagcaataaaaggttccactacctgatcagatacggtgatcctgcccacctccatgagatcgccaaaaacgaggccgtggtgaagttcgtgctcggcaggatcgctgacatccagaaaaaacagggccagaacggcaagaaccagatcgacaggtactacgaaacttgtatcggaaaggataagggcaagagcgtgagcgaaaaggtggacgctctcacaaagatcatcaccggaatgaactacgaccaattcgacaagaaaaggagcgtcattgaggacaccggcagggaaaacgccgagagggagaagtttaaaaagatcatcagcctgtacctcaccgtgatctaccacatcctcaagaatattgtcaatatcaacgccaggtacgtcatcggattccattgcgtcgagcgtgatgctcaactgtacaaggagaaaggctacgacatcaatctcaagaaactggaagagaagggattcagctccgtcaccaagctctgcgctggcattgatgaaactgcccccgataagagaaaggacgtggaaaaggagatggctgaaagagccaaggagagcattgacagcctcgagagcgccaaccccaagctgtatgccaattacatcaaatacagcgacgagaagaaagccgaggagttcaccaggcagattaacagggagaaggccaaaaccgccctgaacgcctacctgaggaacaccaagtggaatgtgatcatcagggaggacctcctgagaattgacaacaagacatgtaccctgttcagaaacaaggccgtccacctggaagtggccaggtatgtccacgcctatatcaacgacattgccgaggtcaattcctacttccaactgtaccattacatcatgcagagaattatcatgaatgagaggtacgagaaaagcagcggaaaggtgtccgagtacttcgacgctgtgaatgacgagaagaagtacaacgataggctcctgaaactgctgtgtgtgcctttcggctactgtatccccaggtttaagaacctgagcatcgaggccctgttcgataggaacgaggccgccaagttcgacaaggagaaaaagaaggtgtccggcaattccggatccggacctaagaaaaagaggaaggtggcggccgcttacccatacgatgttccagattacgcttgaggtaccctagagctcgctgatcagcctcgactgtgccttctagttgccagccatctgttgtttgcccctcccccgtgccttccttgaccctggaaggtgccactcccactgtcctttcctaataaaatgaggaaattgcatcgcattgtctgagtaggtgtcattctattctggggggtggggtggggcaggacagcaagggggaggattgggaagagaatagcaggcatgctggggagagggcctatttcccatgattccttcatatttgcatatacgatacaaggctgttagagagataattggaattaatttgactgtaaacacaaagatattagtacaaaatacgtgacgtagaaagtaataatttcttgggtagtttgcagttttaaaattatgttttaaaatggactatcatatgcttaccgtaacttgaaagtatttcgatttcttggctttatatatcttgtggaaaggacgaaacaccgcaagtaaacccctaccaactggtcggggtttgaaacgggtcttcgagaagacctcaagtaaacccctaccaactggtcggggtttgaaactttttttcccgggaatggccgcaggaacccctagtgatggagttggccactccctctctgcgcgctcgctcgctcactgaggccgggcgaccaaaggtcgcccgacgcccgggctttgcccgggcggcctcagtgagcgagcgagcgcgcagctgcctgcaggggcgcctgatgcggtattttctccttacgcatctgtgcggtatttcacaccgcatacgtcaaagcaaccatagtacgcgccctgtagcggcgcattaagcgcggcgggtgtggtggttacgcgcagcgtgaccgctacacttgccagcgccctagcgcccgctcctttcgctttcttcccttcctttctcgccacgttcgccggctttccccgtcaagctctaaatcgggggctccctttagggttccgatttagtgctttacggcacctcgaccccaaaaaacttgatttgggtgatggttcacgtagtgggccatcgccctgatagacggtttttcgccctttgacgttggagtccacgttctttaatagtggactcttgttccaaactggaacaacactcaaccctatctcgggctattcttttgatttataagggattttgccgatttcggcctattggttaaaaaatgagctgatttaacaaaaatttaacgcgaattttaacaaaatattaacgtttacaattttatggtgcactctcagtacaatctgctctgatgccgcatagttaagccagccccgacacccgccaacacccgctgacgcgccctgacgggcttgtctgctcccggcatccgcttacagacaagctgtgaccgtctccgggagctgcatgtgtcagaggttttcaccgtcatcaccgaaacgcgcgagacgaaagggcctcgtgatacgcctatttttataggttaatgtcatgataataatggtttcttagacgtcaggtggcacttttcggggaaatgtgcgcggaacccctatttgtttatttttctaaatacattcaaatatgtatccgctcatgagacaataaccctgataaatgcttcaataatattgaaaaaggaagagtatgagtattcaacatttccgtgtcgcccttattcccttttttgcggcattttgccttcctgtttttgctcacccagaaacgctggtgaaagtaaaagatgctgaagatcagttgggtgcacgagtgggttacatcgaactggatctcaacagcggtaagatccttgagagttttcgccccgaagaacgttttccaatgatgagcacttttaaagttctgctatgtggcgcggtattatcccgtattgacgccgggcaagagcaactcggtcgccgcatacactattctcagaatgacttggttgagtactcaccagtcacagaaaagcatcttacggatggcatgacagtaagagaattatgcagtgctgccataaccatgagtgataacactgcggccaacttacttctgacaacgatcggaggaccgaaggagctaaccgcttttttgcacaacatgggggatcatgtaactcgccttgatcgttgggaaccggagctgaatgaagccataccaaacgacgagcgtgacaccacgatgcctgtagcaatggcaacaacgttgcgcaaactattaactggcgaactacttactctagcttcccggcaacaattaatagactggatggaggcggataaagttgcaggaccacttctgcgctcggcccttccggctggctggtttattgctgataaatctggagccggtgagcgtggaagccgcggtatcattgcagcactggggccagatggtaagccctcccgtatcgtagttatctacacgacggggagtcaggcaactatggatgaacgaaatagacagatcgctgagataggtgcctcactgattaagcattggtaactgtcagaccaagtttactcatatatactttagattgatttaaaacttcatttttaatttaaaaggatctaggtgaagatcctttttgataatctcatgaccaaaatcccttaacgtgagttttcgttccactgagcgtcagaccccgtagaaaagatcaaaggatcttcttgagatcctttttttctgcgcgtaatctgctgcttgcaaacaaaaaaaccaccgctaccagcggtggtttgtttgccggatcaagagctaccaactctttttccgaaggtaactggcttcagcagagcgcagataccaaatactgtccttctagtgtagccgtagttaggccaccacttcaagaactctgtagcaccgcctacatacctcgctctgctaatcctgttaccagtggctgctgccagtggcgataagtcgtgtcttaccgggttggactcaagacgatagttaccggataaggcgcagcggtcgggctgaacggggggttcgtgcacacagcccagcttggagcgaacgacctacaccgaactgagatacctacagcgtgagctatgagaaagcgccacgcttcccgaagggagaaaggcggacaggtatccggtaagcggcagggtcggaacaggagagcgcacgagggagcttccagggggaaacgcctggtatctttatagtcctgtcgggtttcgccacctctgacttgagcgtcgatttttgtgatgctcgtcaggggggcggagcctatggaaaaacgccagcaacgcggcctttttacggttcctggccttttgctggccttttgctcacatgt

SEQ ID NO: 41 - DNA, 9363 bp, synthetic construct
  source 1..9363: mol_type = other DNA
gtcgacggatcgggagatctcccgatcccctatggtgcactctcagtacaatctgctctgatgccgcatagttaagccagtatctgctccctgcttgtgtgttggaggtcgctgagtagtgcgcgagcaaaatttaagctacaacaaggcaaggcttgaccgacaattgcatgaagaatctgcttagggttaggcgttttgcgctgcttcgcgatgtacgggccagatatacgcgttgacattgattattgactagttattaatagtaatcaattacggggtcattagttcatagcccatatatggagttccgcgttacataacttacggtaaatggcccgcctggctgaccgcccaacgacccccgcccattgacgtcaataatgacgtatgttcccatagtaacgccaatagggactttccattgacgtcaatgggtggagtatttacggtaaactgcccacttggcagtacatcaagtgtatcatatgccaagtacgccccctattgacgtcaatgacggtaaatggcccgcctggcattatgcccagtacatgaccttatgggactttcctacttggcagtacatctacgtattagtcatcgctattaccatggtgatgcggttttggcagtacatcaatgggcgtggatagcggtttgactcacggggatttccaagtctccaccccattgacgtcaatgggagtttgttttggcaccaaaatcaacgggactttccaaaatgtcgtaacaactccgccccattgacgcaaatgggcggtaggcgtgtacggtgggaggtctatagaccagatctgagcctgggagctctctggctaactagggaacccactgcttaagcctcaataaagcttgccttgagtgcttcaagtagtgtgtgcccgtctgttgtgtgactctggtaactagagatccctcagacccttttagtcagtgtggaaaatctctagcagtggcgcccgaacagggacttgaaagcgaaagggaaaccagaggagctctctcgacgcaggactcggcttgctgaagcgcgcacggcaagaggcgaggggcggcgactggtgagtacgccaaaaattttgactagcggaggctagaaggagagagatgggtgcgagagcgtcagtattaagcgggggagaattagatcgcgatgggaaaaaattcggttaaggccagggggaaagaaaaaatataaataaacatatagtatgggcaagcagggagctagaacgattcgcagttaatcctggcctgttagaaacatcagaaggctgtagacaaatactgggacagctacaaccatcccttcagacaggatcagaagaacttagatcattatataatacagtagcaaccctctattgtgtgcatcaaaggatagagataaaagacaccaaggaagctttagacaagatagaggaagagcaaaacaaaagtaagaccaccgcacagcaagcggccggccgcgctgatcttcagacctggaggaggagatatgagggacaattggagaagtgaattatataaatataaagtagtaaaaattgaaccattaggagtagcacccaccaaggcaaagagaagagtggtgcagagagaaaaaagagcagtgggaataggagctttgttccttgggttcttgggagcagcaggaagcactatgggcgcagcgtcaatgacgctgacggtacaggccagacaattattgtctggtatagtgcagcagcagaacaatttgctgagggctattgaggcgcaacagcatctgttgcaactcacagtctggggcatcaagcagctccaggcaagaatcctggctgtggaaagatacctaaaggatcaacagctcctggggatttggggttgctctggaaaactcatttgcaccactgctgtgccttggaatgctagttggagtaataaatctctggaacagatttggaatcacacgacctggatggagtgggacagagaaattaacaattacacaagcttaatacactccttaattgaagaatcgcaaaaccagcaagaaaagaatgaacaagaattattggaattagataaatgggcaagtttgtggaattggtttaacataacaaattggctgtggtatataaaattattcataatgatagtaggaggcttggtaggtttaagaatagtttttgctgtactttctatagtgaatagagttaggcagggatattcaccattatcgtttcagacccacctcccaaccccgaggggacccgacaggcccgaaggaatagaagaagaaggtggagagagagacagagacagatccattcgattagtgaacggatcggcactgcgtgcgccaattctgcagacaaatggcagtattcatccacaattttaaaagaaaaggggggattggggggtacagtgcaggggaaagaatagtagacataatagcaacagacatacaaactaaagaattacaaaaacaaattacaaaaattcaaaattttcgggtttattacagggacagcagagatccagtttggttagtaccgggcccgctctagcgtcgaggagcttggcccattgcatacgttgtatccatatcataatatgtacatttatattggctcatgtccaacattaccgccatgttgacattgattattgactagttattaatagtaatcaattacggggtcattagttcatagcccatatatggagttccgcgttacataacttacggtaaatggcccgcctggctgaccgcccaacgacccccgcccattgacgtcaataatgacgtatgttcccatagtaacgccaatagggactttccattgacgtcaatgggtggagtatttacggtaaactgcccacttggcagtacatcaagtgtatcatatgccaagtacgccccctattgacgtcaatgacggtaaatggcccgcctggcattatgcccagtacatgaccttatgggactttcctacttggcagtacatctacgtattagtcatcgctattaccatggtgatgcggttttggcagtacatcaatgggcgtggatagcggtttgactcacggggatttccaagtctccaccccattgacgtcaatgggagtttgttttggcaccaaaatcaacgggactttccaaaatgtcgtaacaactccgccccattgacgcaaatgggcggtaggcgtgtacggtgggaggtctatataagcagagctcgtttagtgaaccgtcagatcgcctggagacgccatccacgctgttttgacctccatagaagacaccgggaccgatccagcctccgcggccccgaattcgccaccatggccagcgagttcaagaagaagctcttctggagggcagtggtggccgagttcctggccacgaccctctttgtcttcatcagcatcggttctgccctgggcttcaaatacccggtggggaacaaccagacggcggtccaggacaacgtgaaggtgtcgctggccttcgggctgagcatcgccacgctggcgcagagtgtgggccacatcagcggcgcccacctcaacccggctgtcacactggggctgctgctcagctgccagatcagcatcttccgtgccctcatgtacatcatcgcccagtgcgtgggggccatcgtcgccaccgccatcctctcaggcatcacctcctccctgactgggaactcgcttggccgcaatgacctggctgatggtgtgaactcgggccagggcctgggcatcgagatcatcgggaccctccagctggtgctatgcgtgctggctactaccgaccggaggcgccgtgaccttggtggctcagccccccttgccatcggcctctctgtagcccttggacacctcctggctattgactacactggctgtgggattaaccctgctcggtcctttggctccgcggtgatcacacacaacttcagcaaccactggattttctgggtggggccattcatcgggggagccctggctgtactcatctacgacttcatcctggccccacgcagcagtgacctcacagaccgcgtgaaggtgtggaccagcggccaggtggaggagtatgacctggatgccgacgacatcaactccagggtggagatgaagcccaaatacccatacgatgttccagattacgctggatccgctagcggcagtggagagggcagaggaagtctgctaacatgcggtgacgtcgaggagaatcctggcccagtgagcaagggcgaggagctgttcaccggggtggtgcccatcctggtcgagctggacggcgacgtaaacggccacaagttcagcgtgtccggcgagggcgagggcgatgccacctacggcaagctgaccctgaagttcatctgcaccaccggcaagctgcccgtgccctggcccaccctcgtgaccaccctgacctacggcgtgcagtgcttcagccgctaccccgaccacatgaagcagcacgacttcttcaagtccgccatgcccgaaggctacgtccaggagcgcaccatcttcttcaaggacgacggcaactacaagacccgcgccgaggtgaagttcgagggcgacaccctggtgaaccgcatcgagctgaagggcatcgacttcaaggaggacggcaacatcctggggcacaagctggagtacaactacaacagccacaacgtctatatcatggccgacaagcagaagaacggcatcaaggtgaacttcaagatccgccacaacatcgaggacggcagcgtgcagctcgccgaccactaccagcagaacacccccatcggcgacggccccgtgctgctgcccgacaaccactacctgagcacccagtccgccctgagcaaagaccccaacgagaagcgcgatcacatggtcctgctggagttcgtgaccgccgccgggatcactctcggcatggacgagctgtacaagtaaggatcctaggcggccgcgcatgccctgcaggtgatctatcgatcggccggcccctctccctccccccccccctaacgttactggccgaagccgcttggaataaggccggtgtgcgtttgtctatatgttattttccaccatattgccgtcttttggcaatgtgagggcccggaaacctggccctgtcttcttgacgagcattcctaggggtctttcccctctcgccaaaggaatgcaaggtctgttgaatgtcgtgaaggaagcagttcctctggaagcttcttgaagacaaacaacgtctgtagcgaccctttgcaggcagcggaaccccccacctggcgacaggtgcctctgcggccaaaagccacgtgtataagatacacctgcaaaggcggcacaaccccagtgccacgttgtgagttggatagttgtggaaagagtcaaatggctctcctcaagcgtattcaacaaggggctgaaggatgcccagaaggtaccccattgtatgggatctgatctggggcctcggtacacatgctttacatgtgtttagtcgaggttaaaaaaacgtctaggccccccgaaccacggggacgtggttttcctttgaaaaacacgatgataatatggccacaaccgggccggatatcacgcgtgatctgatcagcacgtgttgacaattaatcatcggcatagtatatcggcatagtataatacgacaaggtgaggaactaaaccatggccaagcctttgtctcaagaagaatccaccctcattgaaagagcaacggctacaatcaacagcatccccatctctgaagactacagcgtcgccagcgcagctctctctagcgacggccgcatcttcactggtgtcaatgtatatcattttactgggggaccttgtgcagaactcgtggtgctgggcactgctgctgctgcggcagctggcaacctgacttgtatcgtcgcgatcggaaatgagaacaggggcatcttgagcccctgcggacggtgccgacaggtgcttctcgatctgcatcctgggatcaaagccatagtgaaggacagtgatggacagccgacggcagttgggattcgtgaattgctgccctctggttatgtgtgggagggctaagcaatgcatacatgtgtttaaacctcgacttaattaagtcgagggtcgacggtatcgataagctcgcttcacgagatcatgtttaagggttccggttccactaggtacaattcgatatcaagcttatcgataatcaacctctggattacaaaatttgtgaaagattgactggtattcttaactatgttgctccttttacgctatgtggatacgctgctttaatgcctttgtatcatgctattgcttcccgtatggctttcattttctcctccttgtataaatcctggttgctgtctctttatgaggagttgtggcccgttgtcaggcaacgtggcgtggtgtgcactgtgtttgctgacgcaacccccactggttggggcattgccaccacctgtcagctcctttccgggactttcgctttccccctccctattgccacggcggaactcatcgccgcctgccttgcccgctgctggacaggggctcggctgttgggcactgacaattccgtggtgttgtcggggaaatcatcgtcctttccttggctgctcgcctgtgttgccacctggattctgcgcgggacgtccttctgctacgtcccttcggccctcaatccagcggaccttccttcccgcggcctgctgccggctctgcggcctcttccgcgtcttcgccttcgccctcagacgagtcggatctccctttgggccgcctccccgcatcgataccgtcgacctcgatcgagacctagaaaaacatggagcaatcacaagtagcaatacagcagctaccaatgctgattgtgcctggctagaagcacaagaggaggaggaggtgggttttccagtcacacctcaggtacctttaagaccaatgacttacaaggcagctgtagatcttagccactttttaaaagaaaaggggggactggaagggctaattcactcccaacgaagacaagatatccttgatctgtggatctaccacacacaaggctacttccctgattggcagaactacacaccagggccagggatcagatatccactgacctttggatggtgctacaagctagtaccagttgagcaagagaaggtagaagaagccaatgaaggagagaacacccgcttgttacaccctgtgagcctgcatgggatggatgacccggagagagaagtattagagtggaggtttgacagccgcctagcatttcatcacatggcccgagagctgcatccggactgtactgggtctctctggttagaccagatctgagcctgggagctctctggctaactagggaacccactgcttaagcctcaataaagcttgccttgagtgcttcaagtagtgtgtgcccgtctgttgtgtgactctggtaactagagatccctcagacccttttagtcagtgtggaaaatctctagcagcatgtgagcaaaaggccagcaaaaggccaggaaccgtaaaaaggccgcgttgctggcgtttttccataggctccgcccccctgacgagcatcacaaaaatcgacgctcaagtcagaggtggcgaaacccgacaggactataaagataccaggcgtttccccctggaagctccctcgtgcgctctcctgttccgaccctgccgcttaccggatacctgtccgcctttctcccttcgggaagcgtggcgctttctcatagctcacgctgtaggtatctcagttcggtgtaggtcgttcgctccaagctgggctgtgtgcacgaaccccccgttcagcccgaccgctgcgccttatccggtaactatcgtcttgagtccaacccggtaagacacgacttatcgccactggcagcagccactggtaacaggattagcagagcgaggtatgtaggcggtgctacagagttcttgaagtggtggcctaactacggctacactagaagaacagtatttggtatctgcgctctgctgaagccagttaccttcggaaaaagagttggtagctcttgatccggcaaacaaaccaccgctggtagcggtggtttttttgtttgcaagcagcagattacgcgcagaaaaaaaggatctcaagaagatcctttgatcttttctacggggtctgacgctcagtggaacgaaaactcacgttaagggattttggtcatgagattatcaaaaaggatcttcacctagatccttttaaattaaaaatgaagttttaaatcaatctaaagtatatatgagtaaacttggtctgacagttaccaatgcttaatcagtgaggcacctatctcagcgatctgtctatttcgttcatccatagttgcctgactccccgtcgtgtagataactacgatacgggagggcttaccatctggccccagtgctgcaatgataccgcgagacccacgctcaccggctccagatttatcagcaataaaccagccagccggaagggccgagcgcagaagtggtcctgcaactttatccgcctccatccagtctattaattgttgccgggaagctagagtaagtagttcgccagttaatagtttgcgcaacgttgttgccattgctacaggcatcgtggtgtcacgctcgtcgtttggtatggcttcattcagctccggttcccaacgatcaaggcgagttacatgatcccccatgttgtgcaaaaaagcggttagctccttcggtcctccgatcgttgtcagaagtaagttggccgcagtgttatcactcatggttatggcagcactgcataattctcttactgtcatgccatccgtaagatgcttttctgtgactggtgagtactcaaccaagtcattctgagaatagtgtatgcggcgaccgagttgctcttgcccggcgtcaatacgggataataccgcgccacatagcagaactttaaaagtgctcatcattggaaaacgttcttcggggcgaaaactctcaaggatcttaccgctgttgagatccagttcgatgtaacccactcgtgcacccaactgatcttcagcatcttttactttcaccagcgtttctgggtgagcaaaaacaggaaggcaaaatgccgcaaaaaagggaataagggcgacacggaaatgttgaatactcatactcttcctttttcaatattattgaagcatttatcagggttattgtctcatgagcggatacatatttgaatgtatttagaaaaataaacaaataggggttccgcgcacatttccccgaaaagtgccacctgac

SEQ ID NO: 42 - RNA, 20 nt, synthetic construct
  source 1..20: mol_type = other RNA
gaagacaaagagggtcgtgg

SEQ ID NO: 43 - RNA, 30 nt, synthetic construct
  source 1..30: mol_type = other RNA
gtggttggagaactggatgtagatgggctg

SEQ ID NO: 44 - DNA, 34 bp, synthetic construct
  source 1..34: mol_type = other DNA
caccgtggttggagaactggatgtagatgggctg

SEQ ID NO: 45 - DNA, 34 bp, synthetic construct
  source 1..34: mol_type = other DNA
caaccagcccatctacatccagttctccaaccac

SEQ ID NO: 46 - DNA, 34 bp, synthetic construct
  source 1..34: mol_type = other DNA
aaacgtggttggagaactggatgtagatgggctg

SEQ ID NO: 47 - DNA, 34 bp, synthetic construct
  source 1..34: mol_type = other DNA
aaaacagcccatctacatccagttctccaaccac

SEQ ID NO: 48 - DNA, 34 bp, synthetic construct
  source 1..34: mol_type = other DNA
cttgcagcccatctacatccagttctccaaccac

SEQ ID NO: 49 - DNA, 24 bp, synthetic construct
  source 1..24: mol_type = other DNA
caccgaagacaaagagggtcgtgg

SEQ ID NO: 50 - DNA, 24 bp, synthetic construct
  source 1..24: mol_type = other DNA
caacccacgaccctctttgtcttc

SEQ ID NO: 51 - DNA, 24 bp, synthetic construct
  source 1..24: mol_type = other DNA
aaacgaagacaaagagggtcgtgg

SEQ ID NO: 52 - DNA, 24 bp, synthetic construct
  source 1..24: mol_type = other DNA
aaaaccacgaccctctttgtcttc

SEQ ID NO: 53 - DNA, 24 bp, synthetic construct
  source 1..24: mol_type = other DNA
cttgccacgaccctctttgtcttc

SEQ ID NO: 54 - DNA, 22 bp, synthetic construct
  source 1..22: mol_type = other DNA
attgtcccagatatagccgttg

SEQ ID NO: 55 - DNA, 20 bp, synthetic construct
  source 1..20: mol_type = other DNA
gctgtcatttccgtttgctg

SEQ ID NO: 56 - DNA, 20 bp, synthetic construct
  source 1..20: mol_type = other DNA
gctcttctggagggcagtgg

SEQ ID NO: 57 - DNA, 21 bp, synthetic construct
  source 1..21: mol_type = other DNA
cagtgtgacagccgggttgag

SEQ ID NO: 58 - DNA, 20 bp, synthetic construct
  source 1..20: mol_type = other DNA
ccatggggaaggtgaaggtc

SEQ ID NO: 59 - DNA, 21 bp, synthetic construct
  source 1..21: mol_type = other DNA
gaaggggtcattgatggcaac

SEQ ID NO: 60 - protein, 1188 aa, synthetic construct
MKEQKKFSLQGVRHVCGSYFNMALNNYCRTLNGVFIKCKIKFALKEDDFPRSLSSLRKIFSSGPIMPQTEKKVAKMIASVDTAMKLKQQLFKHFPMLGPIMDKTISCMNHHKGSSVADAPLDLCMNAILNFGECLYHCRNFYTHFKPYNSPEDLKLQYDIQHIIALNLGTLFDVSRRIGKKREGLTPEELEFLTGKNRFNQVGKKFLERNDWYLKIEKPSDMKDYDKTILSDFGMVYLCSIFLAKNYALRLFDESKLFNKETIRNLFSEEQVRFLKEMLVIYRIRTPRGKQLDSHDSKQALAMDMLNELRKCPRPLYDVLSEEYKKRTFYVPVEHENEKTEEYVKMLRSDDRFPYFTLRYIDDMEKFSRIRFQIRLGSYRFKFYDKMNIDGTPRIRSLQKEINGFGRLSDMENKRKREWKDMFQATEEIDYEDQFGDYQTGVTQFVEDTADTKPYVTNHRAAYNVHSNHIGLIWNDADSIILQDDNKLFFPDLKIDENGKADIYQPSPKASLSVFDFPAMVFYMYLREKTEATKEFPSAEQLIINKYDHLVRFFKDISDGRFGPSENKNAFSKKLKEEYDLKTGEIPEKLLHWLSSESEEDPSEKYAKKLEEEIKLRRERVQRRLEKFNQDLREIRKKDSVPYGKKGHVNIRHSQLAKYLMRSIMEWQPTRNDGKNKLTGQNFNVMTAFLATLGYTSQVKDLRDLFSRANMLEGPNAHPFLKKVLNNNSIKDIQGFYRTYLVEELNQIEDKQRRIAKAKNVKDTVRQFPFAHFNRMRYQKRDEDYYRNLAKRYLNIGDNEKDKAVILLPDGMFTSYIYDLIMKLPENNEKMRINLASDVAHCNSSFLISRFFENIRNDYAQPFYREERTYELFSILNNKKVRNTLQPLFISPHDINIQLTEKEKDGKGRLILQKIDHFCKSITQKGNFNNVEEAKEATSRKLKHLITDCKNNERDIRRYKTQDMVIYLMARDILKDIIPDSEKDKYAKDRKLLLKDVCEEGFLRQAVKMEYEYSIEEKGKRTRTVKITHPNMSLKNYGEFHRLLNDERLKSLLQQLANMDEIDYTDLMGEFADYDQKRSEIFRLAQSIEKHLYEQNEQGLNDEKSDLFYHTRYNGKKIPRRNSFSSLLELIGEEESQMTETDKKQTISIRNAFGHNTYKVSLAEMNATELPNVAKTILKKMEELRNKL

SEQ ID NO: 61 - DNA, 3567 bp, synthetic construct
  source 1..3567: mol_type = other DNA
atgaaagaacaaaaaaaattttctctccaaggcgtaagacacgtctgtggtagttatttcaacatggctctcaacaattattgtcgaacgttgaatggagtattcatcaaatgtaaaattaaattcgcattgaaagaggatgattttccacgatcgttatcaagtttgaggaaaattttctcttctgggcctattatgcctcaaacagaaaaaaaagtggcaaagatgattgcttctgttgataccgccatgaagttaaaacagcagttattcaaacactttcccatgttaggtcccattatggataaaaccatcagttgcatgaaccaccataaaggctcttctgttgccgacgctcctcttgacctttgcatgaacgcaattcttaacttcggcgaatgcctttaccattgtaggaatttctatacgcatttcaaaccttacaacagtccagaagacctgaaactacaatatgacatccaacacattattgccttgaatcttggcaccttattcgatgtcagccggagaatcgggaaaaaacgcgaaggtctgacaccggaagagttggaattccttacaggtaaaaataggtttaaccaagtcgggaaaaaattccttgagcgtaacgactggtatttgaaaatagagaaaccatccgacatgaaagattatgacaagaccatattgtcagacttcggcatggtgtacctttgctccatctttcttgccaaaaactacgccctccgcctttttgatgagtcaaaattattcaacaaagaaacaataaggaatttattctctgaagaacaggttcgattccttaaggagatgcttgttatctatcgcatcaggacaccacgagggaagcaactagacagtcacgacagcaaacaagctttggccatggatatgctcaacgaactccgcaaatgcccaagacctctttacgatgtgctatccgaagaatataaaaagaggacattctatgtcccagtggagcatgaaaatgaaaagacagaagaatatgtcaagatgctccgttcggatgacagattcccttatttcacattgaggtatattgacgacatggagaagttcagcagaattcgttttcaaatacgactcggttcctatcgcttcaagttctacgacaagatgaacattgacggtaccccacgtatcagaagtctgcaaaaagaaatcaatggtttcggacgtctatccgacatggaaaacaagaggaaaagggaatggaaagacatgttccaagccaccgaagagatagattacgaggatcaatttggagactatcagacaggggtgacccaatttgtagaagacacggctgatacaaagccctatgttaccaaccatcgagcagcatacaatgttcacagtaatcatattggattgatttggaatgacgctgatagtataatactacaagatgacaataagttgtttttccctgacttgaagattgacgagaatggaaaggcagatatttatcaaccttccccaaaggcttcactcagcgtgttcgattttccagccatggtgttttacatgtacctgcgagagaagaccgaagcaacaaaagaattcccttcagccgaacaactcatcatcaacaaatatgaccatttggttcgattctttaaagatatttccgatggcagatttggaccatcagaaaacaagaacgcttttagcaaaaagctcaaggaagaatatgatttgaaaaccggggaaataccggaaaagctcctgcactggctttcctctgagtcagaagaagacccttccgaaaaatatgcgaagaagcttgaagaagaaatcaaactgcgcagagaacgtgttcaacgtagattggaaaaattcaaccaagaccttagagagataagaaagaaagattccgttccatatgggaaaaaaggtcatgtgaatatccgccacagccaattagccaaatacctaatgaggtctatcatggagtggcaacccacaagaaatgatggaaagaacaaactgactggccaaaacttcaatgtgatgaccgctttccttgccactttaggatatacctcacaagtgaaggatttacgggatttattctctcgtgccaacatgttggaaggtcccaatgcacaccccttcttgaagaaagtgttgaacaataactcgattaaagatatacagggtttttaccggacatatctggtagaagaacttaaccaaatagaagacaagcaaagaaggatcgccaaagctaaaaacgtcaaagatacggtacgccaattcccgtttgctcattttaaccgtatgaggtaccagaaacgagatgaagattattacaggaatttggcaaagagatatctgaatataggcgacaatgaaaaggacaaggctgtcattttgttgcccgacggcatgttcactagttacatctacgacctcattatgaaactccctgaaaacaatgagaagatgcgaatcaacttagccagcgatgtagcccattgcaattcctccttcttaatcagccgcttttttgaaaatattagaaacgactatgctcaacctttctatcgtgaggaaagaacgtatgaactgtttagcatcctaaataacaaaaaagtaagaaatactcttcaacccttatttattagtccccatgatatcaatatccagcttacggagaaagaaaaggatggtaaaggacggcttatcttacaaaagatagatcatttttgcaaatctatcacacaaaaagggaacttcaacaatgtggaagaagccaaagaagccacttctcgcaaattgaaacatctcattaccgattgcaagaacaacgaacgggatatccgccgatataagactcaagacatggtgatttacttgatggcccgcgacattcttaaagacatcatccccgacagcgaaaaagacaaatatgcaaaagaccgcaaattattgctaaaagatgtatgcgaagaaggcttcttacgtcaagccgtcaagatggagtatgagtattctattgaggaaaaagggaaaaggaccagaaccgttaaaatcacccatcctaatatgtctttgaagaactatggtgagtttcaccgtttactcaacgatgaacgccttaaatcattgttacaacagttggctaatatggatgagatcgactatacggatttgatgggggaatttgctgattacgaccaaaaacgttcagaaatcttccgcctagcgcaatccatagagaaacatctttacgagcagaacgagcaagggcttaacgatgaaaagagcgacctcttttatcatactagatacaatggcaaaaagataccacgccgaaacagtttcagttcactgctggaattgataggagaagaagagtcccaaatgaccgaaacagataagaagcaaactatcagcatccgaaatgcctttgggcacaacacttataaagtgtctctcgcagagatgaatgctactgaacttcccaatgtggcaaaaaccattctcaagaaaatggaagaactgagaaacaagctctaa

SEQ ID NO: 62 - RNA, 36 nt, synthetic construct
  source 1..36: mol_type = other RNA
gttgtagaagcctatcgttaggataggtatgacaac

SEQ ID NO: 63 - protein, 1335 aa, synthetic construct
MEKHHSQPRKAQFPFSISEKSVMGGYFNIARLNFYKTIVTIFAQVGVKGEYPEDKIDRVLDALYKNIAGKDNELSKEQAQWKRLKQLKGEQITKLQRLLFNHFPVLGPIMASEASYKIYKSELNAKEAEDAVQNDKEELKKIKKSNVINNEQLMRGVGIDDCLNVLATMAACLTDCRNYYSHYIPYNSIEDQKKQYKRQAQIARWLDKVIVASRRIDKQRNSLTTNEMEFLTGIDHYFQQDKKDDTGKLIRDEKGRTLKEFVEYPDYYFRIKGERQLVDIAGKTLNEEQAQNALTDFGIVFFCTLFLQKTYAKMMQEELKLYENGPYRGDVKGKENDDAKKNTILREMLSIYRIRVPRGKRLDSKDDATTLSMDMLNELRKCPMPLYDVLGKDGQRFFEDEVQHPNEQTPEKVKRLRATDRFPHLALRYIDLHDKTFTRIRFQVQLGNFRFKFYNKKTIDGAEEVRSIQKEINGYGRLQEIEAKRLETYAPLFQKSELVSTKLEHEDLNLDLVQFTEDHADSKPYITNHRATYNIHNNRIGMYWEASQNVKEYKVFSSDGMYLPTLNTIDGKAPISMPAPKASLSIYELPAMLFYQYLLDNNNVKKNEYDAPQDILINKHDALVKFFEAVRGGELIPALSKDELSRKLESEYDLKISEVPNKLVDYLIGKEDNGKRLYDYATHEVLLRLRRSLRRFEHFEEDRKMIGSKDNKYGKKGFVDVRHGRLAQYLAESIMDWRKPLNGEKDKLTGLNYSKMQAALATFGGKTTFDKLNTLFKEAGLYDNRPGSHPFLQSTMQKAPQNIEMLYLAYLEAETDKLKKFVVIKNLNNLSEKELKEYKDLVTFTVKEKRTYSDGRTKMVMVDKVAVNIIGNTNFANLPFIHHQRARFAQRNAEYYKSLAGRYLSVDGKSATIQLPDGIFTKHILKLLKEKYATHEALQLHLTDDDMNHNAAYLISSFFETVLNDCSQPYYRTFHYENNEKKTSKFAHIYDLFNILNNVKEANAYKPYPMTTDDINSRLTKKATNRDGLFVIRKDDNGEDYLVKQITLDIENHLKKMEDAVEAKIKFKNLYGYNADKARKNGAEEREKMLRKLTHCISDVKNNERAIRRYKTQDMVLFLLAKSTLSTILAQQNGVASEELFRLKNVCNNNFLSQTVRFEFPIKVNEMTIKVVQENMALKNYGEFYRFINDDRLMSLLTQLKDVTEISYADLTGELATYDLRRSQVFRLMQELEKIAFEQHTKELTNIDNSMFFKDGDMNNVPRRNNFKALINLFDSIDSHQLTKDDCERLVEIRNAFCHNTYRINIDDLQEKLPTIAIQIVGKIENLLKGADMKK

SEQ ID NO: 64 - RNA, 36 nt, synthetic construct
  source 1..36: mol_type = other RNA
gttttcatacctatccaaacgataggcttctaaaac

SEQ ID NO: 65 - protein, 1124 aa, synthetic construct
MEDDKKTTGSISYELKDKHFWAAFLNLARHNVYITINHINKLLEIREIDNDEKVLDIKTLWQKGNKDLNQKARLRELMTKHFPFLETAIYTKNKEDKKEVKQEKQAEAQSLESLKDCLFLFLDKLQEARNYYSHYKYSEFSKEPEFEEGLLEKMYNIFGNNIQLVINDYQHNKDINPDEDFKHLDRKGQFKYSFADNEGNITESGLLFFVSLFLEKKDAIWMQQKLNGFKDNLENKKKMTHEVFCRSRILMPKLRLESTQTQDWILLDMLNELIRCPKSLYERLQGDDREKFKVPFDPADEDYNAEQEPFKNTLIRHQDRFPYFVLRYFDYNEIFKNLRFQIDLGTYHFSIYKKLIGGQKEDRHLTHKLYGFERIQEFAKQNRPDEWKAIVKDLDTYETSNKRYISETTPHYHLENQKIGIRFRNGNKEIWPSLKTNDENNEKSKYKLDKQYQAEAFLSVHELLPMMFYYLLLKKEKPNNDEINASIVEGFIKREIRNIFKLYDAFANGEINNIDDLEKYCADKGIPKRHLPKQMVAILYDEHKDMVKEAKRKQKEMVKDTKKLLATLEKQTQKEKEDDGRNVKLLKSGEIARWLVNDMMRFQPVQKDNEGKPLNNSKANSTEYQMLQRSLALYNNEEKPTRYFRQVNLIESNNPHPFLKWTKWEECNNILTFYYSYLTKKIEFLNKLKPEDWKKNQYFLKLKEPKTNRETLVQGWKNGFNLPRGIFTEPIREWFKRHQNNSKEYEKVEALDRVGLVTKVIPLFFKEEYFKDKEENFKEDTQKEINDCVQPFYNFPYNVGNIHKPKEKDFLHREERIELWDKKKDKFKGYKEKIKSKKLTEKDKEEFRSYLEFQSWNKFERELRLVRNQDIVTWLLCKELIDKLKIDELNIEELKKLRLNNIDTDTAKKEKNNILNRVMPMELPVTVYEIDDSHKIVKDKPLHTIYIKEAETKLLKQGNFKALVKDRRLNGLFSFVKTNSEAESKRNPISKLRVEYELGEYQEARIEIIQDMLALEEKLINKYKDLPTNKFSEMLNSWLEGKDEADKARFQNDVDFLIAVRNAFSHNQYPMHNKIEFANIKPFSLYTANNSEEKGLGIANQLKDKTKETTDKIKKIEKPIETKE

SEQ ID NO: 66 - RNA, 37 nt, synthetic construct
  source 1..37: mol_type = other RNA
gttgtttttacctttcaaacagaaggcagatacaaca

SEQ ID NO: 67 - DNA, 7679 bp, synthetic construct
  source 1..7679: mol_type = other DNA
cctgcaggcagctgcgcgctcgctcgctcactgaggccgcccgggcgtcgggcgacctttggtcgcccggcctcagtgagcgagcgagcgcgcagagagggagtggccaactccatcactaggggttcctgcggcctctagactcgaggcgttgacattgattattgactagttattaatagtaatcaattacggggtcattagttcatagcccatatatggagttccgcgttacataacttacggtaaatggcccgcctggctgaccgcccaacgacccccgcccattgacgtcaataatgacgtatgttcccatagtaacgccaatagggactttccattgacgtcaatgggtggagtatttacggtaaactgcccacttggcagtacatcaagtgtatcatatgccaagtacgccccctattgacgtcaatgacggtaaatggcccgcctggcattatgcccagtacatgaccttatgggactttcctacttggcagtacatctacgtattagtcatcgctattaccatggtgatgcggttttggcagtacatcaatgggcgtggatagcggtttgactcacggggatttccaagtctccaccccattgacgtcaatgggagtttgttttggcaccaaaatcaacgggactttccaaaatgtcgtaacaactccgccccattgacgcaaatgggcggtaggcgtgtacggtgggaggtctatataagcagagctctctggctaactaccggtgccaccatgccggcagctaagaaaaagaaactggatggcagcgtcgacatgaaggagcagaagaagttcagcctgcagggcgtgagacacgtgtgcggcagctacttcaacatggccctgaacaactactgcagaaccctgaacggcgtgttcatcaagtgcaagatcaagttcgccctgaaggaggacgacttccccagaagcctgagcagcctgagaaagatcttcagcagcggccccatcatgccccagaccgagaagaaggtggccaagatgatcgccagcgtggacaccgccatgaagctgaagcagcagctgttcaagcacttccccatgctgggccccatcatggacaagaccatcagctgcatgaaccaccacaagggcagcagcgtggccgacgcccccctggacctgtgcatgaacgccatcctgaacttcggcgagtgcctgtaccactgcagaaacttctacacccacttcaagccctacaacagccccgaggacctgaagctgcagtacgacatccagcacatcatcgccctgaacctgggcaccctgttcgacgtgagcagaagaatcggcaagaagagagagggcctgacccccgaggagctggagttcctgaccggcaagaacagattcaaccaggtgggcaagaagttcctggagagaaacgactggtacttgaagatcgagaagcccagcgacatgaaggactacgacaagaccatcctgagcgacttcggcatggtgtacctgtgcagcatcttcctggccaagaactacgccctgagactgttcgacgagagcaagctgttcaacaaggagacaatcagaaacctgttcagcgaggagcaggtgagattcctgaaggagatgctggtgatctacagaatcagaacccccagaggcaagcagctggacagccacgacagcaagcaggccctggccatggacatgctgaacgagctgagaaagtgccccagacccctgtacgacgtgctgagcgaggagtacaagaagagaaccttctacgtgcccgtggagcacgagaacgagaaaaccgaggagtacgtgaagatgctgagaagcgacgacagattcccctacttcaccctgagatacatcgacgacatggagaagttcagcagaatcagattccagatcagactgggcagctacagattcaagttctacgacaagatgaacatcgacggcacccccagaatcagaagcctgcagaaggagatcaacggcttcggcagactgagcgacatggagaacaagagaaagagagagtggaaggacatgttccaggccaccgaggagatcgactacgaggaccagttcggcgactaccagaccggcgtgacccagttcgtggaggacaccgccgacaccaagccctacgtgaccaaccacagagccgcctacaacgtgcacagcaaccacatcggcctgatctggaacgacgccgacagcatcatcctgcaggacgacaacaagctgttcttccccgacctgaagatcgacgagaacggcaaggccgacatctaccagcccagccccaaggccagcctgagcgtgttcgacttccccgccatggtgttctacatgtacctgagagagaaaaccgaggccaccaaggagttccccagcgccgagcagctgatcatcaacaagtacgaccacctggtgagattcttcaaggacatcagcgacggcagattcggccccagcgagaacaagaacgccttcagcaagaagctgaaggaggagtacgacctgaaaaccggcgagatccccgagaagctgctgcactggctgagcagcgagagcgaggaggaccccagcgagaagtacgccaagaagctggaggaggagatcaagctgagaagagagagagtgcagagaagattggagaagttcaaccaggacctgagagagatcagaaagaaggacagcgtgccctacggcaagaagggccacgtgaacatcagacacagccagctggccaagtacctgatgagaagcatcatggagtggcagcccaccagaaacgacggcaagaacaagctgaccggccagaacttcaacgtgatgaccgccttcctggccaccctgggctacaccagccaggtgaaggacctgagagacttgttcagcagagccaacatgctggagggccccaacgcccaccccttcctgaagaaggtgctgaacaacaacagcatcaaggacatccagggcttctacagaacctacctggtggaggagctgaaccagatcgaggacaagcagagaagaatcgccaaggccaagaacgtgaaggacaccgtgagacagttccccttcgcccacttcaacagaatgagataccagaagagagacgaggactactacagaaacctggccaagagatacctgaacatcggcgacaacgagaaggacaaggccgtgatcctgctgcccgacggcatgttcaccagctacatctacgacctgatcatgaagctgcccgagaacaacgagaagatgagaatcaacctggccagcgacgtggcccactgcaacagcagcttcctgatcagcagattcttcgagaacatcagaaacgactacgcccagcccttctacagagaggagagaacctacgagctgttcagcatcctgaacaacaagaaggtgagaaacaccctgcagcccctgttcatcagcccccacgacatcaacatccagctgaccgagaaggagaaggacggcaagggcagactgatcctgcagaagatcgaccacttctgcaagagcatcacccagaagggcaacttcaacaacgtggaggaggccaaggaggccaccagcagaaagctgaagcacctgatcaccgactgcaagaacaacgagagagacatcagaagatacaagacccaggacatggtgatctacctgatggccagagacatcctgaaggacatcatccccgacagcgagaaggacaagtacgccaaggacagaaagctgctgctgaaggacgtgtgcgaggagggcttcctgagacaggccgtgaagatggagtacgagtacagcatcgaggagaagggcaagagaaccagaaccgtgaagatcacccaccccaacatgagcctgaagaactacggcgagttccacagactgctgaacgacgagagactgaagagcctgctgcagcagctggccaacatggacgagatcgactacaccgacctgatgggcgagttcgccgactacgaccagaagagaagcgagatcttcagactggcccagagcatcgagaagcacctgtacgagcagaacgagcagggcctgaacgacgagaagagcgacctgttctaccacaccagatacaacggcaagaagatccccagaagaaacagcttcagcagcctgctggagctgatcggcgaggaggagagccagatgaccgagacagacaagaagcagaccatcagcatcagaaacgccttcggccacaacacctacaaggtgagcctggccgagatgaacgccaccgagctgcccaacgtggccaagaccatcctgaagaagatggaggagctgagaaacaagctgacaggcggcggccccggcggcggcgccgccgccggcagcggcagccctaagaaaaaacgaaaagttggcagcggaagcaaaaggccggcggccacgaaaaaggccggccaggcaaaaaagaaaaagctcgagtacccatacgatgttccagattacgcttgagaattccccttgagcatctgacttctggctaataaaggaaatttattttcattgcaatagtgtgttggaattttttgtgtctctcaggtaccgagggcctatttcccatgattccttcatatttgcatatacgatacaaggctgttagagagataattggaattaatttgactgtaaacacaaagatattagtacaaaatacgtgacgtagaaagtaataatttcttgggtagtttgcagttttaaaattatgttttaaaatggactatcatatgcttaccgtaacttgaaagtatttcgatttcttggctttatatatcttgtggaaaggacgaaacaccggagaccacggcaggtctcagttgtagaagcctatcgttaggataggtatgacaactttttttgcggccgcaggaacccctagtgatggagttggccactccctctctgcgcgctcgctcgctcactgaggccgggcgaccaaaggtcgcccgacgcccgggctttgcccgggcggcctcagtgagcgagcgagcgcgcagctgcctgcaggggcgcctgatgcggtattttctccttacgcatctgtgcggtatttcacaccgcatacgtcaaagcaaccatagtacgcgccctgtagcggcgcattaagcgcggcgggtgtggtggttacgcgcagcgtgaccgctacacttgccagcgccttagcgcccgctcctttcgctttcttcccttcctttctcgccacgttcgccggctttccccgtcaagctctaaatcgggggctccctttagggttccgatttagtgctttacggcacctcgaccccaaaaaacttgatttgggtgatggttcacgtagtgggccatcgccctgatagacggtttttcgccctttgacgttggagtccacgttctttaatagtggactcttgttccaaactggaacaacactcaactctatctcgggctattcttttgatttataagggattttgccgatttcggtctattggttaaaaaatgagctgatttaacaaaaatttaacgcgaattttaacaaaatattaacgtttacaattttatggtgcactctcagtacaatctgctctgatgccgcatagttaagccagccccgacacccgccaacacccgctgacgcgccctgacgggcttgtctgctcccggcatccgcttacagacaagctgtgaccgtctccgggagctgcatgtgtcagaggttttcaccgtcatcaccgaaacgcgcgagacgaaagggcctcgtgatacgcctatttttataggttaatgtcatgataataatggtttcttagacgtcaggtggcacttttcggggaaatgtgcgcggaacccctatttgtttatttttctaaatacattcaaatatgtatccgctcatgagacaataaccctgataaatgcttcaataatattgaaaaaggaagagtatgagtattcaacatttccgtgtcgcccttattcccttttttgcggcattttgccttcctgtttttgctcacccagaaacgctggtgaaagtaaaagatgctgaagatcagttgggtgcacgagtgggttacatcgaactggatctcaacagcggtaagatccttgagagttttcgccccgaagaacgttttccaatgatgagcacttttaaagttctgctatgtggcgcggtattatcccgtattgacgccgggcaagagcaactcggtcgccgcatacactattctcagaatgacttggttgagtactcaccagtcacagaaaagcatcttacggatggcatgacagtaagagaattatgcagtgctgccataaccatgagtgataacactgcggccaacttacttctgacaacgatcggaggaccgaaggagctaaccgcttttttgcacaacatgggggatcatgtaactcgccttgatcgttgggaaccggagctgaatgaagccataccaaacgacgagcgtgacaccacgatgcctgtagcaatggcaacaacgttgcgcaaactattaactggcgaactacttactctagcttcccggcaacaattaatagactggatggaggcggataaagttgcaggaccacttctgcgctcggcccttccggctggctggtttattgctgataaatctggagccggtgagcgtggaagccgcggtatcattgcagcactggggccagatggtaagccctcccgtatcgtagttatctacacgacggggagtcaggcaactatggatgaacgaaatagacagatcgctgagataggtgcctcactgattaagcattggtaactgtcagaccaagtttactcatatatactttagattgatttaaaacttcatttttaatttaaaaggatctaggtgaagatcctttttgataatctcatgaccaaaatcccttaacgtgagttttcgttccactgagcgtcagaccccgtagaaaagatcaaaggatcttcttgagatcctttttttctgcgcgtaatctgctgcttgcaaacaaaaaaaccaccgctaccagcggtggtttgtttgccggatcaagagctaccaactctttttccgaaggtaactggcttcagcagagcgcagataccaaatactgttcttctagtgtagccgtagttaggccaccacttcaagaactctgtagcaccgcctacatacctcgctctgctaatcctgttaccagtggctgctgccagtggcgataagtcgtgtcttaccgggttggactcaagacgatagttaccggataaggcgcagcggtcgggctgaacggggggttcgtgcacacagcccagcttggagcgaacgacctacaccgaactgagatacctacagcgtgagctatgagaaagcgccacgcttcccgaagggagaaaggcggacaggtatccggtaagcggcagggtcggaacaggagagcgcacgagggagcttccagggggaaacgcctggtatctttatagtcctgtcgggtttcgccacctctgacttgagcgtcgatttttgtgatgctcgtcaggggggcggagcctatggaaaaacgccagcaacgcggcctttttacggttcctggccttttgctggccttttgctcacatgt

SEQ ID NO: 68 - DNA, 26 bp, synthetic construct
  source 1..26: mol_type = other DNA
agggcagaaccgatgctgatgaagac

SEQ ID NO: 69 - DNA, 31 bp, synthetic construct
  source 1..31: mol_type = other DNA
caccgagggcagaaccgatgctgatgaagac

SEQ ID NO: 70 - DNA, 31 bp, synthetic construct
  source 1..31: mol_type = other DNA
caacgtcttcatcagcatcggttctgccctc

SEQ ID NO: 71 - DNA, 30 bp, synthetic construct
  source 1..30: mol_type = other DNA
aaacagggcagaaccgatgctgatgaagac

SEQ ID NO: 72 - DNA, 30 bp, synthetic construct
  source 1..30: mol_type = other DNA
cttggtcttcatcagcatcggttctgccct

SEQ ID NO: 73 - DNA, 21 bp, synthetic construct
  source 1..21: mol_type = other DNA
gcccatctacatccagttctc

SEQ ID NO: 74 - DNA, 21 bp, synthetic construct
  source 1..21: mol_type = other DNA
cagcccatctacatccagttc

SEQ ID NO: 75 - DNA, 58 bp, synthetic construct
  source 1..58: mol_type = other DNA
caccgcccatctacatccagttctcctcgaggagaactggatgtagatgggctttttt

SEQ ID NO: 76 - DNA, 58 bp, synthetic construct
  source 1..58: mol_type = other DNA
ggccaaaaaagcccatctacatccagttctcctcgaggagaactggatgtagatgggc

SEQ ID NO: 77 - DNA, 58 bp, synthetic construct
  source 1..58: mol_type = other DNA
cacccagcccatctacatccagttcctcgaggaactggatgtagatgggctgtttttt

SEQ ID NO: 78 - DNA, 58 bp, synthetic construct
  source 1..58: mol_type = other DNA
ggccaaaaaacagcccatctacatccagttcctcgaggaactggatgtagatgggctg

SEQ ID NO: 79 - DNA, 4828 bp, synthetic construct; identical to SEQ ID NO: 31
  source 1..4828: mol_type = other DNA

SEQ ID NO: 80 - RNA, 66 nt, synthetic construct
  source 1..66: mol_type = other RNA
gtggttggagaactggatgtagatgggctggttgtagatgacctcgttttggaggggaaacacaac

SEQ ID NO: 81 - RNA, 66 nt, synthetic construct
  source 1..66: mol_type = other RNA
gtggttggagaactggatgtagatgggctggttgtagaagccgttcattcgggacggtatgacaac

SEQ ID NO: 82 - RNA, 66 nt, synthetic construct
  source 1..66: mol_type = other RNA
gtggttggagaactggatgtagatgggctggttgtagaagcctatcgttaggataggtatgacaac

SEQ ID NO: 83 - DNA, 9067 bp, synthetic construct
  source 1..9067: mol_type = other DNA
tggcgaatgggacgcgccctgtagcggcgcattaagcgcggcgggtgtggtggttacgcgcagcgtgaccgctacacttgccagcgccctagcgcccgctcctttcgctttcttcccttcctttctcgccacgttcgccggctttccccgtcaagctctaaatcgggggctccctttagggttccgatttagtgctttacggcacctcgaccccaaaaaacttgattagggtgatggttcacgtagtgggccatcgccctgatagacggtttttcgccctttgacgttggagtccacgttctttaatagtggactcttgttccaaactggaacaacactcaaccctatctcggtctattcttttgatttataagggattttgccgatttcggcctattggttaaaaaatgagctgatttaacaaaaatttaacgcgaattttaacaaaatattaacgtttacaatttcaggtggcacttttcggggaaatgtgcgcggaacccctatttgtttatttttctaaatacattcaaatatgtatccgctcatgaattaattcttagaaaaactcatcgagcatcaaatgaaactgcaatttattcatatcaggattatcaataccatatttttgaaaaagccgtttctgtaatgaaggagaaaactcaccgaggcagttccataggatggcaagatcctggtatcggtctgcgattccgactcgtccaacatcaatacaacctattaatttcccctcgtcaaaaataaggttatcaagtgagaaatcaccatgagtgacgactgaatccggtgagaatggcaaaagtttatgcatttctttccagacttgttcaacaggccagccattacgctcgtcatcaaaatcactcgcatcaaccaaaccgttattcattcgtgattgcgcctgagcgagacgaaatacgcgatcgctgttaaaaggacaattacaaacaggaatcgaatgcaaccggcgcaggaacactgccagcgcatcaacaatattttcacctgaatcaggatattcttctaatacctggaatgctgttttcccggggatcgcagtggtgagtaaccatgcatcatcaggagtacggataaaatgcttgatggtcggaagaggcataaattccgtcagccagtttagtctgaccatctcatctgtaacatcattggcaacgctacctttgccatgtttcagaaacaactctggcgcatcgggcttcccatacaatcgatagattgtcgcacctgattgcccgacattatcgcgagcccatttatacccatataaatcagcatccatgttggaatttaatcgcggcctagagcaagacgtttcccgttgaatatggctcataacaccccttgtattactgtttatgtaagcagacagttttattgttcatgaccaaaatcccttaacgtgagttttcgttccactgagcgtcagaccccgtagaaaagatcaaaggatcttcttgagatcctttttttctgcgcgtaatctgctgcttgcaaacaaaaaaaccaccgctaccagcggtggtttgtttgccggatcaagagctaccaactctttttccgaaggtaactggcttcagcagagcgcagataccaaatactgtccttctagtgtagccgtagttaggccaccacttcaagaactctgtagcaccgcctacatacctcgctctgctaatcctgttaccagtggctgctgccagtggcgataagtcgtgtcttaccgggttggactcaagacgatagttaccggataaggcgcagcggtcgggctgaacggggggttcgtgcacacagcccagcttggagcgaacgacctacaccgaactgagatacctacagcgtgagctatgagaaagcgccacgcttcccgaagggagaaaggcggacaggtatccggtaagcggcagggtcggaacaggagagcgcacgagggagcttccagggggaaacgcctggtatctttatagtcctgtcgggtttcgccacctctgacttgagcgtcgatttttgtgatgctcgtcaggggggcggagcctatggaaaaacgccagcaacgcggcctttttacggttcctggccttttgctggccttttgctcacatgttctttcctgcgttatcccctgattctgtggataaccgtattaccgcctttgagtgagctgataccgctcgccgcagccgaacgaccgagcgcagcgagtcagtgagcgaggaagcggaagagcgcctgatgcggtattttctccttacgcatctgtgcggtatttcacaccgcatatatggtgcactctcagtacaatctgctctgatgccgcatagttaagccagtatacactccgctatcgctacgtgactgggtcatggctgcgccccgacacccgccaacacccgctgacgcgccctgacgggcttgtctgctcccggcatccgcttacagacaagctgtgaccgtctccgggagctgcatgtgtcagaggttttcaccgtcatcaccgaaacgcgcgaggcagctgcggtaaagctcatcagcgtggtcgtgaagcgattcacagatgtctgcctgttcatccgcgtccagctcgttgagtttctccagaagcgttaatgtctggcttctgataaagcgggccatgttaagggcggttttttcctgtttggtcactgatgcctccgtgtaagggggatttctgttcatgggggtaatgataccgatgaaacgagagaggatgctcacgatacgggttactgatgatgaacatgcccggttactggaacgttgtgagggtaaacaactggcggtatggatgcggcgggaccagagaaaaatcactcagggtcaatgccagcgcttcgttaatacagatgtaggtgttccacagggtagccagcagcatcctgcgatgcagatccggaacataatggtgcagggcgctgacttccgcgtttccagactttacgaaacacggaaaccgaagaccattcatgttgttgctcaggtcgcagacgttttgcagcagcagtcgcttcacgttcgctcgcgtatcggtgattcattctgctaaccagtaaggcaaccccgccagcctagccgggtcctcaacgacaggagcacgatcatgcgcacccgtggggccgccatgccggcgataatggcctgcttctcgccgaaacgtttggtggcgggaccagtgacgaaggcttgagcgagggcgtgcaagattccgaataccgcaagcgacaggccgatcatcgtcgcgctccagcgaaagcggtcctcgccgaaaatgacccagagcgctgccggcacctgtcctacgagttgcatgataaagaagacagtcataagtgcggcgacgatagtcatgccccgcgcccaccggaaggagctgactgggttgaaggctctcaagggcatcggtcgagatcccggtgcctaatgagtgagctaacttacattaattgcgttgcgctcactgcccgctttccagtcgggaaacctgtcgtgccagctgcattaatgaatcggccaacgcgcggggagaggcggtttgcgtattgggcgccagggtggtttttcttttcaccagtgagacgggcaacagctgattgcccttcaccgcctggccctgagagagttgcagcaagcggtccacgctggtttgccccagcaggcgaaaatcctgtttgatggtggttaacggcgggatataacatgagctgtcttcggtatcgtcgtatcccactaccgagatatccgcaccaacgcgcagcccggactcggtaatggcgcgcattgcgcccagcgccatctgatcgttggcaaccagcatcgcagtgggaacgatgccctcattcagcatttgcatggtttgttgaaaaccggacatggcactccagtcgccttcccgttccgctatcggctgaatttgattgcgagtgagatatttatgccagccagccagacgcagacgcgccgagacagaacttaatgggcccgctaacagcgcgatttgctggtgacccaatgcgaccagatgctccacgcccagtcgcgtaccgtcttcatgggagaaaataatactgttgatgggtgtctggtcagagacatcaagaaataacgccggaacattagtgcaggcagcttccacagcaatggcatcctggtcatccagcggatagttaatgatcagcccactgacgcgttgcgcgagaagattgtgcaccgccgctttacaggcttcgacgccgcttcgttctaccatcgacaccaccacgctggcacccagttgatcggcgcgagatttaatcgccgcgacaatttgcgacggcgcgtgcagggccagactggaggtggcaacgccaatcagcaacgactgtttgcccgccagttgttgtgccacgcggttgggaatgtaattcagctccgccatcgccgcttccactttttcccgcgttttcgcagaaacgtggctggcctggttcaccacgcgggaaacggtctgataagagacaccggcatactctgcgacatcgtataacgttactggtttcacattcaccaccctgaattgactctcttccgggcgctatcatgccataccgcgaaaggttttgcgccattcgatggtgtccgggatctcgacgctctcccttatgcgactcctgcattaggaagcagcccagtagtaggttgaggccgttgagcaccgccgccgcaaggaatggtgcatgcaaggagatggcgcccaacagtcccccggccacggggcctgccaccatacccacgccgaaacaagcgctcatgagcccgaagtggcgagcccgatcttccccatcggtgatgtcggcgatataggcgccagcaaccgcacctgtggcgccggtgatgccggccacgatgcgtccggcgtagaggatcgagatctcgatcccgcgaaattaatacgactcactataggggaattgtgagcggataacaattcccctctagaaataattttgtttaactttaagaaggagatataccatgggcagcagccatcatcatcatcatcacagcagcggcctggtgccgcgcggcagccatatggctagcatgactggtggacagcaaatgggtcgcggatccccggcagctaagaaaaagaaactggatggcagcgtcgacatgaaggagcagaagaagttcagcctgcagggcgtgagacacgtgtgcggcagctacttcaacatggccctgaacaactactgcagaaccctgaacggcgtgttcatcaagtgcaagatcaagttcgccctgaaggaggacgacttccccagaagcctgagcagcctgagaaagatcttcagcagcggccccatcatgccccagaccgagaagaaggtggccaagatgatcgccagcgtggacaccgccatgaagctgaagcagcagctgttcaagcacttccccatgctgggccccatcatggacaagaccatcagctgcatgaaccaccacaagggcagcagcgtggccgacgcccccctggacctgtgcatgaacgccatcctgaacttcggcgagtgcctgtaccactgcagaaacttctacacccacttcaagccctacaacagccccgaggacctgaagctgcagtacgacatccagcacatcatcgccctgaacctgggcaccctgttcgacgtgagcagaagaatcggcaagaagagagagggcctgacccccgaggagctggagttcctgaccggcaagaacagattcaaccaggtgggcaagaagttcctggagagaaacgactggtacttgaagatcgagaagcccagcgacatgaaggactacgacaagaccatcctgagcgacttcggcatggtgtacctgtgcagcatcttcctggccaagaactacgccctgagactgttcgacgagagcaagctgttcaacaaggagacaatcagaaacctgttcagcgaggagcaggtgagattcctgaaggagatgctggtgatctacagaatcagaacccccagaggcaagcagctggacagccacgacagcaagcaggccctggccatggacatgctgaacgagctgagaaagtgccccagacccctgtacgacgtgctgagcgaggagtacaagaagagaaccttctacgtgcccgtggagcacgagaacgagaaaaccgaggagtacgtgaagatgctgagaagcgacgacagattcccctacttcaccctgagatacatcgacgacatggagaagttcagcagaatcagattccagatcagactgggcagctacagattcaagttctacgacaagatgaacatcgacggcacccccagaatcagaagcctgcagaaggagatcaacggcttcggcagactgagcgacatggagaacaagagaaagagagagtggaaggacatgttccaggccaccgaggagatcgactacgaggaccagttcggcgactaccagaccggcgtgacccagttcgtggaggacaccgccgacaccaagccctacgtgaccaaccacagagccgcctacaacgtgcacagcaaccacatcggcctgatctggaacgacgccgacagcatcatcctgcaggacgacaacaagctgttcttccccgacctgaagatcgacgagaacggcaaggccgacatctaccagcccagccccaaggccagcctgagcgtgttcgacttccccgccatggtgttctacatgtacctgagagagaaaaccgaggccaccaaggagttccccagcgccgagcagctgatcatcaacaagtacgaccacctggtgagattcttcaaggacatcagcgacggcagattcggccccagcgagaacaagaacgccttcagcaagaagctgaaggaggagtacgacctgaaaaccggcgagatccccgagaagctgctgcactggctgagcagcgagagcgaggaggaccccagcgagaagtacgccaagaagctggaggaggagatcaagctgagaagagagagagtgcagagaagattggagaagttcaaccaggacctgagagagatcagaaagaaggacagcgtgccctacggcaagaagggccacgtgaacatcagacacagccagctggccaagtacctgatgagaagcatcatggagtggcagcccaccagaaacgacggcaagaacaagctgaccggccagaacttcaacgtgatgaccgccttcctggccaccctgggctacaccagccaggtgaaggacctgagagacttgttcagcagagccaacatgctggagggccccaacgcccaccccttcctgaagaaggtgctgaacaacaacagcatcaaggacatccagggcttctacagaacctacctggtggaggagctgaaccagatcgaggacaagcagagaagaatcgccaaggccaagaacgtgaaggacaccgtgagacagttccccttcgcccacttcaacagaatgagataccagaagagagacgaggactactacagaaacctggccaagagatacctgaacatcggcgacaacgagaaggacaaggccgtgatcctgctgcccgacggcatgttcaccagctacatctacgacctgatcatgaagctgcccgagaacaacgagaagatgagaatcaacctggccagcgacgtggcccactgcaacagcagcttcctgatcagcagattcttcgagaacatcagaaacgactacgcccagcccttctacagagaggagagaacctacgagctgttcagcatcctgaacaacaagaaggtgagaaacaccctgcagcccctgttcatcagcccccacgacatcaacatccagctgaccgagaaggagaaggacggcaagggcagactgatcctgcagaagatcgaccacttctgcaagagcatcacccagaagggcaacttcaacaacgtggaggaggccaaggaggccaccagcagaaagctgaagcacctgatcaccgactgcaagaacaacgagagagacatcagaagatacaagacccaggacatggtgatctacctgatggccagagacatcctgaaggacatcatccccgacagcgagaaggacaagtacgccaaggacagaaagctgctgctgaaggacgtgtgcgaggagggcttcctgagacaggccgtgaagatggagtacgagtacagcatcgaggagaagggcaagagaaccagaaccgtgaagatcacccaccccaacatgagcctgaagaactacggcgagttccacagactgctgaacgacgagagactgaagagcctgctgcagcagctggccaacatggacgagatcgactacaccgacctgatgggcgagttcgccgactacgaccagaagagaagcgagatcttcagactggcccagagcatcgagaagcacctgtacgagcagaacgagcagggcctgaacgacgagaagagcgacctgttctaccacaccagatacaacggcaagaagatccccagaagaaacagcttcagcagcctgctggagctgatcggcgaggaggagagccagatgaccgagacagacaagaagcagaccatcagcatcagaaacgccttcggccacaacacctacaaggtgagcctggccgagatgaacgccaccgagctgcccaacgtggccaagaccatcctgaagaagatggaggagctgagaaacaagctgacaggcggcggccccggcggcggcgccgccgccggcagcggcagccctaagaaaaaacgaaaagttggcagcggaagcaaaaggccggcggccacgaaaaaggccggccaggcaaaaaagaaaaagtaactcgagcaccaccaccaccaccactgagatccggctgctaacaaagcccgaaaggaagctgagttggctgctgccaccgctgagcaataactagcataaccccttggggcctctaaacgggtcttgaggggttttttgctgaaaggaggaactatatccggat

SEQ ID NO: 84 - protein, 10 aa, synthetic construct
  VARIANT 9: note = X is S or T.
LXXXRNXYXH

SEQ ID NO: 85 - protein, 12 aa, synthetic construct
  VARIANT 7: note = X is V or I.
RXXXKXXNGFGR

SEQ ID NO: 86 - protein, 19 aa, synthetic construct
  VARIANT 3: note = X is I or V.
  VARIANT 12: note = X is I or V.
PYXTXXXXXYXXXXNXIGL

SEQ ID NO: 87 - protein, 15 aa, synthetic construct
  VARIANT 3: note = X is A or C.
  VARIANT 9: note = X is E or D.
  VARIANT 10: note = X is L or F.
PXXXLSXXXXPAXXF

SEQ ID NO: 88 - protein, 13 aa, synthetic construct
  VARIANT 2: note = X is D, R or K.
  VARIANT 7: note = X is D or S.
  VARIANT 8: note = X is M or I.
  VARIANT 9: note = X is M or V.
  VARIANT 11: note = X is F or W.
AXXLXXXXXXXQP

SEQ ID NO: 89 - protein, 6 aa, synthetic construct
KLTXXN

SEQ ID NO: 90 - protein, 12 aa, synthetic construct
  VARIANT 7: note = X is L or M.
IXLPXGXFXXXI

SEQ ID NO: 91 - protein, 13 aa, synthetic construct
  VARIANT 1: note = X is D or N.
  VARIANT 2: note = X is T or N.
  VARIANT 6: note = X is I or L.
  VARIANT 7: note = X is K or R.
  VARIANT 8: note = X is V or R.
  VARIANT 10: note = X is K or R.
XXEXXXXXYXXQD

SEQ ID NO: 92 - protein, 9 aa, synthetic construct
  VARIANT 3: note = X is S or A.
  VARIANT 4: note = X is F or A.
RNXXXHXXY

SEQ ID NO: 93 - protein, 10 aa, synthetic construct
  VARIANT 2: note = X is R, V or Y.
  VARIANT 3: note = X is E, Y or H.
  VARIANT 4: note = X is L, Y or C.
  VARIANT 7: note = X is V, F or M.
  VARIANT 9: note = X is S or T.
LXXXRNXYXH

SEQ ID NO: 94 - protein, 12 aa, synthetic construct
  VARIANT 2: note = X is S or T.
  VARIANT 3: note = X is I, V or L.
  VARIANT 4: note = X is S or Q.
  VARIANT 6: note = X is N, A or E.
  VARIANT 7: note = X is V or I.
RXXXKXXNGFGR

SEQ ID NO: 95 - protein, 19 aa, synthetic construct
  VARIANT 3: note = X is I or V.
  VARIANT 5: note = X is D or N.
  VARIANT 6: note = X is H or W.
  VARIANT 7: note = X is H or R.
  VARIANT 8: note = X is A or T.
  VARIANT 9: note = X is K, A or T.
  VARIANT 11: note = X is L or N.
  VARIANT 12: note = X is I or V.
  VARIANT 13: note = X is H or S.
  VARIANT 14: note = X is N, S or A.
  VARIANT 15: note = X is R or H.
PYXTXXXXXYXXXXNXIGL

SEQ ID NO: 96 - protein, 20 aa, synthetic construct
  VARIANT 2: note = X isT, M or K.
  VARIANT 3: note = X is A or C.
  VARIANT 4: note = X is W, Y or S.
  VARIANT 7: note = X is I or V.
  VARIANT 8: note = X is F or Y.
  VARIANT 9: note = X is E or D.
  VARIANT 10: note = X is L or F.
  VARIANT 13: note = X is L or M.
  VARIANT 14: note = X is A, L or V.
  VARIANT 16: note = X is L or Y.
  VARIANT 17: note = X is L, C or M.
  VARIANT 18: note = X is H or Y.
  VARIANT 19: note = X is L or I.
  VARIANT 20: note = X is Y or R.
PXXXLSXXXXPAXXFXXXXX

SEQ ID NO: 97 - protein, 13 aa, synthetic construct
  VARIANT 2: note = X is D, R or K.
  VARIANT 3: note = X is F or Y.
  VARIANT 5: note = X is A or M.
  VARIANT 6: note = X is H, T or R.
  VARIANT 7: note = X is D or S.
  VARIANT 8: note = X is M or I.
  VARIANT 9: note = X is M or V.
  VARIANT 10: note = X is F, R or E.
  VARIANT 11: note = X is F or W.
AXXLXXXXXXXQP

SEQ ID NO: 98 - protein, 9 aa, synthetic construct
  VARIANT 1: note = X is C or G.
  VARIANT 2: note = X is N, G or K.
  VARIANT 3: note = X is N or D.
  VARIANT 7: note = X is G or S.
  VARIANT 8: note = X is L, A or Q.
XXXKLTXXN

SEQ ID NO: 99 - protein, 14 aa, synthetic construct
  VARIANT 1: note = X is K or A.
  VARIANT 2: note = X is S, P or V.
  VARIANT 4: note = X is E, L or M.
  VARIANT 7: note = X is R or D.
  VARIANT 9: note = X is L or M.
  VARIANT 11: note = X is E or T.
  VARIANT 12: note = X is S or T.
  VARIANT 13: note = X is Y or H.
XXIXLPXGXFXXXI

SEQ ID NO: 100 - protein, 19 aa, synthetic construct
  VARIANT 1: note = X is L or I.
  VARIANT 5: note = X is Y, W or F.
  VARIANT 12: note = X is D or Q.
  VARIANT 16: note = X is P or T.
  VARIANT 19: note = X is D or R.
XIXXXFXXXXXXXXQXFYX

SEQ ID NO: 101 - protein, 13 aa, synthetic construct
  VARIANT 1: note = X is D or N.
  VARIANT 2: note = X is T or N.
  VARIANT 4: note = X is K, T or R.
  VARIANT 5: note = X is E or D.
  VARIANT 6: note = X is I or L.
  VARIANT 7: note = X is K or R.
  VARIANT 8: note = X is V or R.
  VARIANT 10: note = X is K or R.
  VARIANT 11: note = X is I, L or T.
XXEXXXXXYXXQD

SEQ ID NO: 102 - protein, 10 aa, synthetic construct
  VARIANT 3: note = X is S or A.
  VARIANT 4: note = X is F or A.
  VARIANT 5: note = X is A or G.
  VARIANT 7: note = X is N or L.
  VARIANT 8: note = X is S, R or T.
  VARIANT 10: note = X is P or K.
RNXXXHXXYX

SEQ ID NO: 103 - DNA, 18 bp, synthetic construct
  source 1..18: mol_type = other DNA
gggtcttcgagaagacct

SEQ ID NO: 104 - DNA, 24 bp, synthetic construct
  source 1..24: mol_type = other DNA
gatcaacattaaatgtgagcgagt

SEQ ID NO: 105 - DNA, 7690 bp, synthetic construct
  source 1..7690: mol_type = other DNA
cctgcaggcagctgcgcgctcgctcgctcactgaggccgcccgggcgtcgggcgacctttggtcgcccggcctcagtgagcgagcgagcgcgcagagagggagtggccaactccatcactaggggttcctgcggcctctagactcgaggcgttgacattgattattgactagttattaatagtaatcaattacggggtcattagttcatagcccatatatggagttccgcgttacataacttacggtaaatggcccgcctggctgaccgcccaacgacccccgcccattgacgtcaataatgacgtatgttcccatagtaacgccaatagggactttccattgacgtcaatgggtggagtatttacggtaaactgcccacttggcagtacatcaagtgtatcatatgccaagtacgccccctattgacgtcaatgacggtaaatggcccgcctggcattatgcccagtacatgaccttatgggactttcctacttggcagtacatctacgtattagtcatcgctattaccatggtgatgcggttttggcagtacatcaatgggcgtggatagcggtttgactcacggggatttccaagtctccaccccattgacgtcaatgggagtttgttttggcaccaaaatcaacgggactttccaaaatgtcgtaacaactccgccccattgacgcaaatgggcggtaggcgtgtacggtgggaggtctatataagcagagctctctggctaactaccggtgccaccatgccggcagctaagaaaaagaaactggatggcagcgtcgacatgaaggagcagaagaagttcagcctgcagggcgtgagacacgtgtgcggcagctacttcaacatggccctgaacaactactgcagaaccctgaacggcgtgttcatcaagtgcaagatcaagttcgccctgaaggaggacgacttccccagaagcctgagcagcctgagaaagatcttcagcagcggccccatcatgccccagaccgagaagaaggtggccaagatgatcgccagcgtggacaccgccatgaagctgaagcagcagctgttcaagcacttccccatgctgggccccatcatggacaagaccatcagctgcatgaaccaccacaagggcagcagcgtggccgacgcccccctggacctgtgcatgaacgccatcctgaacttcggcgagtgcctgtaccactgcagaaacttctacacccacttcaagccctacaacagccccgaggacctgaagctgcagtacgacatccagcacatcatcgccctgaacctgggcaccctgttcgacgtgagcagaagaatcggcaagaagagagagggcctgacccccgaggagctggagttcctgaccggcaagaacagattcaaccaggtgggcaagaagttcctggagagaaacgactggtacttgaagatcgagaagcccagcgacatgaaggactacgacaagaccatcctgagcgacttcggcatggtgtacctgtgcagcatcttcctggccaagaactacgccctgagactgttcgacgagagcaagctgttcaacaaggagacaatcagaaacctgttcagcgaggagcaggtgagattcctgaaggagatgctggtgatctacagaatcagaacccccagaggcaagcagctggacagccacgacagcaagcaggccctggccatggacatgctgaacgagctgagaaagtgccccagacccctgtacgacgtgctgagcgaggagtacaagaagagaaccttctacgtgcccgtggagcacgagaacgagaaaaccgaggagtacgtgaagatgctgagaagcgacgacagattcccctacttcaccctgagatacatcgacgacatggagaagttcagcagaatcagattccagatcagactgggcagctacagattcaagttctacgacaagatgaacatcgacggcacccccagaatcagaagcctgcagaaggagatcaacggcttcggcagactgagcgacatggagaacaagagaaagagagagtggaaggacatgttccaggccaccgaggagatcgactacgaggaccagttcggcgactaccagaccggcgtgacccagttcgtggaggacaccgccgacaccaagccctacgtgaccaaccacagagccgcctacaacgtgcacagcaaccacatcggcctgatctggaacgacgccgacagcatcatcctgcaggacgacaacaagctgttcttccccgacctgaagatcgacgagaacggcaaggccgacatctaccagcccagccccaaggccagcctgagcgtgttcgacttccccgccatggtgttctacatgtacctgagagagaaaaccgaggccaccaaggagttccccagcgccgagcagctgatcatcaacaagtacgaccacctggtgagattcttcaaggacatcagcgacggcagattcggccccagcgagaacaagaacgccttcagcaagaagctgaaggaggagtacgacctgaaaaccggcgagatccccgagaagctgctgcactggctgagcagcgagagcgaggaggaccccagcgagaagtacgccaagaagctggaggaggagatcaagctgagaagagagagagtgcagagaagattggagaagttcaaccaggacctgagagagatcagaaagaaggacagcgtgccctacggcaagaagggccacgtgaacatcagacacagccagctggccaagtacctgatgagaagcatcatggagtggcagcccaccagaaacgacggcaagaacaagctgaccggccagaacttcaacgtgatgaccgccttcctggccaccctgggctacaccagccaggtgaaggacctgagagacttgttcagcagagccaacatgctggagggccccaacgcccaccccttcctgaagaaggtgctgaacaacaacagcatcaaggacatccagggcttctacagaacctacctggtggaggagctgaaccagatcgaggacaagcagagaagaatcgccaaggccaagaacgtgaaggacaccgtgagacagttccccttcgcccacttcaacagaatgagataccagaagagagacgaggactactacagaaacctggccaagagatacctgaacatcggcgacaacgagaaggacaaggccgtgatcctgctgcccgacggcatgttcaccagctacatctacgacctgatcatgaagctgcccgagaacaacgagaagatgagaatcaacctggccagcgacgtggcccactgcaacagcagcttcctgatcagcagattcttcgagaacatcagaaacgactacgcccagcccttctacagagaggagagaacctacgagctgttcagcatcctgaacaacaagaaggtgagaaacaccctgcagcccctgttcatcagcccccacgacatcaacatccagctgaccgagaaggagaaggacggcaagggcagactgatcctgcagaagatcgaccacttctgcaagagcatcacccagaagggcaacttcaacaacgtggaggaggccaaggaggccaccagcagaaagctgaagcacctgatcaccgactgcaagaacaacgagagagacatcagaagatacaagacccaggacatggtgatctacctgatggccagagacatcctgaaggacatcatccccgacagcgagaaggacaagtacgccaaggacagaaagctgctgctgaaggacgtgtgcgaggagggcttcctgagacaggccgtgaagatggagtacgagtacagcatcgaggagaagggcaagagaaccagaaccgtgaagatcacccaccccaacatgagcctgaagaactacggcgagttccacagactgctgaacgacgagagactgaagagcctgctgcagcagctggccaacatggacgagatcgactacaccgacctgatgggcgagttcgccgactacgaccagaagagaagcgagatcttcagactggcccagagcatcgagaagcacctgtacgagcagaacgagcagggcctgaacgacgagaagagcgacctgttctaccacaccagatacaacggcaagaagatccccagaagaaacagcttcagcagcctgctggagctgatcggcgaggaggagagccagatgaccgagacagacaagaagcagaccatcagcatcagaaacgccttcggccacaacacctacaaggtgagcctggccgagatgaacgccaccgagctgcccaacgtggccaagaccatcctgaagaagatggaggagctgagaaacaagctgacaggcggcggccccggcggcggcgccgccgccggcagcggcagccctaagaaaaaacgaaaagttggcagcggaagcaaaaggccggcggccacgaaaaaggccggccaggcaaaaaagaaaaagctcgagtacccatacgatgttccagattacgcttgagaattccccttgagcatctgacttctggctaataaaggaaatttattttcattgcaatagtgtgttggaattttttgtgtctctcaggtaccgagggcctatttcccatgattccttcatatttgcatatacgatacaaggctgttagagagataattggaattaatttgactgtaaacacaaagatattagtacaaaatacgtgacgtagaaagtaataatttcttgggtagtttgcagttttaaaattatgttttaaaatggactatcatatgcttaccgtaacttgaaagtatttcgatttcttggctttatatatcttgtggaaaggacgaaacaccgtgccgttcttctgcttgtcggccatgatatgttgtagaagcctatcgttaggataggtatgacaactttttttgcggccgcaggaacccctagtgatggagttggccactccctctctgcgcgctcgctcgctcactgaggccgggcgaccaaaggtcgcccgacgcccgggctttgcccgggcggcctcagtgagcgagcgagcgcgcagctgcctgcaggggcgcctgatgcggtattttctccttacgcatctgtgcggtatttcacaccgcatacgtcaaagcaaccatagtacgcgccctgtagcggcgcattaagcgcggcgggtgtggtggttacgcgcagcgtgaccgctacacttgccagcgccttagcgcccgctcctttcgctttcttcccttcctttctcgccacgttcgccggctttccccgtcaagctctaaatcgggggctccctttagggttccgatttagtgctttacggcacctcgaccccaaaaaacttgatttgggtgatggttcacgtagtgggccatcgccctgatagacggtttttcgccctttgacgttggagtccacgttctttaatagtggactcttgttccaaactggaacaacactcaactctatctcgggctattcttttgatttataagggattttgccgatttcggtctattggttaaaaaatgagctgatttaacaaaaatttaacgcgaattttaacaaaatattaacgtttacaattttatggtgcactctcagtacaatctgctctgatgccgcatagttaagccagccccgacacccgccaacacccgctgacgcgccctgacgggcttgtctgctcccggcatccgcttacagacaagctgtgaccgtctccgggagctgcatgtgtcagaggttttcaccgtcatcaccgaaacgcgcgagacgaaagggcctcgtgatacgcctatttttataggttaatgtcatgataataatggtttcttagacgtcaggtggcacttttcggggaaatgtgcgcggaacccctatttgtttatttttctaaatacattcaaatatgtatccgctcatgagacaataaccctgataaatgcttcaataatattgaaaaaggaagagtatgagtattcaacatttccgtgtcgcccttattcccttttttgcggcattttgccttcctgtttttgctcacccagaaacgctggtgaaagtaaaagatgctgaagatcagttgggtgcacgagtgggttacatcgaactggatctcaacagcggtaagatccttgagagttttcgccccgaagaacgttttccaatgatgagcacttttaaagttctgctatgtggcgcggtattatcccgtattgacgccgggcaagagcaactcggtcgccgcatacactattctcagaatgacttggttgagtactcaccagtcacagaaaagcatcttacggatggcatgacagtaagagaattatgcagtgctgccataaccatgagtgataacactgcggccaacttacttctgacaacgatcggaggaccgaaggagctaaccgcttttttgcacaacatgggggatcatgtaactcgccttgatcgttgggaaccggagctgaatgaagccataccaaacgacgagcgtgacaccacgatgcctgtagcaatggcaacaacgttgcgcaaactattaactggcgaactacttactctagcttcccggcaacaattaatagactggatggaggcggataaagttgcaggaccacttctgcgctcggcccttccggctggctggtttattgctgataaatctggagccggtgagcgtggaagccgcggtatcattgcagcactggggccagatggtaagccctcccgtatcgtagttatctacacgacggggagtcaggcaactatggatgaacgaaatagacagatcgctgagataggtgcctcactgattaagcattggtaactgtcagaccaagtttactcatatatactttagattgatttaaaacttcatttttaatttaaaaggatctaggtgaagatcctttttgataatctcatgaccaaaatcccttaacgtgagttttcgttccactgagcgtcagaccccgtagaaaagatcaaaggatcttcttgagatcctttttttctgcgcgtaatctgctgcttgcaaacaaaaaaaccaccgctaccagcggtggtttgtttgccggatcaagagctaccaactctttttccgaaggtaactggcttcagcagagcgcagataccaaatactgttcttctagtgtagccgtagttaggccaccacttcaagaactctgtagcaccgcctacatacctcgctctgctaatcctgttaccagtggctgctgccagtggcgataagtcgtgtcttaccgggttggactcaagacgatagttaccggataaggcgcagcggtcgggctgaacggggggttcgtgcacacagcccagcttggagcgaacgacctacaccgaactgagatacctacagcgtgagctatgagaaagcgccacgcttcccgaagggagaaaggcggacaggtatccggtaagcggcagggtcggaacaggagagcgcacgagggagcttccagggggaaacgcctggtatctttatagtcctgtcgggtttcgccacctctgacttgagcgtcgatttttgtgatgctcgtcaggggggcggagcctatggaaaaacgccagcaacgcggcctttttacggttcctggccttttgctggccttttgctcacatgt